European Patent Application EP 4 252 857 A2, published October 4, 2023. Title: METHODS FOR REDUCING LIPOPROTEIN(A) LEVELS BY ADMINISTERING AN INHIBITOR OF PROPROTEIN CONVERTASE SUBTILISIN KEXIN-9 (PCSK9). Applicant: Regeneron Pharmaceuticals, Inc. The sequence listing filed with the application follows.

SEQUENCE LISTING (763 sequences)

SEQ ID NO: 1 - DNA, 351 bp, synthetic construct
  misc_feature 1..351: note = Synthetic
  source 1..351: mol_type = other DNA
caggtccagctggtgcagtctgggggaggcttggtacagcctggggggtccctgagactctcctgtgcagcctctggatttactctaagtagttacgacatgcactgggtccgccaatctacaggaaaaggtctggagtgggtctcagctattggttctaccggtgacacatactatccaggctccgtgaagggccgattcaccatcaccagagaaaaagccaagaactccgtgtatcttcaaatgaacagcctgagagccggggacacggctgtgtattactgtgtaagagaggggtgggaggtaccctttgactactggggccagggaaccctggtcactgtctcctca

SEQ ID NO: 2 - protein, 117 aa, synthetic construct
  REGION 1..117: note = Synthetic
QVQLVQSGGGLVQPGGSLRLSCAASGFTLSSYDMHWVRQSTGKGLEWVSAIGSTGDTYYPGSVKGRFTITREKAKNSVYLQMNSLRAGDTAVYYCVREGWEVPFDYWGQGTLVTVSS

SEQ ID NO: 3 - DNA, 24 bp, synthetic construct
  misc_feature 1..24: note = Synthetic
  source 1..24: mol_type = other DNA
ggatttactctaagtagttacgac

SEQ ID NO: 4 - protein, 8 aa, synthetic construct
  REGION 1..8: note = Synthetic
GFTLSSYD

SEQ ID NO: 5 - DNA, 21 bp, synthetic construct
  misc_feature 1..21: note = Synthetic
  source 1..21: mol_type = other DNA
attggttctaccggtgacaca

SEQ ID NO: 6 - protein, 7 aa, synthetic construct
  REGION 1..7: note = Synthetic
IGSTGDT

SEQ ID NO: 7 - DNA, 33 bp, synthetic construct
  misc_feature 1..33: note = Synthetic
  source 1..33: mol_type = other DNA
gtaagagaggggtgggaggtaccctttgactac

SEQ ID NO: 8 - protein, 11 aa, synthetic construct
  REGION 1..11: note = Synthetic
VREGWEVPFDY

SEQ ID NO: 9 - DNA, 327 bp, synthetic construct
  misc_feature 1..327: note = Synthetic
  source 1..327: mol_type = other DNA
gacatccagatgacccagtctccagccaccctgtctgtgtctccaggggaaagagccgccctctcctgcagggccagtcagagtgttagcagcaacttagcctggtaccaccagaaacctggccaggctcccaggctcctcatctatggtgcatccaccagggccactggtatcccagccaggttcagtggcattgggtctgggacagagttcactctcattatcagcagcctgcagtctgaagattttgcattttatttctgtcagcagtataataactggcctccattcactttcggccctgggaccaaggtggagatcaaacga

SEQ ID NO: 10 - protein, 109 aa, synthetic construct
  REGION 1..109: note = Synthetic
DIQMTQSPATLSVSPGERAALSCRASQSVSSNLAWYHQKPGQAPRLLIYGASTRATGIPARFSGIGSGTEFTLIISSLQSEDFAFYFCQQYNNWPPFTFGPGTKVEIKR

SEQ ID NO: 11 - DNA, 18 bp, synthetic construct
  misc_feature 1..18: note = Synthetic
  source 1..18: mol_type = other DNA
cagagtgttagcagcaac

SEQ ID NO: 12 - protein, 6 aa, synthetic construct
  REGION 1..6: note = Synthetic
QSVSSN

SEQ ID NO: 13-14 - skipped (2 entries)

SEQ ID NO: 15 - DNA, 30 bp, synthetic construct
  misc_feature 1..30: note = Synthetic
  source 1..30: mol_type = other DNA
cagcagtataataactggcctccattcact

SEQ ID NO: 16 - protein, 10 aa, synthetic construct
  REGION 1..10: note = Synthetic
QQYNNWPPFT

SEQ ID NO: 17 - DNA, 351 bp, synthetic construct
  misc_feature 1..351: note = Synthetic
  source 1..351: mol_type = other DNA
gaggtgcagctggtggagtctgggggaggcttggtacagcctggggggtccctgagactctcctgtgcagcctctggatttactctaagtagttacgacatgcactgggtccgccaatctacaggaaaaggtctggagtgggtctcagctattggttctaccggtgacacatactatccaggctccgtgaagggccgattcaccatcaccagagaaaaagccaagaactccgtgtatcttcaaatgaacagcctgagagccggggacacggctgtgtattactgtgtaagagaggggtgggaggtaccctttgactactggggccagggaaccctggtcaccgtctcctca

SEQ ID NO: 18 - protein, 117 aa, synthetic construct
  REGION 1..117: note = Synthetic
EVQLVESGGGLVQPGGSLRLSCAASGFTLSSYDMHWVRQSTGKGLEWVSAIGSTGDTYYPGSVKGRFTITREKAKNSVYLQMNSLRAGDTAVYYCVREGWEVPFDYWGQGTLVTVSS

SEQ ID NO: 19 - DNA, 324 bp, synthetic construct
  misc_feature 1..324: note = Synthetic
  source 1..324: mol_type = other DNA
gaaatagtgatgacgcagtctccagccaccctgtctgtgtctccaggggaaagagccgccctctcctgcagggccagtcagagtgttagcagcaacttagcctggtaccaccagaaacctggccaggctcccaggctcctcatctatggtgcatccaccagggccactggtatcccagccaggttcagtggcattgggtctgggacagagttcactctcattatcagcagcctgcagtctgaagattttgcattttatttctgtcagcagtataataactggcctccattcactttcggccctgggaccaaagtggatatcaaa

SEQ ID NO: 20 - protein, 108 aa, synthetic construct
  REGION 1..108: note = Synthetic
EIVMTQSPATLSVSPGERAALSCRASQSVSSNLAWYHQKPGQAPRLLIYGASTRATGIPARFSGIGSGTEFTLIISSLQSEDFAFYFCQQYNNWPPFTFGPGTKVDIK

SEQ ID NO: 21 - DNA, 351 bp, synthetic construct
  misc_feature 1..351: note = Synthetic
  source 1..351: mol_type = other DNA
gaggtgcagctggtggagtctgggggaggcttggtacagcctggggggtccctgagactctcctgtgcagcctctggatttactctaagtagttacgacatgcactgggtccgccaagctacaggaaaaggtctggagtgggtctcagctattggttctaccggtgacacatactatccaggctccgtgaagggccgattcaccatctccagagaaaatgccaagaactccttgtatcttcaaatgaacagcctgagagccggggacacggctgtgtattactgtgtaagagaggggtgggaggtaccctttgactactggggccagggaaccctggtcaccgtctcctca

SEQ ID NO: 22 - protein, 117 aa, synthetic construct
  REGION 1..117: note = Synthetic
EVQLVESGGGLVQPGGSLRLSCAASGFTLSSYDMHWVRQATGKGLEWVSAIGSTGDTYYPGSVKGRFTISRENAKNSLYLQMNSLRAGDTAVYYCVREGWEVPFDYWGQGTLVTVSS

SEQ ID NO: 23 - DNA, 324 bp, synthetic construct
  misc_feature 1..324: note = Synthetic
  source 1..324: mol_type = other DNA
gaaatagtgatgacgcagtctccagccaccctgtctgtgtctccaggggaaagagccaccctctcctgcagggccagtcagagtgttagcagcaacttagcctggtaccagcagaaacctggccaggctcccaggctcctcatctatggtgcatccaccagggccactggtatcccagccaggttcagtggcagtgggtctgggacagagttcactctcaccatcagcagcctgcagtctgaagattttgcagtttattactgtcagcagtataataactggcctccattcactttcggccctgggaccaaagtggatatcaaa

SEQ ID NO: 24 - protein, 108 aa, synthetic construct
  REGION 1..108: note = Synthetic
EIVMTQSPATLSVSPGERATLSCRASQSVSSNLAWYQQKPGQAPRLLIYGASTRATGIPARFSGSGSGTEFTLTISSLQSEDFAVYYCQQYNNWPPFTFGPGTKVDIK

SEQ ID NO: 25 - DNA, 342 bp, synthetic construct
  misc_feature 1..342: note = Synthetic
  source 1..342: mol_type = other DNA
caggtgcagctggtgcagtctgggggaggcgtggtccagcctgggaggtccctgagactctcctgtgcagcgtctggattcaccttcagtagctatggcatgcactgggtccgccaggctccaggcaaggggctggagtgggtggcgtttataggatttgatggaagtaatatacattatggagactccgtgaggggccgaatcatcatatccagagacaattccgagaacacgttgtatctggaaatgaacagcctgagagccgaggacacggcaatgtactattgtgcgagagagaagggtttagactggggccagggaaccacggtcaccgtctcctca

SEQ ID NO: 26 - protein, 114 aa, synthetic construct
  REGION 1..114: note = Synthetic
QVQLVQSGGGVVQPGRSLRLSCAASGFTFSSYGMHWVRQAPGKGLEWVAFIGFDGSNIHYGDSVRGRIIISRDNSENTLYLEMNSLRAEDTAMYYCAREKGLDWGQGTTVTVSS

SEQ ID NO: 27 - DNA, 24 bp, synthetic construct
  misc_feature 1..24: note = Synthetic
  source 1..24: mol_type = other DNA
ggattcaccttcagtagctatggc

SEQ ID NO: 28 - protein, 8 aa, synthetic construct
  REGION 1..8: note = Synthetic
GFTFSSYG

SEQ ID NO: 29 - DNA, 24 bp, synthetic construct
  misc_feature 1..24: note = Synthetic
  source 1..24: mol_type = other DNA
ataggatttgatggaagtaatata

SEQ ID NO: 30 - protein, 8 aa, synthetic construct
  REGION 1..8: note = Synthetic
IGFDGSNI

SEQ ID NO: 31 - DNA, 21 bp, synthetic construct
  misc_feature 1..21: note = Synthetic
  source 1..21: mol_type = other DNA
gcgagagagaagggtttagac

SEQ ID NO: 32 - protein, 7 aa, synthetic construct
  REGION 1..7: note = Synthetic
AREKGLD

SEQ ID NO: 33 - DNA, 321 bp, synthetic construct
  misc_feature 1..321: note = Synthetic
  source 1..321: mol_type = other DNA
gccatccagatgacccagtctccttccaccctgtctgcatctgtaggagacagagtcaccatcacttgccgggccagtcagagtattagtagctggttggcctggtatcagcagaaaccagggaaagcccctaagctcctgatctataaggcgtctagtttagaaagtggggtcccatcaaggttcagcggcagtggatctgggacagaattcactctcaccatcagcagcctgcagcctgatgattttgcaacttattactgccaacagtataatagttattacacttttggccaggggaccaaggtggaaatcaaacga

SEQ ID NO: 34 - protein, 107 aa, synthetic construct
  REGION 1..107: note = Synthetic
AIQMTQSPSTLSASVGDRVTITCRASQSISSWLAWYQQKPGKAPKLLIYKASSLESGVPSRFSGSGSGTEFTLTISSLQPDDFATYYCQQYNSYYTFGQGTKVEIKR

SEQ ID NO: 35 - DNA, 18 bp, synthetic construct
  misc_feature 1..18: note = Synthetic
  source 1..18: mol_type = other DNA
cagagtattagtagctgg

SEQ ID NO: 36 - protein, 6 aa, synthetic construct
  REGION 1..6: note = Synthetic
QSISSW

SEQ ID NO: 37-38 - skipped (2 entries)

SEQ ID NO: 39 - DNA, 24 bp, synthetic construct
  misc_feature 1..24: note = Synthetic
  source 1..24: mol_type = other DNA
caacagtataatagttattacact

SEQ ID NO: 40 - protein, 8 aa, synthetic construct
  REGION 1..8: note = Synthetic
QQYNSYYT

SEQ ID NO: 41 - DNA, 342 bp, synthetic construct
  misc_feature 1..342: note = Synthetic
  source 1..342: mol_type = other DNA
caggtgcagctggtggagtctgggggaggcgtggtccagcctgggaggtccctgagactctcctgtgcagcgtctggattcaccttcagtagctatggcatgcactgggtccgccaggctccaggcaaggggctggagtgggtggcgtttataggatttgatggaagtaatatacattatggagactccgtgaggggccgaatcatcatatccagagacaattccgagaacacgttgtatctggaaatgaacagcctgagagccgaggacacggcaatgtactattgtgcgagagagaagggtttagactggggccagggaaccctggtcaccgtctcctca

SEQ ID NO: 42 - protein, 114 aa, synthetic construct
  REGION 1..114: note = Synthetic
QVQLVESGGGVVQPGRSLRLSCAASGFTFSSYGMHWVRQAPGKGLEWVAFIGFDGSNIHYGDSVRGRIIISRDNSENTLYLEMNSLRAEDTAMYYCAREKGLDWGQGTLVTVSS

SEQ ID NO: 43 - DNA, 318 bp, synthetic construct
  misc_feature 1..318: note = Synthetic
  source 1..318: mol_type = other DNA
gacatccagatgacccagtctccttccaccctgtctgcatctgtaggagacagagtcaccatcacttgccgggccagtcagagtattagtagctggttggcctggtatcagcagaaaccagggaaagcccctaagctcctgatctataaggcgtctagtttagaaagtggggtcccatcaaggttcagcggcagtggatctgggacagaattcactctcaccatcagcagcctgcagcctgatgattttgcaacttattactgccaacagtataatagttattacacttttggccaggggaccaagctggagatcaaa

SEQ ID NO: 44 - protein, 106 aa, synthetic construct
  REGION 1..106: note = Synthetic
DIQMTQSPSTLSASVGDRVTITCRASQSISSWLAWYQQKPGKAPKLLIYKASSLESGVPSRFSGSGSGTEFTLTISSLQPDDFATYYCQQYNSYYTFGQGTKLEIK

SEQ ID NO: 45 - DNA, 342 bp, synthetic construct
  misc_feature 1..342: note = Synthetic
  source 1..342: mol_type = other DNA
caggtgcagctggtggagtctgggggaggcgtggtccagcctgggaggtccctgagactctcctgtgcagcctctggattcaccttcagtagctatggcatgcactgggtccgccaggctccaggcaaggggctggagtgggtggcagttataggatttgatggaagtaatatatactatgcagactccgtgaagggccgattcaccatctccagagacaattccaagaacacgctgtatctgcaaatgaacagcctgagagctgaggacacggctgtgtattactgtgcgagagagaagggtttagactggggccagggaaccctggtcaccgtctcctca

SEQ ID NO: 46 - protein, 114 aa, synthetic construct
  REGION 1..114: note = Synthetic
QVQLVESGGGVVQPGRSLRLSCAASGFTFSSYGMHWVRQAPGKGLEWVAVIGFDGSNIYYADSVKGRFTISRDNSKNTLYLQMNSLRAEDTAVYYCAREKGLDWGQGTLVTVSS

SEQ ID NO: 47 - DNA, 319 bp, synthetic construct
  misc_feature 1..319: note = Synthetic
  source 1..319: mol_type = other DNA
gacatccagatgacccagtctccttccaccctgtctgcatctgtaggagacagagtcaccatcacttgccgggccagtcagagtattagtagctggttggcctggtatcagcagaaaccagggaaagcccctaagctcctgatctataaggcgtctagtttagaaagtggggtcccatcaaggttcagcggcagtggatctgggacagaattcactctcaccatcagcagcctgcagcctgatgattttgcaacttattactgccaacagtataatagttattacacttttggccaggggaccaagctggagatcaaac

SEQ ID NO: 48 - protein, 106 aa, synthetic construct; identical to SEQ ID NO: 44
  REGION 1..106: note = Synthetic

SEQ ID NO: 49 - DNA, 342 bp, synthetic construct
  misc_feature 1..342: note = Synthetic
  source 1..342: mol_type = other DNA
caggtgcagctgcaggagtctgggggaggcgtggtccagcctgggaggtccctgagactctcctgtgcagcgtctggattcaccttcagtagctatggcatgcactgggtccgccaggctccaggcaaggggctggagtgggtggcgtttataggatttgatggaagtaatatatattatggagactccgtgaggggccgaatcatcatatccagagacaattccgagaacacgttgtatctggaaatgaacagcctgagagccgaggacacggcagtgtattattgtgcgagagagaagggtttagactggggccagggaaccctggtcactgtctcctca

SEQ ID NO: 50 - protein, 114 aa, synthetic construct
  REGION 1..114: note = Synthetic
QVQLQESGGGVVQPGRSLRLSCAASGFTFSSYGMHWVRQAPGKGLEWVAFIGFDGSNIYYGDSVRGRIIISRDNSENTLYLEMNSLRAEDTAVYYCAREKGLDWGQGTLVTVSS

SEQ ID NO: 51 - DNA, 24 bp, synthetic construct
  misc_feature 1..24: note = Synthetic
  source 1..24: mol_type = other DNA
ggattcaccttcagtagctatggc

SEQ ID NO: 52 - protein, 8 aa, synthetic construct
  REGION 1..8: note = Synthetic
GFTFSSYG

SEQ ID NO: 53 - DNA, 24 bp, synthetic construct
  misc_feature 1..24: note = Synthetic
  source 1..24: mol_type = other DNA
ataggatttgatggaagtaatata

SEQ ID NO: 54 - protein, 8 aa, synthetic construct
  REGION 1..8: note = Synthetic
IGFDGSNI

SEQ ID NO: 55 - DNA, 21 bp, synthetic construct
  misc_feature 1..21: note = Synthetic
  source 1..21: mol_type = other DNA
gcgagagagaagggtttagac

SEQ ID NO: 56 - protein, 7 aa, synthetic construct
  REGION 1..7: note = Synthetic
AREKGLD

SEQ ID NO: 57 - DNA, 342 bp, synthetic construct
  misc_feature 1..342: note = Synthetic
  source 1..342: mol_type = other DNA
gccatccagatgacccagtctccagactccctggctgtgtctctgggcgagagggccaccatcaactgcaagtccagccagagtgtttttcacacctccaacaataagaactacttagtttggtatcagcagaaaccaggacagcctcctaagttgctcctttactgggcctctacccgggaatccggggtccctgaccgattcagtggcagcgggtctgggacagatttcactctcaccatcagcagcctgcaggctgaagatgtggcaaattattactgtcaccaatattacagtattccgtggacgttcggccaagggaccaaggtggagatcaaacga

SEQ ID NO: 58 - protein, 114 aa, synthetic construct
  REGION 1..114: note = Synthetic
AIQMTQSPDSLAVSLGERATINCKSSQSVFHTSNNKNYLVWYQQKPGQPPKLLLYWASTRESGVPDRFSGSGSGTDFTLTISSLQAEDVANYYCHQYYSIPWTFGQGTKVEIKR

SEQ ID NO: 59 - DNA, 36 bp, synthetic construct
  misc_feature 1..36: note = Synthetic
  source 1..36: mol_type = other DNA
cagagtgtttttcacacctccaacaataagaactac

SEQ ID NO: 60 - protein, 12 aa, synthetic construct
  REGION 1..12: note = Synthetic
QSVFHTSNNKNY

SEQ ID NO: 61-62 - skipped (2 entries)

SEQ ID NO: 63 - DNA, 27 bp, synthetic construct
  misc_feature 1..27: note = Synthetic
  source 1..27: mol_type = other DNA
caccaatattacagtattccgtggacg

SEQ ID NO: 64 - protein, 9 aa, synthetic construct
  REGION 1..9: note = Synthetic
HQYYSIPWT

SEQ ID NO: 65 - DNA, 342 bp, synthetic construct
  misc_feature 1..342: note = Synthetic
  source 1..342: mol_type = other DNA
caggtgcagctggtggagtctgggggaggcgtggtccagcctgggaggtccctgagactctcctgtgcagcgtctggattcaccttcagtagctatggcatgcactgggtccgccaggctccaggcaaggggctggagtgggtggcgtttataggatttgatggaagtaatatatattatggagactccgtgaggggccgaatcatcatatccagagacaattccgagaacacgttgtatctggaaatgaacagcctgagagccgaggacacggcagtgtattattgtgcgagagagaagggtttagactggggccagggaaccctggtcaccgtctcctca

SEQ ID NO: 66 - protein, 114 aa, synthetic construct
  REGION 1..114: note = Synthetic
QVQLVESGGGVVQPGRSLRLSCAASGFTFSSYGMHWVRQAPGKGLEWVAFIGFDGSNIYYGDSVRGRIIISRDNSENTLYLEMNSLRAEDTAVYYCAREKGLDWGQGTLVTVSS

SEQ ID NO: 67 - DNA, 339 bp, synthetic construct
  misc_feature 1..339: note = Synthetic
  source 1..339: mol_type = other DNA
gacatcgtgatgacccagtctccagactccctggctgtgtctctgggcgagagggccaccatcaactgcaagtccagccagagtgtttttcacacctccaacaataagaactacttagtttggtatcagcagaaaccaggacagcctcctaagttgctcctttactgggcctctacccgggaatccggggtccctgaccgattcagtggcagcgggtctgggacagatttcactctcaccatcagcagcctgcaggctgaagatgtggcaaattattactgtcaccaatattacagtattccgtggacgttcggccaagggaccaaggtggaaatcaaa

SEQ ID NO: 68 - protein, 113 aa, synthetic construct
  REGION 1..113: note = Synthetic
DIVMTQSPDSLAVSLGERATINCKSSQSVFHTSNNKNYLVWYQQKPGQPPKLLLYWASTRESGVPDRFSGSGSGTDFTLTISSLQAEDVANYYCHQYYSIPWTFGQGTKVEIK

SEQ ID NO: 69 - DNA, 342 bp, synthetic construct; identical to SEQ ID NO: 45
  misc_feature 1..342: note = Synthetic
  source 1..342: mol_type = other DNA

SEQ ID NO: 70 - protein, 114 aa, synthetic construct; identical to SEQ ID NO: 46
  REGION 1..114: note = Synthetic

SEQ ID NO: 71 - DNA, 339 bp, synthetic construct
  misc_feature 1..339: note = Synthetic
  source 1..339: mol_type = other DNA
gacatcgtgatgacccagtctccagactccctggctgtgtctctgggcgagagggccaccatcaactgcaagtccagccagagtgtttttcacacctccaacaataagaactacttagcttggtaccagcagaaaccaggacagcctcctaagctgctcatttactgggcctctacccgggaatccggggtccctgaccgattcagtggcagcgggtctgggacagatttcactctcaccatcagcagcctgcaggctgaagatgtggcagtttattactgtcaccaatattacagtattccgtggacgttcggccaagggaccaaggtggaaatcaaa

SEQ ID NO: 72 - protein, 113 aa, synthetic construct
  REGION 1..113: note = Synthetic
DIVMTQSPDSLAVSLGERATINCKSSQSVFHTSNNKNYLAWYQQKPGQPPKLLIYWASTRESGVPDRFSGSGSGTDFTLTISSLQAEDVAVYYCHQYYSIPWTFGQGTKVEIK

SEQ ID NO: 73 - DNA, 354 bp, synthetic construct
  misc_feature 1..354: note = Synthetic
  source 1..354: mol_type = other DNA
gaagtgcagctggtgcagtctgggggaggcttggtacagcctggggggtccctgagactctcctgtgcagcctctggattcacctttaacaactatgccatgaactgggtccgccaggctccaggaaagggactggactgggtctcaactattagtggtagcggtggtactacaaactacgcagactccgtgaagggccgtttcattatttcccgagacagttccaaacacacgctgtatctgcaaatgaacagcctgagagccgaggacacggccgtatattactgtgcgaaagattctaactggggaaatttcgatctctggggccgtggcaccacggtcactgtctcctca

SEQ ID NO: 74 - protein, 118 aa, synthetic construct
  REGION 1..118: note = Synthetic
EVQLVQSGGGLVQPGGSLRLSCAASGFTFNNYAMNWVRQAPGKGLDWVSTISGSGGTTNYADSVKGRFIISRDSSKHTLYLQMNSLRAEDTAVYYCAKDSNWGNFDLWGRGTTVTVSS

SEQ ID NO: 75 - DNA, 24 bp, synthetic construct
  misc_feature 1..24: note = Synthetic
  source 1..24: mol_type = other DNA
ggattcacctttaacaactatgcc

SEQ ID NO: 76 - protein, 8 aa, synthetic construct
  REGION 1..8: note = Synthetic
GFTFNNYA

SEQ ID NO: 77 - DNA, 24 bp, synthetic construct
  misc_feature 1..24: note = Synthetic
  source 1..24: mol_type = other DNA
attagtggtagcggtggtactaca

SEQ ID NO: 78 - protein, 8 aa, synthetic construct
  REGION 1..8: note = Synthetic
ISGSGGTT

SEQ ID NO: 79 - DNA, 33 bp, synthetic construct
  misc_feature 1..33: note = Synthetic
  source 1..33: mol_type = other DNA
gcgaaagattctaactggggaaatttcgatctc

SEQ ID NO: 80 - protein, 11 aa, synthetic construct
  REGION 1..11: note = Synthetic
AKDSNWGNFDL

SEQ ID NO: 81 - DNA, 342 bp, synthetic construct
  misc_feature 1..342: note = Synthetic
  source 1..342: mol_type = other DNA
gacatccagatgacccagtctccagactccctggctgtgtctctgggcgagagggccaccatcaactgcaagtccagccagagtgttttatacaggtccaacaataggaacttcttaggttggtaccagcagaaaccagggcagcctcctaatctactcatttactgggcatctacccgggaatccggggtccctgaccgattcagtggcagcgggtctgggacagatttcactctcaccatcagcagcctgcaggctgaagatgtggcagtttattactgtcaacaatattatactactccgtacacttttggccaggggaccaaggtggaaatcaaacga

SEQ ID NO: 82 - protein, 114 aa, synthetic construct
  REGION 1..114: note = Synthetic
DIQMTQSPDSLAVSLGERATINCKSSQSVLYRSNNRNFLGWYQQKPGQPPNLLIYWASTRESGVPDRFSGSGSGTDFTLTISSLQAEDVAVYYCQQYYTTPYTFGQGTKVEIKR

SEQ ID NO: 83 - DNA, 36 bp, synthetic construct
  misc_feature 1..36: note = Synthetic
  source 1..36: mol_type = other DNA
cagagtgttttatacaggtccaacaataggaacttc

SEQ ID NO: 84 - protein, 12 aa, synthetic construct
  REGION 1..12: note = Synthetic
QSVLYRSNNRNF

SEQ ID NO: 85-86 - skipped (2 entries)

SEQ ID NO: 87 - DNA, 27 bp, synthetic construct
  misc_feature 1..27: note = Synthetic
  source 1..27: mol_type = other DNA
caacaatattatactactccgtacact

SEQ ID NO: 88 - protein, 9 aa, synthetic construct
  REGION 1..9: note = Synthetic
QQYYTTPYT

SEQ ID NO: 89 - DNA, 354 bp, synthetic construct
  misc_feature 1..354: note = Synthetic
  source 1..354: mol_type = other DNA
gaggtgcagctggtggagtctgggggaggcttggtacagcctggggggtccctgagactctcctgtgcagcctctggattcacctttaacaactatgccatgaactgggtccgccaggctccaggaaagggactggactgggtctcaactattagtggtagcggtggtactacaaactacgcagactccgtgaagggccgtttcattatttcccgagacagttccaaacacacgctgtatctgcaaatgaacagcctgagagccgaggacacggccgtatattactgtgcgaaagattctaactggggaaatttcgatctctggggccgtggcaccctggtcactgtctcctca

SEQ ID NO: 90 - protein, 118 aa, synthetic construct [sequence omitted]

SEQ ID NO: 91 - DNA, 339 bp, synthetic construct
  misc_feature 1..339: note = Synthetic
  source 1..339: mol_type = other DNA
gacatcgtgatgacccagtctccagactccctggctgtgtctctgggcgagagggccaccatcaactgcaagtccagccagagtgttttatacaggtccaacaataggaacttcttaggttggtaccagcagaaaccagggcagcctcctaatctactcatttactgggcatctacccgggaatccggggtccctgaccgattcagtggcagcgggtctgggacagatttcactctcaccatcagcagcctgcaggctgaagatgtggcagtttattactgtcaacaatattatactactccgtacacttttggccaggggaccaagctggagatcaaa

SEQ ID NO: 92 - protein, 113 aa, synthetic construct [sequence omitted]

SEQ ID NO: 93 - DNA, 354 bp, synthetic construct
  misc_feature 1..354: note = Synthetic
  source 1..354: mol_type = other DNA
gaggtgcagctggtggagtctgggggaggcttggtacagcctggggggtccctgagactctcctgtgcagcctctggattcacctttaacaactatgccatgagctgggtccgccaggctccagggaaggggctggagtgggtctcagctattagtggtagcggtggtactacatactacgcagactccgtgaagggccggttcaccatctccagagacaattccaagaacacgctgtatctgcaaatgaacagcctgagagccgaggacacggccgtatattactgtgcgaaagattctaactggggaaatttcgatctctggggccgtggcaccctggtcactgtctcctca

SEQ ID NO: 94 - protein, 118 aa, synthetic construct
  REGION 1..118: note = Synthetic
EVQLVESGGGLVQPGGSLRLSCAASGFTFNNYAMSWVRQAPGKGLEWVSAISGSGGTTYYADSVKGRFTISRDNSKNTLYLQMNSLRAEDTAVYYCAKDSNWGNFDLWGRGTLVTVSS

SEQ ID NO: 95 - DNA, 339 bp, synthetic construct
  misc_feature 1..339: note = Synthetic
  source 1..339: mol_type = other DNA
gacatcgtgatgacccagtctccagactccctggctgtgtctctgggcgagagggccaccatcaactgcaagtccagccagagtgttttatacaggtccaacaataggaacttcttagcttggtaccagcagaaaccaggacagcctcctaagctgctcatttactgggcatctacccgggaatccggggtccctgaccgattcagtggcagcgggtctgggacagatttcactctcaccatcagcagcctgcaggctgaagatgtggcagtttattactgtcaacaatattatactactccgtacacttttggccaggggaccaagctggagatcaaa

SEQ ID NO: 96 - protein, 113 aa, synthetic construct
  REGION 1..113: note = Synthetic
DIVMTQSPDSLAVSLGERATINCKSSQSVLYRSNNRNFLAWYQQKPGQPPKLLIYWASTRESGVPDRFSGSGSGTDFTLTISSLQAEDVAVYYCQQYYTTPYTFGQGTKLEIK

SEQ ID NO: 97 - DNA, 351 bp, synthetic construct
  misc_feature 1..351: note = Synthetic
  source 1..351: mol_type = other DNA
caggtgcagctggtgcagtctgggggaggcttggtacagcctggggggtccctgagactctcctgtgcagtctctggattcaccctcagtagctacgatatgcactgggtccgccaacctacaggaaaaggtctggagtgggtctcagctattggttctactggtgacacatactatccaggctccgtgaagggccgattcaccatctccagagaaaatgccaagaactccttgtatcttcaaatgaacagcctgagagccggggacacggctgtgtattactgtgcaagagagggatgggacgtaccctttgacttctggggccagggaaccctggtcaccgtctcctca

SEQ ID NO: 98 - protein, 117 aa, synthetic construct
  REGION 1..117: note = Synthetic
QVQLVQSGGGLVQPGGSLRLSCAVSGFTLSSYDMHWVRQPTGKGLEWVSAIGSTGDTYYPGSVKGRFTISRENAKNSLYLQMNSLRAGDTAVYYCAREGWDVPFDFWGQGTLVTVSS

SEQ ID NO: 99 - DNA, 24 bp, synthetic construct
  misc_feature 1..24: note = Synthetic
  source 1..24: mol_type = other DNA
ggattcaccctcagtagctacgat

SEQ ID NO: 100 - protein, 8 aa, synthetic construct
  REGION 1..8: note = Synthetic
GFTLSSYD

SEQ ID NO: 101 - DNA, 21 bp, synthetic construct
  misc_feature 1..21: note = Synthetic
  source 1..21: mol_type = other DNA
attggttctactggtgacaca

SEQ ID NO: 102 - protein, 7 aa, synthetic construct
  REGION 1..7: note = Synthetic
IGSTGDT

SEQ ID NO: 103 - DNA, 33 bp, synthetic construct
  misc_feature 1..33: note = Synthetic
  source 1..33: mol_type = other DNA
gcaagagagggatgggacgtaccctttgacttc

SEQ ID NO: 104 - protein, 11 aa, synthetic construct
  REGION 1..11: note = Synthetic
AREGWDVPFDF

SEQ ID NO: 105 - DNA, 324 bp, synthetic construct
  misc_feature 1..324: note = Synthetic
  source 1..324: mol_type = other DNA
gccatccagttgacccagtctccatcctccctgtctgcatctgtaggagacagagtcaccatcacttgccgggcaagtcaggacattagaaatgatttaggctggtatcagcagaaaccagggaaagcccctaagctcctgatctatgctgcatccagtttacaaagtggggtcccatcacggttcagcggcagtggatctggcacagatttcactctcaccatcagcagcctgcagcctgaagattttgcaacttattactgtctacaagattacaattacccgtggacgttcggccaagggaccaaggtggagatcaaacga

SEQ ID NO: 106 - protein, 108 aa, synthetic construct
  REGION 1..108: note = Synthetic
AIQLTQSPSSLSASVGDRVTITCRASQDIRNDLGWYQQKPGKAPKLLIYAASSLQSGVPSRFSGSGSGTDFTLTISSLQPEDFATYYCLQDYNYPWTFGQGTKVEIKR

SEQ ID NO: 107 - DNA, 18 bp, synthetic construct
  misc_feature 1..18: note = Synthetic
  source 1..18: mol_type = other DNA
caggacattagaaatgat

SEQ ID NO: 108 - protein, 6 aa, synthetic construct
  REGION 1..6: note = Synthetic
QDIRND

SEQ ID NO: 109-110 - skipped (2 entries)

SEQ ID NO: 111 - DNA, 27 bp, synthetic construct
  misc_feature 1..27: note = Synthetic
  source 1..27: mol_type = other DNA
ctacaagattacaattacccgtggacg

SEQ ID NO: 112 - protein, 9 aa, synthetic construct
  REGION 1..9: note = Synthetic
LQDYNYPWT

SEQ ID NO: 113 - DNA, 351 bp, synthetic construct
  misc_feature 1..351: note = Synthetic
  source 1..351: mol_type = other DNA
gaggtgcagctggtggagtctgggggaggcttggtacagcctggggggtccctgagactctcctgtgcagtctctggattcaccctcagtagctacgatatgcactgggtccgccaacctacaggaaaaggtctggagtgggtctcagctattggttctactggtgacacatactatccaggctccgtgaagggccgattcaccatctccagagaaaatgccaagaactccttgtatcttcaaatgaacagcctgagagccggggacacggctgtgtattactgtgcaagagagggatgggacgtaccctttgacttctggggccagggaaccctggtcaccgtctcctca

SEQ ID NO: 114 - protein, 117 aa, synthetic construct
  REGION 1..117: note = Synthetic
EVQLVESGGGLVQPGGSLRLSCAVSGFTLSSYDMHWVRQPTGKGLEWVSAIGSTGDTYYPGSVKGRFTISRENAKNSLYLQMNSLRAGDTAVYYCAREGWDVPFDFWGQGTLVTVSS

SEQ ID NO: 115 - DNA, 321 bp, synthetic construct
  misc_feature 1..321: note = Synthetic
  source 1..321: mol_type = other DNA
gccatccagatgacccagtctccatcctccctgtctgcatctgtaggagacagagtcaccatcacttgccgggcaagtcaggacattagaaatgatttaggctggtatcagcagaaaccagggaaagcccctaagctcctgatctatgctgcatccagtttacaaagtggggtcccatcacggttcagcggcagtggatctggcacagatttcactctcaccatcagcagcctgcagcctgaagattttgcaacttattactgtctacaagattacaattacccgtggacgttcggccaagggaccaaggtggaaatcaaa

SEQ ID NO: 116 - protein, 107 aa, synthetic construct
  REGION 1..107: note = Synthetic
AIQMTQSPSSLSASVGDRVTITCRASQDIRNDLGWYQQKPGKAPKLLIYAASSLQSGVPSRFSGSGSGTDFTLTISSLQPEDFATYYCLQDYNYPWTFGQGTKVEIK

SEQ ID NO: 117 - DNA, 351 bp, synthetic construct
  misc_feature 1..351: note = Synthetic
  source 1..351: mol_type = other DNA
gaggtgcagctggtggagtctgggggaggcttggtacagcctggggggtccctgagactctcctgtgcagcctctggattcaccctcagtagctacgatatgcactgggtccgccaagctacaggaaaaggtctggagtgggtctcagctattggttctactggtgacacatactatccaggctccgtgaagggccgattcaccatctccagagaaaatgccaagaactccttgtatcttcaaatgaacagcctgagagccggggacacggctgtgtattactgtgcaagagagggatgggacgtaccctttgacttctggggccagggaaccctggtcaccgtctcctca

SEQ ID NO: 118 - protein, 117 aa, synthetic construct
  REGION 1..117: note = Synthetic
EVQLVESGGGLVQPGGSLRLSCAASGFTLSSYDMHWVRQATGKGLEWVSAIGSTGDTYYPGSVKGRFTISRENAKNSLYLQMNSLRAGDTAVYYCAREGWDVPFDFWGQGTLVTVSS

SEQ ID NO: 119 - DNA, 321 bp, synthetic construct
  misc_feature 1..321: note = Synthetic
  source 1..321: mol_type = other DNA
gccatccagatgacccagtctccatcctccctgtctgcatctgtaggagacagagtcaccatcacttgccgggcaagtcaggacattagaaatgatttaggctggtatcagcagaaaccagggaaagcccctaagctcctgatctatgctgcatccagtttacaaagtggggtcccatcaaggttcagcggcagtggatctggcacagatttcactctcaccatcagcagcctgcagcctgaagattttgcaacttattactgtctacaagattacaattacccgtggacgttcggccaagggaccaaggtggaaatcaaa

SEQ ID NO: 120 - protein, 107 aa, synthetic construct; identical to SEQ ID NO: 116
  REGION 1..107: note = Synthetic

SEQ ID NO: 121 - DNA, 384 bp, synthetic construct
  misc_feature 1..384: note = Synthetic
  source 1..384: mol_type = other DNA
caggtgcagctgcaggagtcggggccaggactggtgaagccttcggagaccctgtccctcacctgcactgtctctggggactccatcaatacttactactggagctggttccggcagcccccagggaagggactggagtggattgggtatatctattatagtggaaccaccaactacaacccctccctcaagagtcgagtcaccatatcaatagacacgcccaggaaccagttctccctgaagctgatctctgtgaccgcagcggacacggccgtgtattactgtgcgagagagaggattactatgattcggggagttaccctctactattactcctacggtatggacgtctggggccaagggaccacggtcaccgtctcctca

SEQ ID NO: 122 - protein, 128 aa, synthetic construct
  REGION 1..128: note = Synthetic
QVQLQESGPGLVKPSETLSLTCTVSGDSINTYYWSWFRQPPGKGLEWIGYIYYSGTTNYNPSLKSRVTISIDTPRNQFSLKLISVTAADTAVYYCARERITMIRGVTLYYYSYGMDVWGQGTTVTVSS

SEQ ID NO: 123 - DNA, 24 bp, synthetic construct
  misc_feature 1..24: note = Synthetic
  source 1..24: mol_type = other DNA
ggggactccatcaatacttactac

SEQ ID NO: 124 - protein, 8 aa, synthetic construct
  REGION 1..8: note = Synthetic
GDSINTYY

SEQ ID NO: 125 - DNA, 21 bp, synthetic construct
  misc_feature 1..21: note = Synthetic
  source 1..21: mol_type = other DNA
atctattatagtggaaccacc

SEQ ID NO: 126 - protein, 7 aa, synthetic construct
  REGION 1..7: note = Synthetic
IYYSGTT

SEQ ID NO: 127 - DNA, 66 bp, synthetic construct
  misc_feature 1..66: note = Synthetic
  source 1..66: mol_type = other DNA
gcgagagagaggattactatgattcggggagttaccctctactattactcctacggtatggacgtc

SEQ ID NO: 128 - protein, 22 aa, synthetic construct
  REGION 1..22: note = Synthetic
ARERITMIRGVTLYYYSYGMDV

SEQ ID NO: 129 - DNA, 324 bp, synthetic construct
  misc_feature 1..324: note = Synthetic
  source 1..324: mol_type = other DNA
gacatccagatgacccagtctccatccttcctgtctgcatctgtaggagacagagtcaccatcacttgctgggccagtcaggacattagcagttatttagcctggtatcagcaaaaaccagggatagcccctaagctcctgatctatgctgcatccactttgcaaagtggggtcccatcaaggttcggcggcagtggatctgggacagaattcactctcacaatcagcagcctgcagcctgaagattttgcaacttattactgtcaacagcttaatagttaccctcggacgttcggccaagggaccaaggtggaaatcaaacga

SEQ ID NO: 130 - protein, 108 aa, synthetic construct
  REGION 1..108: note = Synthetic
DIQMTQSPSFLSASVGDRVTITCWASQDISSYLAWYQQKPGIAPKLLIYAASTLQSGVPSRFGGSGSGTEFTLTISSLQPEDFATYYCQQLNSYPRTFGQGTKVEIKR

SEQ ID NO: 131 - DNA, 18 bp, synthetic construct
  misc_feature 1..18: note = Synthetic
  source 1..18: mol_type = other DNA
caggacattagcagttat

SEQ ID NO: 132 - protein, 6 aa, synthetic construct
  REGION 1..6: note = Synthetic
QDISSY

SEQ ID NO: 133-134 - skipped (2 entries)

SEQ ID NO: 135 - DNA, 27 bp, synthetic construct
  misc_feature 1..27: note = Synthetic
  source 1..27: mol_type = other DNA
caacagcttaatagttaccctcggacg

SEQ ID NO: 136 - protein, 9 aa, synthetic construct
  REGION 1..9: note = Synthetic
QQLNSYPRT

SEQ ID NO: 137 - DNA, 384 bp, synthetic construct; identical to SEQ ID NO: 121
  misc_feature 1..384: note = Synthetic
  source 1..384: mol_type = other DNA

SEQ ID NO: 138 - protein, 128 aa, synthetic construct; identical to SEQ ID NO: 122
  REGION 1..128: note = Synthetic

SEQ ID NO: 139 - DNA, 321 bp, synthetic construct
  misc_feature 1..321: note = Synthetic
  source 1..321: mol_type = other DNA
gacatccagatgacccagtctccatccttcctgtctgcatctgtaggagacagagtcaccatcacttgctgggccagtcaggacattagcagttatttagcctggtatcagcaaaaaccagggatagcccctaagctcctgatctatgctgcatccactttgcaaagtggggtcccatcaaggttcggcggcagtggatctgggacagaattcactctcacaatcagcagcctgcagcctgaagattttgcaacttattactgtcaacagcttaatagttaccctcggacgttcggccaagggaccaaggtggaaatcaaa

SEQ ID NO: 140 - protein, 107 aa, synthetic construct
  REGION 1..107: note = Synthetic
DIQMTQSPSFLSASVGDRVTITCWASQDISSYLAWYQQKPGIAPKLLIYAASTLQSGVPSRFGGSGSGTEFTLTISSLQPEDFATYYCQQLNSYPRTFGQGTKVEIK

SEQ ID NO: 141 - DNA, 384 bp, synthetic construct
  misc_feature 1..384: note = Synthetic
  source 1..384: mol_type = other DNA
caggtgcagctgcaggagtcgggcccaggactggtgaagccttcggagaccctgtccctcacctgcactgtctctggggactccatcaatacttactactggagctggatccggcagcccccagggaagggactggagtggattgggtatatctattatagtggaaccaccaactacaacccctccctcaagagtcgagtcaccatatcagtagacacgtccaagaaccagttctccctgaagctgagctctgtgaccgctgcggacacggccgtgtattactgtgcgagagagaggattactatgattcggggagttaccctctactattactcctacggtatggacgtctggggccaagggaccacggtcaccgtctcctca

SEQ ID NO: 142 - protein, 128 aa, synthetic construct
  REGION 1..128: note = Synthetic
QVQLQESGPGLVKPSETLSLTCTVSGDSINTYYWSWIRQPPGKGLEWIGYIYYSGTTNYNPSLKSRVTISVDTSKNQFSLKLSSVTAADTAVYYCARERITMIRGVTLYYYSYGMDVWGQGTTVTVSS

SEQ ID NO: 143 - DNA, 321 bp, synthetic construct
  misc_feature 1..321: note = Synthetic
  source 1..321: mol_type = other DNA
gacatccagatgacccagtctccatcctccctgtctgcatctgtaggagacagagtcaccatcacttgccgggcaagtcaggacattagcagttatttaggctggtatcagcagaaaccagggaaagcccctaagcgcctgatctatgctgcatccagtttgcaaagtggggtcccatcaaggttcagcggcagtggatctgggacagaattcactctcacaatcagcagcctgcagcctgaagattttgcaacttattactgtcaacagcttaatagttaccctcggacgttcggccaagggaccaaggtggaaatcaaa

SEQ ID NO: 144 - protein, 107 aa, synthetic construct
  REGION 1..107: note = Synthetic
DIQMTQSPSSLSASVGDRVTITCRASQDISSYLGWYQQKPGKAPKRLIYAASSLQSGVPSRFSGSGSGTEFTLTISSLQPEDFATYYCQQLNSYPRTFGQGTKVEIK

SEQ ID NO: 145 - DNA, 378 bp, synthetic construct
  misc_feature 1..378: note = Synthetic
  source 1..378: mol_type = other DNA
caggtgcagctggtgcagtctggagctgaggtgaagaagcctggggcctcagtgaaggtctcctgcaaggcttctggttacacctttaccaactatggtatcagctgggtgcgacaggcccctggacaaggacttgagttaatgggatggattagtggttacaatggtaacacaaactatgcacaagaactccaggccagagtcaccatgaccacagacacatccacgagcacagcctacatggagctgaggaacctgagatctgacgacacggccgtatattactgtgcgagagatagagtcgttgtagcagctgctaattactacttttattctatggacgtctggggccaagggaccacggtcaccgtctcctca

SEQ ID NO: 146 - protein, 126 aa, synthetic construct
  REGION 1..126: note = Synthetic
QVQLVQSGAEVKKPGASVKVSCKASGYTFTNYGISWVRQAPGQGLELMGWISGYNGNTNYAQELQARVTMTTDTSTSTAYMELRNLRSDDTAVYYCARDRVVVAAANYYFYSMDVWGQGTTVTVSS

SEQ ID NO: 147 - DNA, 24 bp, synthetic construct
  misc_feature 1..24: note = Synthetic
  source 1..24: mol_type = other DNA
ggttacacctttaccaactatggt

SEQ ID NO: 148 - protein, 8 aa, synthetic construct
  REGION 1..8: note = Synthetic
GYTFTNYG

SEQ ID NO: 149 - DNA, 24 bp, synthetic construct
  misc_feature 1..24: note = Synthetic
  source 1..24: mol_type = other DNA
attagtggttacaatggtaacaca

SEQ ID NO: 150 - protein, 8 aa, synthetic construct
  REGION 1..8: note = Synthetic
ISGYNGNT

SEQ ID NO: 151 - DNA, 57 bp, synthetic construct
  misc_feature 1..57: note = Synthetic
  source 1..57: mol_type = other DNA
gcgagagatagagtcgttgtagcagctgctaattactacttttattctatggacgtc

SEQ ID NO: 152 - protein, 19 aa, synthetic construct
  REGION 1..19: note = Synthetic
ARDRVVVAAANYYFYSMDV

SEQ ID NO: 153 - DNA, 339 bp, synthetic construct
  misc_feature 1..339: note = Synthetic
  source 1..339: mol_type = other DNA
gccatccagatgacccagtctccactctccctgtccgtcacccttggacagccggcctccatctcctgcaggtctagtcaaagcctcgtatacagtgatggagacacctacttgaattggtttcagcagaggccaggccaatctccaaggcgcctaatttataaggtttctaaccgggactctggggtcccagacagattcagcggcagtgggtcaggcactgctttcacactgaaaatcagcggggtggaggccgaggatgttggggtttactactgcatgcaagctacacactggcctcggacgttcggccaagggaccaaggtggaaatcaaacga

SEQ ID NO: 154 - protein, 113 aa, synthetic construct
  REGION 1..113: note = Synthetic
AIQMTQSPLSLSVTLGQPASISCRSSQSLVYSDGDTYLNWFQQRPGQSPRRLIYKVSNRDSGVPDRFSGSGSGTAFTLKISGVEAEDVGVYYCMQATHWPRTFGQGTKVEIKR

SEQ ID NO: 155 - DNA, 33 bp, synthetic construct
  misc_feature 1..33: note = Synthetic
  source 1..33: mol_type = other DNA
caaagcctcgtatacagtgatggagacacctac

SEQ ID NO: 156 - protein, 11 aa, synthetic construct
  REGION 1..11: note = Synthetic
QSLVYSDGDTY

SEQ ID NO: 157-158 - skipped (2 entries)

SEQ ID NO: 159 - DNA, 27 bp, synthetic construct
  misc_feature 1..27: note = Synthetic
  source 1..27: mol_type = other DNA
atgcaagctacacactggcctcggacg

SEQ ID NO: 160 - protein, 9 aa, synthetic construct
  REGION 1..9: note = Synthetic
MQATHWPRT

SEQ ID NO: 161 - DNA, 378 bp, synthetic construct
  misc_feature 1..378: note = Synthetic
  source 1..378: mol_type = other DNA
caggttcagctggtgcagtctggagctgaggtgaagaagcctggggcctcagtgaaggtctcctgcaaggcttctggttacacctttaccaactatggtatcagctgggtgcgacaggcccctggacaaggacttgagttaatgggatggattagtggttacaatggtaacacaaactatgcacaagaactccaggccagagtcaccatgaccacagacacatccacgagcacagcctacatggagctgaggaacctgagatctgacgacacggccgtatattactgtgcgagagatagagtcgttgtagcagctgctaattactacttttattctatggacgtctggggccaagggaccacggtcaccgtctcctca

SEQ ID NO: 162 - protein, 126 aa, synthetic construct; identical to SEQ ID NO: 146
  REGION 1..126: note = Synthetic

SEQ ID NO: 163 - DNA, 336 bp, synthetic construct
  misc_feature 1..336: note = Synthetic
  source 1..336: mol_type = other DNA
gatgttgtgatgactcagtctccactctccctgtccgtcacccttggacagccggcctccatctcctgcaggtctagtcaaagcctcgtatacagtgatggagacacctacttgaattggtttcagcagaggccaggccaatctccaaggcgcctaatttataaggtttctaaccgggactctggggtcccagacagattcagcggcagtgggtcaggcactgctttcacactgaaaatcagcggggtggaggccgaggatgttggggtttactactgcatgcaagctacacactggcctcggacgttcggccaagggaccaaggtggaaatcaaa

SEQ ID NO: 164 - protein, 112 aa, synthetic construct
  REGION 1..112: note = Synthetic
DVVMTQSPLSLSVTLGQPASISCRSSQSLVYSDGDTYLNWFQQRPGQSPRRLIYKVSNRDSGVPDRFSGSGSGTAFTLKISGVEAEDVGVYYCMQATHWPRTFGQGTKVEIK

SEQ ID NO: 165 - DNA, 378 bp, synthetic construct
  misc_feature 1..378: note = Synthetic
  source 1..378: mol_type = other DNA
caggttcagctggtgcagtctggagctgaggtgaagaagcctggggcctcagtgaaggtctcctgcaaggcttctggttacacctttaccaactatggtatcagctgggtgcgacaggcccctggacaagggcttgagtggatgggatggattagtggttacaatggtaacacaaactatgcacagaagctccagggcagagtcaccatgaccacagacacatccacgagcacagcctacatggagctgaggagcctgagatctgacgacacggccgtgtattactgtgcgagagatagagtcgttgtagcagctgctaattactacttttattctatggacgtctggggccaagggaccacggtcaccgtctcctca

SEQ ID NO: 166 - protein, 126 aa, synthetic construct
  REGION 1..126: note = Synthetic
QVQLVQSGAEVKKPGASVKVSCKASGYTFTNYGISWVRQAPGQGLEWMGWISGYNGNTNYAQKLQGRVTMTTDTSTSTAYMELRSLRSDDTAVYYCARDRVVVAAANYYFYSMDVWGQGTTVTVSS

SEQ ID NO: 167 - DNA, 336 bp, synthetic construct
  misc_feature 1..336: note = Synthetic
  source 1..336: mol_type = other DNA
gatgttgtgatgactcagtctccactctccctgcccgtcacccttggacagccggcctccatctcctgcaggtctagtcaaagcctcgtatacagtgatggagacacctacttgaattggtttcagcagaggccaggccaatctccaaggcgcctaatttataaggtttctaaccgggactctggggtcccagacagattcagcggcagtgggtcaggcactgatttcacactgaaaatcagcagggtggaggctgaggatgttggggtttattactgcatgcaagctacacactggcctcggacgttcggccaagggaccaaggtggaaatcaaa

SEQ ID NO: 168 - protein, 112 aa, synthetic construct
  REGION 1..112: note = Synthetic
DVVMTQSPLSLPVTLGQPASISCRSSQSLVYSDGDTYLNWFQQRPGQSPRRLIYKVSNRDSGVPDRFSGSGSGTDFTLKISRVEAEDVGVYYCMQATHWPRTFGQGTKVEIK

SEQ ID NO: 169 - DNA, 375 bp, synthetic construct
  misc_feature 1..375: note = Synthetic
  source 1..375: mol_type = other DNA
caggtccacttgaaggagtctggtcctacgctggtgaaacccacacagaccctcacgctgacctgcaccttctctggattctcactcatcactagtggagtgggtgtgggctggattcgtcagccccccggaaaggccctggagtggcttgcactcatttattggaatggtgataagcgctacagcccatctctgaagagcaggctcaccatcaccaaggacacctccaaaaaccaggtggtccttacaatgaccaacatggaccctgtggacacagccacatattactgtgcacacaggataactgaaactagttactacttctactacggtatggacgtctggggccaagggaccacggtcaccgtctcctca

SEQ ID NO: 170 - protein, 125 aa, synthetic construct
  REGION 1..125: note = Synthetic
QVHLKESGPTLVKPTQTLTLTCTFSGFSLITSGVGVGWIRQPPGKALEWLALIYWNGDKRYSPSLKSRLTITKDTSKNQVVLTMTNMDPVDTATYYCAHRITETSYYFYYGMDVWGQGTTVTVSS

SEQ ID NO: 171 - DNA, 30 bp, synthetic construct
  misc_feature 1..30: note = Synthetic
  source 1..30: mol_type = other DNA
ggattctcactcatcactagtggagtgggt

SEQ ID NO: 172 - protein, 10 aa, synthetic construct
  REGION 1..10: note = Synthetic
GFSLITSGVG

SEQ ID NO: 173 - DNA, 21 bp, synthetic construct
  misc_feature 1..21: note = Synthetic
  source 1..21: mol_type = other DNA
atttattggaatggtgataag

SEQ ID NO: 174 - protein, 7 aa, synthetic construct
  REGION 1..7: note = Synthetic
IYWNGDK

SEQ ID NO: 175 - DNA, 51 bp, synthetic construct
  misc_feature 1..51: note = Synthetic
  source 1..51: mol_type = other DNA
gcacacaggataactgaaactagttactacttctactacggtatggacgtc

SEQ ID NO: 176 - protein, 17 aa, synthetic construct
  REGION 1..17: note = Synthetic
AHRITETSYYFYYGMDV

SEQ ID NO: 177 - DNA, 339 bp, synthetic construct
  misc_feature 1..339: note = Synthetic
  source 1..339: mol_type = other DNA
gacatccagatgacccagtctccactctccctgcccgtcacccctggagagccggcctccatctcctgcaggtctagtcagagcctcctgcatagtcatggatacgactatttggattggtacctgcagaagccagggcagtctccacagctcctgatctatttgggttctaatcgggcctccggggtccctgacaggttcagtggcagtggatcaggcacagattttacactgaaaatcagcagagtggaggctgaggatgttggggtttattactgcatgcaagctctacaaactccgctcactttcggcggagggaccaaggtggaaatcaaacga

SEQ ID NO: 178 - protein, 113 aa, synthetic construct
  REGION 1..113: note = Synthetic
DIQMTQSPLSLPVTPGEPASISCRSSQSLLHSHGYDYLDWYLQKPGQSPQLLIYLGSNRASGVPDRFSGSGSGTDFTLKISRVEAEDVGVYYCMQALQTPLTFGGGTKVEIKR

SEQ ID NO: 179 - DNA, 33 bp, synthetic construct
  misc_feature 1..33: note = Synthetic
  source 1..33: mol_type = other DNA
cagagcctcctgcatagtcatggatacgactat

SEQ ID NO: 180 - protein, 11 aa, synthetic construct
  REGION 1..11: note = Synthetic
QSLLHSHGYDY

SEQ ID NO: 181-182 - skipped (2 entries)

SEQ ID NO: 183 - DNA, 27 bp, synthetic construct
  misc_feature 1..27: note = Synthetic
  source 1..27: mol_type = other DNA
atgcaagctctacaaactccgctcact

SEQ ID NO: 184 - protein, 9 aa, synthetic construct
  REGION 1..9: note = Synthetic
MQALQTPLT

SEQ ID NO: 185 - DNA, 375 bp, synthetic construct
  misc_feature 1..375: note = Synthetic
  source 1..375: mol_type = other DNA
cagatcaccttgaaggagtctggtcctacgctggtgaaacccacacagaccctcacgctgacctgcaccttctctggattctcactcatcactagtggagtgggtgtgggctggattcgtcagccccccggaaaggccctggagtggcttgcactcatttattggaatggtgataagcgctacagcccatctctgaagagcaggctcaccatcaccaaggacacctccaaaaaccaggtggtccttacaatgaccaacatggaccctgtggacacagccacatattactgtgcacacaggataactgaaactagttactacttctactacggtatggacgtctggggccaagggaccacggtcaccgtctcctca

SEQ ID NO: 186 - protein, 125 aa, synthetic construct
  REGION 1..125: note = Synthetic
QITLKESGPTLVKPTQTLTLTCTFSGFSLITSGVGVGWIRQPPGKALEWLALIYWNGDKRYSPSLKSRLTITKDTSKNQVVLTMTNMDPVDTATYYCAHRITETSYYFYYGMDVWGQGTTVTVSS

SEQ ID NO: 187 - DNA, 336 bp, synthetic construct
  misc_feature 1..336: note = Synthetic
  source 1..336: mol_type = other DNA
gatattgtgatgactcagtctccactctccctgcccgtcacccctggagagccggcctccatctcctgcaggtctagtcagagcctcctgcatagtcatggatacgactatttggattggtacctgcagaagccagggcagtctccacagctcctgatctatttgggttctaatcgggcctccggggtccctgacaggttcagtggcagtggatcaggcacagattttacactgaaaatcagcagagtggaggctgaggatgttggggtttattactgcatgcaagctctacaaactccgctcactttcggcggagggaccaaggtggagatcaaa

SEQ ID NO: 188 - protein, 112 aa, synthetic construct
  REGION 1..112: note = Synthetic
DIVMTQSPLSLPVTPGEPASISCRSSQSLLHSHGYDYLDWYLQKPGQSPQLLIYLGSNRASGVPDRFSGSGSGTDFTLKISRVEAEDVGVYYCMQALQTPLTFGGGTKVEIK

SEQ ID NO: 189 - DNA, 375 bp, synthetic construct
  misc_feature 1..375: note = Synthetic
  source 1..375: mol_type = other DNA
cagatcaccttgaaggagtctggtcctacgctggtgaaacccacacagaccctcacgctgacctgcaccttctctggattctcactcatcactagtggagtgggtgtgggctggatccgtcagcccccaggaaaggccctggagtggcttgcactcatttattggaatggtgataagcgctacagcccatctctgaagagcaggctcaccatcaccaaggacacctccaaaaaccaggtggtccttacaatgaccaacatggaccctgtggacacagccacatattactgtgcacacaggataactgaaactagttactacttctactacggtatggacgtctggggccaagggaccacggtcaccgtctcctca

SEQ ID NO: 190 - protein, 125 aa, synthetic construct; identical to SEQ ID NO: 186
  REGION 1..125: note = Synthetic

SEQ ID NO: 191 - DNA, 336 bp, synthetic construct; identical to SEQ ID NO: 187
  misc_feature 1..336: note = Synthetic
  source 1..336: mol_type = other DNA

SEQ ID NO: 192 - protein, 112 aa, synthetic construct; identical to SEQ ID NO: 188
  REGION 1..112: note = Synthetic

SEQ ID NO: 193 - DNA, 375 bp, synthetic construct
  misc_feature 1..375: note = Synthetic
  source 1..375: mol_type = other DNA
cagatcaccttgaaggagtctggtcctactctggtgaaaccctcacagaccctcacgctgacctgcaccttctctgggttctcactcagcactagtggagtgggtgtgggctggatccgtcagcccccaggaaaggccctggagtggcttgcactcatttattggaattctgataagcgctacagcccatctctgaagagcaggctcaccatcaccaaggacacctccaaaaaccaggtagtccttacaatgaccaacatggaccctgtggacacagccacatattactgtgcacacagacatgacagctcgtcctactacttctactacggtatggacgtctggggccaagggatcacggtcaccgtctcctca

SEQ ID NO: 194 - protein, 125 aa, synthetic construct
  REGION 1..125: note = Synthetic
QITLKESGPTLVKPSQTLTLTCTFSGFSLSTSGVGVGWIRQPPGKALEWLALIYWNSDKRYSPSLKSRLTITKDTSKNQVVLTMTNMDPVDTATYYCAHRHDSSSYYFYYGMDVWGQGITVTVSS

SEQ ID NO: 195 - DNA, 30 bp, synthetic construct
  misc_feature 1..30: note = Synthetic
  source 1..30: mol_type = other DNA
gggttctcactcagcactagtggagtgggt

SEQ ID NO: 196 - protein, 10 aa, synthetic construct
  REGION 1..10: note = Synthetic
GFSLSTSGVG

SEQ ID NO: 197 - DNA, 21 bp, synthetic construct
  misc_feature 1..21: note = Synthetic
  source 1..21: mol_type = other DNA
atttattggaattctgataag

SEQ ID NO: 198 - protein, 7 aa, synthetic construct
  REGION 1..7: note = Synthetic
IYWNSDK

SEQ ID NO: 199 - DNA, 51 bp, synthetic construct
  misc_feature 1..51: note = Synthetic
  source 1..51: mol_type = other DNA
gcacacagacatgacagctcgtcctactacttctactacggtatggacgtc

SEQ ID NO: 200 - protein, 17 aa, synthetic construct
  REGION 1..17: note = Synthetic
AHRHDSSSYYFYYGMDV

SEQ ID NO: 201 - DNA, 339 bp, synthetic construct
  misc_feature 1..339: note = Synthetic
  source 1..339: mol_type = other DNA
gacatccagatgacccagtctccgctctccctgcccgtcacccctggagagccggcctccatctcctgcaggtctagtcagagcctcctccatagtcatggatacaactatttggattggtacctgcagaagccagggcagtctccacaactcctgatctatttgggttctaatcgggcctccggggtccctgacaggttcagtggcggtggatcaggcacagattttacactgaaaatcagcagagtggaggctgaggatgttgggatttattactgcatgcaagctctacagactcctctcactttcggcggagggaccaaggtggagatcaaacga

SEQ ID NO: 202 - protein, 113 aa, synthetic construct
  REGION 1..113: note = Synthetic
DIQMTQSPLSLPVTPGEPASISCRSSQSLLHSHGYNYLDWYLQKPGQSPQLLIYLGSNRASGVPDRFSGGGSGTDFTLKISRVEAEDVGIYYCMQALQTPLTFGGGTKVEIKR

SEQ ID NO: 203 - DNA, 33 bp, synthetic construct
  misc_feature 1..33: note = Synthetic
  source 1..33: mol_type = other DNA
cagagcctcctccatagtcatggatacaactat

SEQ ID NO: 204 - protein, 11 aa, synthetic construct
  REGION 1..11: note = Synthetic
QSLLHSHGYNY

SEQ ID NO: 205-206 - skipped (2 entries)

SEQ ID NO: 207 - DNA, 27 bp, synthetic construct
  misc_feature 1..27: note = Synthetic
  source 1..27: mol_type = other DNA
atgcaagctctacagactcctctcact

SEQ ID NO: 208 - protein, 9 aa, synthetic construct
  REGION 1..9: note = Synthetic
MQALQTPLT

SEQ ID NO: 209 - DNA, 375 bp, synthetic construct
  misc_feature 1..375: note = Synthetic
  source 1..375: mol_type = other DNA
cagatcaccttgaaggagtctggtcctactctggtgaaaccctcacagaccctcacgctgacctgcaccttctctgggttctcactcagcactagtggagtgggtgtgggctggatccgtcagcccccaggaaaggccctggagtggcttgcactcatttattggaattctgataagcgctacagcccatctctgaagagcaggctcaccatcaccaaggacacctccaaaaaccaggtagtccttacaatgaccaacatggaccctgtggacacagccacatattactgtgcacacagacatgacagctcgtcctactacttctactacggtatggacgtctggggccaagggaccacggtcaccgtctcctca

SEQ ID NO: 210 - protein, 125 aa, synthetic construct
  REGION 1..125: note = Synthetic
QITLKESGPTLVKPSQTLTLTCTFSGFSLSTSGVGVGWIRQPPGKALEWLALIYWNSDKRYSPSLKSRLTITKDTSKNQVVLTMTNMDPVDTATYYCAHRHDSSSYYFYYGMDVWGQGTTVTVSS

SEQ ID NO: 211 - DNA, 336 bp, synthetic construct
  misc_feature 1..336: note = Synthetic
  source 1..336: mol_type = other DNA
gatattgtgatgactcagtctccgctctccctgcccgtcacccctggagagccggcctccatctcctgcaggtctagtcagagcctcctccatagtcatggatacaactatttggattggtacctgcagaagccagggcagtctccacaactcctgatctatttgggttctaatcgggcctccggggtccctgacaggttcagtggcggtggatcaggcacagattttacactgaaaatcagcagagtggaggctgaggatgttgggatttattactgcatgcaagctctacagactcctctcactttcggcggagggaccaaggtggagatcaaa

SEQ ID NO: 212 - protein, 112 aa, synthetic construct
  REGION 1..112: note = Synthetic
DIVMTQSPLSLPVTPGEPASISCRSSQSLLHSHGYNYLDWYLQKPGQSPQLLIYLGSNRASGVPDRFSGGGSGTDFTLKISRVEAEDVGIYYCMQALQTPLTFGGGTKVEIK

SEQ ID NO: 213 - DNA, 375 bp, synthetic construct
  misc_feature 1..375: note = Synthetic
  source 1..375: mol_type = other DNA
cagatcaccttgaaggagtctggtcctacgctggtgaaacccacacagaccctcacgctgacctgcaccttctctgggttctcactcagcactagtggagtgggtgtgggctggatccgtcagcccccaggaaaggccctggagtggcttgcactcatttattggaattctgataagcgctacagcccatctctgaagagcaggctcaccatcaccaaggacacctccaaaaaccaggtggtccttacaatgaccaacatggaccctgtggacacagccacatattactgtgcacacagacatgacagctcgtcctactacttctactacggtatggacgtctggggccaagggaccacggtcaccgtctcctca

SEQ ID NO: 214 - protein, 125 aa, synthetic construct
  REGION 1..125: note = Synthetic
QITLKESGPTLVKPTQTLTLTCTFSGFSLSTSGVGVGWIRQPPGKALEWLALIYWNSDKRYSPSLKSRLTITKDTSKNQVVLTMTNMDPVDTATYYCAHRHDSSSYYFYYGMDVWGQGTTVTVSS

SEQ ID NO: 215 - DNA, 336 bp, synthetic construct
  misc_feature 1..336: note = Synthetic
  source 1..336: mol_type = other DNA
gatattgtgatgactcagtctccactctccctgcccgtcacccctggagagccggcctccatctcctgcaggtctagtcagagcctcctccatagtcatggatacaactatttggattggtacctgcagaagccagggcagtctccacagctcctgatctatttgggttctaatcgggcctccggggtccctgacaggttcagtggcagtggatcaggcacagattttacactgaaaatcagcagagtggaggctgaggatgttggggtttattactgcatgcaagctctacagactcctctcactttcggcggagggaccaaggtggagatcaaa

SEQ ID NO: 216 - protein, 112 aa, synthetic construct
  REGION 1..112: note = Synthetic
DIVMTQSPLSLPVTPGEPASISCRSSQSLLHSHGYNYLDWYLQKPGQSPQLLIYLGSNRASGVPDRFSGSGSGTDFTLKISRVEAEDVGVYYCMQALQTPLTFGGGTKVEIK

SEQ ID NO: 217 - DNA, 381 bp, synthetic construct
  misc_feature 1..381: note = Synthetic
  source 1..381: mol_type = other DNA
gagatgcaactggtggagtctgggggaggcttggtccagcctggggggtccctgagactctcctgtgcagcctctggattcacctttagtagtcactggatgaagtgggtccgccaggctccagggaaggggctggagtgggtggccaacataaaccaagatggaagtgagaaatactatgtggactctgtgaagggccgattcaccatctccagagacaacgccaagaactcactgtttctgcaaatgaacagcctgagagccgaggacacggctgtgtattactgtgcgagagatattgtactaatggtctatgatatggactactactactacggtatggacgtctggggccaagggaccacggtcaccgtctcctca

SEQ ID NO: 218 - protein, 127 aa, synthetic construct
  REGION 1..127: note = Synthetic
EMQLVESGGGLVQPGGSLRLSCAASGFTFSSHWMKWVRQAPGKGLEWVANINQDGSEKYYVDSVKGRFTISRDNAKNSLFLQMNSLRAEDTAVYYCARDIVLMVYDMDYYYYGMDVWGQGTTVTVSS

SEQ ID NO: 219 - DNA, 24 bp, synthetic construct
  misc_feature 1..24: note = Synthetic
  source 1..24: mol_type = other DNA
ggattcacctttagtagtcactgg

SEQ ID NO: 220 - protein, 8 aa, synthetic construct
  REGION 1..8: note = Synthetic
GFTFSSHW

SEQ ID NO: 221 - DNA, 24 bp, synthetic construct
  misc_feature 1..24: note = Synthetic
  source 1..24: mol_type = other DNA
ataaaccaagatggaagtgagaaa

SEQ ID NO: 222 - protein, 8 aa, synthetic construct
  REGION 1..8: note = Synthetic
INQDGSEK

SEQ ID NO: 223 - DNA, 60 bp, synthetic construct
  misc_feature 1..60: note = Synthetic
  source 1..60: mol_type = other DNA
gcgagagatattgtactaatggtctatgatatggactactactactacggtatggacgtc

SEQ ID NO: 224 - protein, 20 aa, synthetic construct
  REGION 1..20: note = Synthetic
ARDIVLMVYDMDYYYYGMDV

SEQ ID NO: 225 - DNA, 336 bp, synthetic construct
  misc_feature 1..336: note = Synthetic
  source 1..336: mol_type = other DNA
gatattgtgatgactcagtctccactctccctgcccgtcacccctggagagccggcctccatctcctgcaggtctagtcagagcctcctgcatagtaatggaaacaactatttggattggtacctgcagaagccagggcagtctccacagctcctgatctatttgggttctaatcgggcctccggggtccctgacaggttcagtggcagtggatcaggcacagattttacactgaaaatcagcagagtggaggctgaggatgttggggtttattactgcatgcaaactctacaaactccgctcactttcggcggagggaccaaggtggagatcaaa

SEQ ID NO: 226 - protein, 112 aa, synthetic construct
  REGION 1..112: note = Synthetic
DIVMTQSPLSLPVTPGEPASISCRSSQSLLHSNGNNYLDWYLQKPGQSPQLLIYLGSNRASGVPDRFSGSGSGTDFTLKISRVEAEDVGVYYCMQTLQTPLTFGGGTKVEIK

SEQ ID NO: 227 - DNA, 33 bp, synthetic construct
  misc_feature 1..33: note = Synthetic
  source 1..33: mol_type = other DNA
cagagcctcctgcatagtaatggaaacaactat

SEQ ID NO: 228 - protein, 11 aa, synthetic construct
  REGION 1..11: note = Synthetic
QSLLHSNGNNY

SEQ ID NO: 229-230 - skipped (2 entries)

SEQ ID NO: 231 - DNA, 27 bp, synthetic construct
  misc_feature 1..27: note = Synthetic
  source 1..27: mol_type = other DNA
atgcaaactctacaaactccgctcact

SEQ ID NO: 232 - protein, 9 aa, synthetic construct
  REGION 1..9: note = Synthetic
MQTLQTPLT

SEQ ID NO: 233 - DNA, 381 bp, synthetic construct
  misc_feature 1..381: note = Synthetic
  source 1..381: mol_type = other DNA
gaggtgcagctggtggagtctgggggaggcttggtccagcctggggggtccctgagactctcctgtgcagcctctggattcacctttagtagtcactggatgaagtgggtccgccaggctccagggaaggggctggagtgggtggccaacataaaccaagatggaagtgagaaatactatgtggactctgtgaagggccgattcaccatctccagagacaacgccaagaactcactgtttctgcaaatgaacagcctgagagccgaggacacggctgtgtattactgtgcgagagatattgtactaatggtctatgatatggactactactactacggtatggacgtctggggccaagggaccacggtcaccgtctcctca

SEQ ID NO: 234 - protein, 127 aa, synthetic construct
  REGION 1..127: note = Synthetic
EVQLVESGGGLVQPGGSLRLSCAASGFTFSSHWMKWVRQAPGKGLEWVANINQDGSEKYYVDSVKGRFTISRDNAKNSLFLQMNSLRAEDTAVYYCARDIVLMVYDMDYYYYGMDVWGQGTTVTVSS

SEQ ID NO: 235 - DNA, 336 bp, synthetic construct; identical to SEQ ID NO: 225
  misc_feature 1..336: note = Synthetic
  source 1..336: mol_type = other DNA

SEQ ID NO: 236 - protein, 112 aa, synthetic construct; identical to SEQ ID NO: 226
  REGION 1..112: note = Synthetic

SEQ ID NO: 237 - DNA, 381 bp, synthetic construct
  misc_feature 1..381: note = Synthetic
  source 1..381: mol_type = other DNA
gaggtgcagctggtggagtctgggggaggcttggtccagcctggggggtccctgagactctcctgtgcagcctctggattcacctttagtagtcactggatgagctgggtccgccaggctccagggaaggggctggagtgggtggccaacataaaccaagatggaagtgagaaatactatgtggactctgtgaagggccgattcaccatctccagagacaacgccaagaactcactgtatctgcaaatgaacagcctgagagccgaggacacggctgtgtattactgtgcgagagatattgtactaatggtctatgatatggactactactactacggtatggacgtctgggggcaagggaccacggtcaccgtctcctca

SEQ ID NO: 238 - protein, 127 aa, synthetic construct
  REGION 1..127: note = Synthetic
EVQLVESGGGLVQPGGSLRLSCAASGFTFSSHWMSWVRQAPGKGLEWVANINQDGSEKYYVDSVKGRFTISRDNAKNSLYLQMNSLRAEDTAVYYCARDIVLMVYDMDYYYYGMDVWGQGTTVTVSS

SEQ ID NO: 239 - DNA, 336 bp, synthetic construct; identical to SEQ ID NO: 225
  misc_feature 1..336: note = Synthetic
  source 1..336: mol_type = other DNA

SEQ ID NO: 240 - protein, 112 aa, synthetic construct; identical to SEQ ID NO: 226
  REGION 1..112: note = Synthetic

SEQ ID NO: 241 - DNA, 381 bp, synthetic construct
  misc_feature 1..381: note = Synthetic
  source 1..381: mol_type = other DNA
caggtgcagctggtggagtctgggggaggcgtggtccagcctgggaggtccctgagactctcctgtgcagtctctggattcaccttcagtagctatggcatgcactgggtccgccaggctccaggcaaggggctggagtgggtggcagctatatcatatgatggaagtaataaatactatgtagactccgtgaagggccgattcaccatctccagagacaattccaagaaaacgctgtatctgcaaatgaacagcctgagagctgaggacacggctgtgtataattgtgcgaaaaatattgtactagtgatgtatgatatagactatcactactatgggatggacgtctggggccaagggaccacggtcaccgtctcctca

SEQ ID NO: 242 - protein, 127 aa, synthetic construct
  REGION 1..127: note = Synthetic
QVQLVESGGGVVQPGRSLRLSCAVSGFTFSSYGMHWVRQAPGKGLEWVAAISYDGSNKYYVDSVKGRFTISRDNSKKTLYLQMNSLRAEDTAVYNCAKNIVLVMYDIDYHYYGMDVWGQGTTVTVSS

SEQ ID NO: 243 - DNA, 24 bp, synthetic construct
  misc_feature 1..24: note = Synthetic
  source 1..24: mol_type = other DNA
ggattcaccttcagtagctatggc

SEQ ID NO: 244 - protein, 8 aa, synthetic construct
  REGION 1..8: note = Synthetic
GFTFSSYG

SEQ ID NO: 245 - DNA, 24 bp, synthetic construct
  misc_feature 1..24: note = Synthetic
  source 1..24: mol_type = other DNA
atatcatatgatggaagtaataaa

SEQ ID NO: 246 - protein, 8 aa, synthetic construct
  REGION 1..8: note = Synthetic
ISYDGSNK

SEQ ID NO: 247 - DNA, 60 bp, synthetic construct
  misc_feature 1..60: note = Synthetic
  source 1..60: mol_type = other DNA
gcgaaaaatattgtactagtgatgtatgatatagactatcactactatgggatggacgtc

SEQ ID NO: 248 - protein, 20 aa, synthetic construct
  REGION 1..20: note = Synthetic
AKNIVLVMYDIDYHYYGMDV

SEQ ID NO: 249 - DNA, 336 bp, synthetic construct
  misc_feature 1..336: note = Synthetic
  source 1..336: mol_type = other DNA
gatattgtgatgactcagtctccactctccctgcccgtcacccctggagagccggcctccatctcctgcaggtctagtcagagcctcctgcatagtaatggatacaactatttggattggtacctgcagaagccagggcagtctccacaactcctgatctatttgggttttaatcgggcctccggggtccctgacaggttcagtggcagtggatcaggcacagattttacactgaaaatcagcagagtggaggctgaggatgttggggtttattactgcatgcaagctctacaaactcctctcactttcggcggagggaccaaggtggagatcaga

SEQ ID NO: 250 - protein, 112 aa, synthetic construct
  REGION 1..112: note = Synthetic
DIVMTQSPLSLPVTPGEPASISCRSSQSLLHSNGYNYLDWYLQKPGQSPQLLIYLGFNRASGVPDRFSGSGSGTDFTLKISRVEAEDVGVYYCMQALQTPLTFGGGTKVEIR

SEQ ID NO: 251 - DNA, 33 bp, synthetic construct
  misc_feature 1..33: note = Synthetic
  source 1..33: mol_type = other DNA
cagagcctcctgcatagtaatggatacaactat

SEQ ID NO: 252 - protein, 11 aa, synthetic construct
  REGION 1..11: note = Synthetic
QSLLHSNGYNY

SEQ ID NO: 253-254 - skipped (2 entries)

SEQ ID NO: 255 - DNA, 27 bp, synthetic construct
  misc_feature 1..27: note = Synthetic
  source 1..27: mol_type = other DNA
atgcaagctctacaaactcctctcact

SEQ ID NO: 256 - protein, 9 aa, synthetic construct
  REGION 1..9: note = Synthetic
MQALQTPLT

SEQ ID NO: 257 - DNA, 381 bp, synthetic construct; identical to SEQ ID NO: 241
  misc_feature 1..381: note = Synthetic
  source 1..381: mol_type = other DNA

SEQ ID NO: 258 - protein, 127 aa, synthetic construct; identical to SEQ ID NO: 242
  REGION 1..127: note = Synthetic

SEQ ID NO: 259 - DNA, 336 bp, synthetic construct
  misc_feature 1..336: note = Synthetic
  source 1..336: mol_type = other DNA
gatattgtgatgactcagtctccactctccctgcccgtcacccctggagagccggcctccatctcctgcaggtctagtcagagcctcctgcatagtaatggatacaactatttggattggtacctgcagaagccagggcagtctccacaactcctgatctatttgggttttaatcgggcctccggggtccctgacaggttcagtggcagtggatcaggcacagattttacactgaaaatcagcagagtggaggctgaggatgttggggtttattactgcatgcaagctctacaaactcctctcactttcggcggagggaccaaggtggagatcaaa

SEQ ID NO: 260 - protein, 112 aa, synthetic construct
  REGION 1..112: note = Synthetic
DIVMTQSPLSLPVTPGEPASISCRSSQSLLHSNGYNYLDWYLQKPGQSPQLLIYLGFNRASGVPDRFSGSGSGTDFTLKISRVEAEDVGVYYCMQALQTPLTFGGGTKVEIK

SEQ ID NO: 261 - DNA, 381 bp, synthetic construct
  misc_feature 1..381: note = Synthetic
  source 1..381: mol_type = other DNA
caggtgcagctggtggagtctgggggaggcgtggtccagcctgggaggtccctgagactctcctgtgcagcctctggattcaccttcagtagctatggcatgcactgggtccgccaggctccaggcaaggggctggagtgggtggcagttatatcatatgatggaagtaataaatactatgcagactccgtgaagggccgattcaccatctccagagacaattccaagaacacgctgtatctgcaaatgaacagcctgagagctgaggacacggctgtgtattactgtgcgaaaaatattgtactagtgatgtatgatatagactatcactactatgggatggacgtctgggggcaagggaccacggtcaccgtctcctca

SEQ ID NO: 262 - protein, 127 aa, synthetic construct
  REGION 1..127: note = Synthetic
QVQLVESGGGVVQPGRSLRLSCAASGFTFSSYGMHWVRQAPGKGLEWVAVISYDGSNKYYADSVKGRFTISRDNSKNTLYLQMNSLRAEDTAVYYCAKNIVLVMYDIDYHYYGMDVWGQGTTVTVSS

SEQ ID NO: 263 - DNA, 336 bp, synthetic construct
  misc_feature 1..336: note = Synthetic
  source 1..336: mol_type = other DNA
gatattgtgatgactcagtctccactctccctgcccgtcacccctggagagccggcctccatctcctgcaggtctagtcagagcctcctgcatagtaatggatacaactatttggattggtacctgcagaagccagggcagtctccacagctcctgatctatttgggttttaatcgggcctccggggtccctgacaggttcagtggcagtggatcaggcacagattttacactgaaaatcagcagagtggaggctgaggatgttggggtttattactgcatgcaagctctacaaactcctctcactttcggcggagggaccaaggtggagatcaaa

SEQ ID NO: 264 - protein, 112 aa, synthetic construct; identical to SEQ ID NO: 260
  REGION 1..112: note = Synthetic

SEQ ID NO: 265 - DNA, 381 bp, synthetic construct; identical to SEQ ID NO: 241
  misc_feature 1..381: note = Synthetic
  source 1..381: mol_type = other DNA

SEQ ID NO: 266 - protein, 127 aa, synthetic construct; identical to SEQ ID NO: 242
  REGION 1..127: note = Synthetic

SEQ ID NO: 267 - DNA, 24 bp, synthetic construct
  misc_feature 1..24: note = Synthetic
  source 1..24: mol_type = other DNA
ggattcaccttcagtagctatggc

SEQ ID NO: 268 - protein, 8 aa, synthetic construct
  REGION 1..8: note = Synthetic
GFTFSSYG

SEQ ID NO: 269 - DNA, 24 bp, synthetic construct
  misc_feature 1..24: note = Synthetic
  source 1..24: mol_type = other DNA
atatcatatgatggaagtaataaa

SEQ ID NO: 270 - protein, 8 aa, synthetic construct
  REGION 1..8: note = Synthetic
ISYDGSNK

SEQ ID NO: 271 - DNA, 60 bp, synthetic construct; identical to SEQ ID NO: 247
  misc_feature 1..60: note = Synthetic
  source 1..60: mol_type = other DNA

SEQ ID NO: 272 - protein, 20 aa, synthetic construct
  REGION 1..20: note = Synthetic
AKNIVLVMYDIDYHYYGMDV

SEQ ID NO: 273 - DNA, 336 bp, synthetic construct; identical to SEQ ID NO: 249
  misc_feature 1..336: note = Synthetic
  source 1..336: mol_type = other DNA

SEQ ID NO: 274 - protein, 112 aa, synthetic construct; identical to SEQ ID NO: 250
  REGION 1..112: note = Synthetic

SEQ ID NO: 275 - DNA, 33 bp, synthetic construct; identical to SEQ ID NO: 251
  misc_feature 1..33: note = Synthetic
  source 1..33: mol_type = other DNA

SEQ ID NO: 276 - protein, 11 aa, synthetic construct
  REGION 1..11: note = Synthetic
QSLLHSNGYNY

SEQ ID NO: 277-278 - skipped (2 entries)

SEQ ID NO: 279 - DNA, 27 bp, synthetic construct
  misc_feature 1..27: note = Synthetic
  source 1..27: mol_type = other DNA
atgcaagctctacaaactcctctcact

SEQ ID NO: 280 - protein, 9 aa, synthetic construct
  REGION 1..9: note = Synthetic
MQALQTPLT

SEQ ID NO: 281 - DNA, 381 bp, synthetic construct; identical to SEQ ID NO: 241
  misc_feature 1..381: note = Synthetic
  source 1..381: mol_type = other DNA

SEQ ID NO: 282 - protein, 127 aa, synthetic construct; identical to SEQ ID NO: 242
  REGION 1..127: note = Synthetic

SEQ ID NO: 283 - DNA, 336 bp, synthetic construct; identical to SEQ ID NO: 259
  misc_feature 1..336: note = Synthetic
  source 1..336: mol_type = other DNA

SEQ ID NO: 284 - protein, 112 aa, synthetic construct; identical to SEQ ID NO: 260
  REGION 1..112: note = Synthetic

SEQ ID NO: 285 - DNA, 381 bp, synthetic construct; identical to SEQ ID NO: 261
  misc_feature 1..381: note = Synthetic
  source 1..381: mol_type = other DNA

SEQ ID NO: 286 - protein, 127 aa, synthetic construct; identical to SEQ ID NO: 262
  REGION 1..127: note = Synthetic

SEQ ID NO: 287 - DNA, 336 bp, synthetic construct; identical to SEQ ID NO: 263
  misc_feature 1..336: note = Synthetic
  source 1..336: mol_type = other DNA

SEQ ID NO: 288 - protein, 112 aa, synthetic construct; identical to SEQ ID NO: 260
  REGION 1..112: note = Synthetic

SEQ ID NO: 289 - DNA, 372 bp, synthetic construct
  misc_feature 1..372: note = Synthetic
  source 1..372: mol_type = other DNA
cagatcaccttgaaggagtctggtcctacgctggtaaaacccacacagaccctcacgctgacctgcaccttctctgggttctcactcagcgctagtggagtgggtgtgggctggttccgtcagcccccaggaaaggccctggagtggcttgcactcatttattggaatgatgataagcgttacagcccatctctaaagaacagcctcaccatcaccaaggacacctccaaaaaccaggtggtccttacaatgaccaacatggaccctgtggacacagccacatattactgtgcacacagaatacatctatggtcctacttctactacggtatggacgtctggggccaagggaccacggtcaccgtctcctca

SEQ ID NO: 290 - protein, 124 aa, synthetic construct
  REGION 1..124: note = Synthetic
QITLKESGPTLVKPTQTLTLTCTFSGFSLSASGVGVGWFRQPPGKALEWLALIYWNDDKRYSPSLKNSLTITKDTSKNQVVLTMTNMDPVDTATYYCAHRIHLWSYFYYGMDVWGQGTTVTVSS

SEQ ID NO: 291 - DNA, 30 bp, synthetic construct
  misc_feature 1..30: note = Synthetic
  source 1..30: mol_type = other DNA
gggttctcactcagcgctagtggagtgggt

SEQ ID NO: 292 - protein, 10 aa, synthetic construct
  REGION 1..10: note = Synthetic
GFSLSASGVG

SEQ ID NO: 293 - DNA, 21 bp, synthetic construct
  misc_feature 1..21: note = Synthetic
  source 1..21: mol_type = other DNA
atttattggaatgatgataag

SEQ ID NO: 294 - protein, 7 aa, synthetic construct
  REGION 1..7: note = Synthetic
IYWNDDK

SEQ ID NO: 295 - DNA, 48 bp, synthetic construct
  misc_feature 1..48: note = Synthetic
  source 1..48: mol_type = other DNA
gcacacagaatacatctatggtcctacttctactacggtatggacgtc

SEQ ID NO: 296 - protein, 16 aa, synthetic construct
  REGION 1..16: note = Synthetic
AHRIHLWSYFYYGMDV

SEQ ID NO: 297 - DNA, 336 bp, synthetic construct
  misc_feature 1..336: note = Synthetic
  source 1..336: mol_type = other DNA
gatattgtgatgactcagtctccactctccctgcccgtcacccctggagagccggcctccatctcctgcaggtctagtcagactctcctgcatagtaatggatacaactatttcgattggtacctgcagaagccagggcagtctccacagctcctgatctatttgggttctaatcgggcctccggggtccctgacagattcagtggcagtggatcaggcacagattttacactgaaaatcagcagagtggaggctgaggatgttggaatttattactgcatgcaagctctacaaactcctctcactttcggcggagggaccaaggtggagatcaga

SEQ ID NO: 298 - protein, 112 aa, synthetic construct
  REGION 1..112: note = Synthetic
DIVMTQSPLSLPVTPGEPASISCRSSQTLLHSNGYNYFDWYLQKPGQSPQLLIYLGSNRASGVPDRFSGSGSGTDFTLKISRVEAEDVGIYYCMQALQTPLTFGGGTKVEIR

SEQ ID NO: 299 - DNA, 33 bp, synthetic construct
  misc_feature 1..33: note = Synthetic
  source 1..33: mol_type = other DNA
cagactctcctgcatagtaatggatacaactat

SEQ ID NO: 300 - protein, 11 aa, synthetic construct
  REGION 1..11: note = Synthetic
QTLLHSNGYNY

SEQ ID NO: 301-302 - skipped (2 entries)

SEQ ID NO: 303 - DNA, 27 bp, synthetic construct
  misc_feature 1..27: note = Synthetic
  source 1..27: mol_type = other DNA
atgcaagctctacaaactcctctcact

SEQ ID NO: 304 - protein, 9 aa, synthetic construct
  REGION 1..9: note = Synthetic
MQALQTPLT

SEQ ID NO: 305 - DNA, 372 bp, synthetic construct; identical to SEQ ID NO: 289
  misc_feature 1..372: note = Synthetic
  source 1..372: mol_type = other DNA

SEQ ID NO: 306 - protein, 124 aa, synthetic construct; identical to SEQ ID NO: 290
  REGION 1..124: note = Synthetic

SEQ ID NO: 307 - DNA, 336 bp, synthetic construct
  misc_feature 1..336: note = Synthetic
  source 1..336: mol_type = other DNA
gatattgtgatgactcagtctccactctccctgcccgtcacccctggagagccggcctccatctcctgcaggtctagtcagactctcctgcatagtaatggatacaactatttcgattggtacctgcagaagccagggcagtctccacagctcctgatctatttgggttctaatcgggcctccggggtccctgacagattcagtggcagtggatcaggcacagattttacactgaaaatcagcagagtggaggctgaggatgttggaatttattactgcatgcaagctctacaaactcctctcactttcggcggagggaccaaggtggagatcaaa

SEQ ID NO: 308 - protein, 112 aa, synthetic construct
  REGION 1..112: note = Synthetic
DIVMTQSPLSLPVTPGEPASISCRSSQTLLHSNGYNYFDWYLQKPGQSPQLLIYLGSNRASGVPDRFSGSGSGTDFTLKISRVEAEDVGIYYCMQALQTPLTFGGGTKVEIK

SEQ ID NO: 309 - DNA, 372 bp, synthetic construct
  misc_feature 1..372: note = Synthetic
  source 1..372: mol_type = other DNA
cagatcaccttgaaggagtctggtcctacgctggtgaaacccacacagaccctcacgctgacctgcaccttctctgggttctcactcagcgctagtggagtgggtgtgggctggatccgtcagcccccaggaaaggccctggagtggcttgcactcatttattggaatgatgataagcgctacagcccatctctgaagagcaggctcaccatcaccaaggacacctccaaaaaccaggtggtccttacaatgaccaacatggaccctgtggacacagccacatattactgtgcacacagaatacatctatggtcctacttctactacggtatggacgtctgggggcaagggaccacggtcaccgtctcctca

SEQ ID NO: 310 - protein, 124 aa, synthetic construct
  REGION 1..124: note = Synthetic
QITLKESGPTLVKPTQTLTLTCTFSGFSLSASGVGVGWIRQPPGKALEWLALIYWNDDKRYSPSLKSRLTITKDTSKNQVVLTMTNMDPVDTATYYCAHRIHLWSYFYYGMDVWGQGTTVTVSS

SEQ ID NO: 311 - DNA, 336 bp, synthetic construct
  misc_feature 1..336: note = Synthetic
  source 1..336: mol_type = other DNA
gatattgtgatgactcagtctccactctccctgcccgtcacccctggagagccggcctccatctcctgcaggtctagtcagactctcctgcatagtaatggatacaactatttggattggtacctgcagaagccagggcagtctccacagctcctgatctatttgggttctaatcgggcctccggggtccctgacaggttcagtggcagtggatcaggcacagattttacactgaaaatcagcagagtggaggctgaggatgttggggtttattactgcatgcaagctctacaaactcctctcactttcggcggagggaccaaggtggagatcaaa

SEQ ID NO: 312 - protein, 112 aa, synthetic construct
  REGION 1..112: note = Synthetic
DIVMTQSPLSLPVTPGEPASISCRSSQTLLHSNGYNYLDWYLQKPGQSPQLLIYLGSNRASGVPDRFSGSGSGTDFTLKISRVEAEDVGVYYCMQALQTPLTFGGGTKVEIK

SEQ ID NO: 313 - DNA, 381 bp, synthetic construct
  misc_feature 1..381: note = Synthetic
  source 1..381: mol_type = other DNA
caggttcagctggtgcagtctggacctgaggtgaagaaccctggggcctcagtgaaggtctcctgcaaggcttctggttacacctttaccacctatggtatcagttgggtacgacaggcccctggacaagggcttgagtggatgggatggatcagcggttacaatggtaaaacaaacgatgcacagaagttccaggacagagtcgccatgaccacagacacatccacgagcacagcctacatggagctgaggagcctgagatctgacgacacggccatttattactgttcgagagatcgtttagtagtaccacctgcccttaattattcctactacgttatggacgtctggggccaagggaccacggtcaccgtctcctca

SEQ ID NO: 314 - protein, 127 aa, synthetic construct
  REGION 1..127: note = Synthetic
QVQLVQSGPEVKNPGASVKVSCKASGYTFTTYGISWVRQAPGQGLEWMGWISGYNGKTNDAQKFQDRVAMTTDTSTSTAYMELRSLRSDDTAIYYCSRDRLVVPPALNYSYYVMDVWGQGTTVTVSS

SEQ ID NO: 315 - DNA, 24 bp, synthetic construct
  misc_feature 1..24: note = Synthetic
  source 1..24: mol_type = other DNA
ggttacacctttaccacctatggt

SEQ ID NO: 316 - protein, 8 aa, synthetic construct
  REGION 1..8: note = Synthetic
GYTFTTYG

SEQ ID NO: 317 - DNA, 24 bp, synthetic construct
  misc_feature 1..24: note = Synthetic
  source 1..24: mol_type = other DNA
atcagcggttacaatggtaaaaca

SEQ ID NO: 318 - protein, 8 aa, synthetic construct
  REGION 1..8: note = Synthetic
ISGYNGKT

SEQ ID NO: 319 - DNA, 60 bp, synthetic construct
  misc_feature 1..60: note = Synthetic
  source 1..60: mol_type = other DNA
tcgagagatcgtttagtagtaccacctgcccttaattattcctactacgttatggacgtc

SEQ ID NO: 320 - protein, 20 aa, synthetic construct
  REGION 1..20: note = Synthetic
SRDRLVVPPALNYSYYVMDV

SEQ ID NO: 321 - DNA, 336 bp, synthetic construct
  misc_feature 1..336: note = Synthetic
  source 1..336: mol_type = other DNA
gatgttgtgatgactcagtctccactctccctgcccgtcacccttggacagccggcctccatctcctgcaggtctagtcaaagcctcgtatacagtgatggaaacacctacttgaattggtctcagcagaggccaggtcaatctccaaggcgcctaatttataaggtttctaaccgggactctggggtcccagacagattcagcggcagtgggtcaggcactgatttcacactgaaaatcagcagggtggaggctgaggatgttggggtttattactgcatgcaaggtacacactggccgtacacttttggccaggggaccaagctggagatcaaa

SEQ ID NO: 322 - protein, 112 aa, synthetic construct
  REGION 1..112: note = Synthetic
DVVMTQSPLSLPVTLGQPASISCRSSQSLVYSDGNTYLNWSQQRPGQSPRRLIYKVSNRDSGVPDRFSGSGSGTDFTLKISRVEAEDVGVYYCMQGTHWPYTFGQGTKLEIK

SEQ ID NO: 323 - DNA, 33 bp, synthetic construct
  misc_feature 1..33: note = Synthetic
  source 1..33: mol_type = other DNA
caaagcctcgtatacagtgatggaaacacctac

SEQ ID NO: 324 - protein, 11 aa, synthetic construct
  REGION 1..11: note = Synthetic
QSLVYSDGNTY

SEQ ID NO: 325-326 - skipped (2 entries)

SEQ ID NO: 327 - DNA, 27 bp, synthetic construct
  misc_feature 1..27: note = Synthetic
  source 1..27: mol_type = other DNA
atgcaaggtacacactggccgtacact

SEQ ID NO: 328 - protein, 9 aa, synthetic construct
  REGION 1..9: note = Synthetic
MQGTHWPYT

SEQ ID NO: 329 - DNA, 381 bp, synthetic construct; identical to SEQ ID NO: 313
  misc_feature 1..381: note = Synthetic
  source 1..381: mol_type = other DNA

SEQ ID NO: 330 - protein, 127 aa, synthetic construct; identical to SEQ ID NO: 314
  REGION 1..127: note = Synthetic

SEQ ID NO: 331 - DNA, 336 bp, synthetic construct; identical to SEQ ID NO: 321
  misc_feature 1..336: note = Synthetic
  source 1..336: mol_type = other DNA

SEQ ID NO: 332 - protein, 112 aa, synthetic construct; identical to SEQ ID NO: 322
  REGION 1..112: note = Synthetic

SEQ ID NO: 333 - DNA, 381 bp, synthetic construct
  misc_feature 1..381: note = Synthetic
  source 1..381: mol_type = other DNA
caggttcagctggtgcagtctggagctgaggtgaagaagcctggggcctcagtgaaggtctcctgcaaggcttctggttacacctttaccacctatggtatcagctgggtgcgacaggcccctggacaagggcttgagtggatgggatggatcagcggttacaatggtaaaacaaactatgcacagaagctccagggcagagtcaccatgaccacagacacatccacgagcacagcctacatggagctgaggagcctgagatctgacgacacggccgtgtattactgttcgagagatcgtttagtagtaccacctgcccttaattattcctactacgttatggacgtctgggggcaagggaccacggtcaccgtctcctca

SEQ ID NO: 334 - protein, 127 aa, synthetic construct
  REGION 1..127: note = Synthetic
QVQLVQSGAEVKKPGASVKVSCKASGYTFTTYGISWVRQAPGQGLEWMGWISGYNGKTNYAQKLQGRVTMTTDTSTSTAYMELRSLRSDDTAVYYCSRDRLVVPPALNYSYYVMDVWGQGTTVTVSS

SEQ ID NO: 335 - DNA, 336 bp, synthetic construct
  misc_feature 1..336: note = Synthetic
  source 1..336: mol_type = other DNA
gatgttgtgatgactcagtctccactctccctgcccgtcacccttggacagccggcctccatctcctgcaggtctagtcaaagcctcgtatacagtgatggaaacacctacttgaattggtttcagcagaggccaggccaatctccaaggcgcctaatttataaggtttctaaccgggactctggggtcccagacagattcagcggcagtgggtcaggcactgatttcacactgaaaatcagcagggtggaggctgaggatgttggggtttattactgcatgcaaggtacacactggccgtacacttttggccaggggaccaagctggagatcaaa

SEQ ID NO: 336 - protein, 112 aa, synthetic construct
  REGION 1..112: note = Synthetic
DVVMTQSPLSLPVTLGQPASISCRSSQSLVYSDGNTYLNWFQQRPGQSPRRLIYKVSNRDSGVPDRFSGSGSGTDFTLKISRVEAEDVGVYYCMQGTHWPYTFGQGTKLEIK

SEQ ID NO: 337 - DNA, 354 bp, synthetic construct
  misc_feature 1..354: note = Synthetic
  source 1..354: mol_type = other DNA
gaggtgcagctggtggagtctgggggaggcctggtcaagcctggggggtccctgagactctcctgtgcagcctctggattcaccttcagtagctatagcatggactgggtccgccaggctccagggaaggggctggagtgggtctcatccattagtagtagtagtagttacatatactacgcagactctgtgaagggccgattcaccatctccagagacaccgccaagaactcactgtatctgcaaatgaacagcctgagagacgaggacacggctgtttattactgtgcgagagagggcagtagcagactttttgactactggggccagggaaccctggtcaccgtctcctca

SEQ ID NO: 338 - protein, 118 aa, synthetic construct
  REGION 1..118: note = Synthetic
EVQLVESGGGLVKPGGSLRLSCAASGFTFSSYSMDWVRQAPGKGLEWVSSISSSSSYIYYADSVKGRFTISRDTAKNSLYLQMNSLRDEDTAVYYCAREGSSRLFDYWGQGTLVTVSS

SEQ ID NO: 339 - DNA, 24 bp, synthetic construct
  misc_feature 1..24: note = Synthetic
  source 1..24: mol_type = other DNA
ggattcaccttcagtagctatagc

SEQ ID NO: 340 - protein, 8 aa, synthetic construct
  REGION 1..8: note = Synthetic
GFTFSSYS

SEQ ID NO: 341 - DNA, 24 bp, synthetic construct
  misc_feature 1..24: note = Synthetic
  source 1..24: mol_type = other DNA
attagtagtagtagtagttacata

SEQ ID NO: 342 - protein, 8 aa, synthetic construct
  REGION 1..8: note = Synthetic
ISSSSSYI

SEQ ID NO: 343 - DNA, 33 bp, synthetic construct
  misc_feature 1..33: note = Synthetic
  source 1..33: mol_type = other DNA
gcgagagagggcagtagcagactttttgactac

SEQ ID NO: 344 - protein, 11 aa, synthetic construct
  REGION 1..11: note = Synthetic
AREGSSRLFDY

SEQ ID NO: 345 - DNA, 321 bp, synthetic construct
  misc_feature 1..321: note = Synthetic
  source 1..321: mol_type = other DNA
gacatccagatgacccagtctccttccaccctgtctgcatctgtaggagacagagtcaccatcacttgccgggccagtcagagtattagtagctggttggcctggtatcagcagagaccagggaaagcccctaagctcctgatctataaggcgtctagtttagaaggtggagtcccatcaaggttcagcggcagtggatctgggacagaattcactctcaccatcagcagcctgcagcctgaggattttgcaacttattactgccaacagtataatagttattggtacacttttggccaggggaccaagctggagatcaaa

SEQ ID NO: 346 - protein, 107 aa, synthetic construct
  REGION 1..107: note = Synthetic
DIQMTQSPSTLSASVGDRVTITCRASQSISSWLAWYQQRPGKAPKLLIYKASSLEGGVPSRFSGSGSGTEFTLTISSLQPEDFATYYCQQYNSYWYTFGQGTKLEIK

SEQ ID NO: 347 - DNA, 18 bp, synthetic construct
  misc_feature 1..18: note = Synthetic
  source 1..18: mol_type = other DNA
cagagtattagtagctgg

SEQ ID NO: 348 - protein, 6 aa, synthetic construct
  REGION 1..6: note = Synthetic
QSISSW

SEQ ID NO: 349-350 - skipped (2 entries)

SEQ ID NO: 351 - DNA, 27 bp, synthetic construct
  misc_feature 1..27: note = Synthetic
  source 1..27: mol_type = other DNA
caacagtataatagttattggtacact

SEQ ID NO: 352 - protein, 9 aa, synthetic construct
  REGION 1..9: note = Synthetic
QQYNSYWYT

SEQ ID NO: 353 - DNA, 354 bp, synthetic construct; identical to SEQ ID NO: 337
  misc_feature 1..354: note = Synthetic
  source 1..354: mol_type = other DNA

SEQ ID NO: 354 - protein, 118 aa, synthetic construct; identical to SEQ ID NO: 338
  REGION 1..118: note = Synthetic

SEQ ID NO: 355 - DNA, 321 bp, synthetic construct; identical to SEQ ID NO: 345
  misc_feature 1..321: note = Synthetic
  source 1..321: mol_type = other DNA

SEQ ID NO: 356 - protein, 107 aa, synthetic construct; identical to SEQ ID NO: 346
  REGION 1..107: note = Synthetic

SEQ ID NO: 357 - DNA, 354 bp, synthetic construct
  misc_feature 1..354: note = Synthetic
  source 1..354: mol_type = other DNA
gaggtgcagctggtggagtctgggggaggcctggtcaagcctggggggtccctgagactctcctgtgcagcctctggattcaccttcagtagctatagcatgaactgggtccgccaggctccagggaaggggctggagtgggtctcatccattagtagtagtagtagttacatatactacgcagactcagtgaagggccgattcaccatctccagagacaacgccaagaactcactgtatctgcaaatgaacagcctgagagccgaggacacggctgtgtattactgtgcgagagagggcagtagcagactttttgactactggggccaaggaaccctggtcaccgtctcctca

SEQ ID NO: 358 - protein, 118 aa, synthetic construct
  REGION 1..118: note = Synthetic
EVQLVESGGGLVKPGGSLRLSCAASGFTFSSYSMNWVRQAPGKGLEWVSSISSSSSYIYYADSVKGRFTISRDNAKNSLYLQMNSLRAEDTAVYYCAREGSSRLFDYWGQGTLVTVSS

SEQ ID NO: 359 - DNA, 321 bp, synthetic construct
  misc_feature 1..321: note = Synthetic
  source 1..321: mol_type = other DNA
gacatccagatgacccagtctccttccaccctgtctgcatctgtaggagacagagtcaccatcacttgccgggccagtcagagtattagtagctggttggcctggtatcagcagaaaccagggaaagcccctaagctcctgatctataaggcgtctagtttagaaagtggggtcccatcaaggttcagcggcagtggatctgggacagaattcactctcaccatcagcagcctgcagcctgatgattttgcaacttattactgccaacagtataatagttattggtacacttttggccaggggaccaagctggagatcaaa

SEQ ID NO: 360 - protein, 107 aa, synthetic construct
  REGION 1..107: note = Synthetic
DIQMTQSPSTLSASVGDRVTITCRASQSISSWLAWYQQKPGKAPKLLIYKASSLESGVPSRFSGSGSGTEFTLTISSLQPDDFATYYCQQYNSYWYTFGQGTKLEIK

SEQ ID NO: 361 - DNA, 384 bp, synthetic construct
  misc_feature 1..384: note = Synthetic
  source 1..384: mol_type = other DNA
caggtgcacctggtggagtctgggggaggcttggtcaagcctggagggtccctgagactctcctgtgcagcctctggattcaccttcagtgaccactacatgagctggatccgccaggctccagggaaggggctggagtggatttcatacattagtaatgatggtggtaccaaatactatgtggactctgtggagggccgattcatcatttccagggacaacgccaagaactcattgtatctacatatgaacagcctcagagccgacgacacggccgtgtattactgtgcgagagatcagggatatattggctacgactcgtattattactattcctacggtatggacgtctggggccaagggaccacggtcaccgtcgcctca

SEQ ID NO: 362 - protein, 128 aa, synthetic construct
  REGION 1..128: note = Synthetic
QVHLVESGGGLVKPGGSLRLSCAASGFTFSDHYMSWIRQAPGKGLEWISYISNDGGTKYYVDSVEGRFIISRDNAKNSLYLHMNSLRADDTAVYYCARDQGYIGYDSYYYYSYGMDVWGQGTTVTVAS

SEQ ID NO: 363 - DNA, 24 bp, synthetic construct
  misc_feature 1..24: note = Synthetic
  source 1..24: mol_type = other DNA
ggattcaccttcagtgaccactac

SEQ ID NO: 364 - protein, 8 aa, synthetic construct
  REGION 1..8: note = Synthetic
GFTFSDHY

SEQ ID NO: 365 - DNA, 24 bp, synthetic construct
  misc_feature 1..24: note = Synthetic
  source 1..24: mol_type = other DNA
attagtaatgatggtggtaccaaa

SEQ ID NO: 366 - protein, 8 aa, synthetic construct
  REGION 1..8: note = Synthetic
ISNDGGTK

SEQ ID NO: 367 - DNA, 63 bp, synthetic construct
  misc_feature 1..63: note = Synthetic
  source 1..63: mol_type = other DNA
gcgagagatcagggatatattggctacgactcgtattattactattcctacggtatggacgtc

SEQ ID NO: 368 - protein, 21 aa, synthetic construct
  REGION 1..21: note = Synthetic
ARDQGYIGYDSYYYYSYGMDV

SEQ ID NO: 369 - DNA, 321 bp, synthetic construct
  misc_feature 1..321: note = Synthetic
  source 1..321: mol_type = other DNA
aaaattgtgttgacgcagtctccaggcaccctgcctttgtttccaggggaaagagccaccctctcctgtagggccagtcagagtgttaacaacaaattcttagcctggtaccagcagaaatctggccaggctcccaggctcctcatctatggtgcatccagcagggccactggcatcccagacaggttcagtggcagtgggtctgggaccgacttcactctcaccatcagcggactggagcctgaagattttgaagtgtattattgtcaagtatatggtaactcactcactctcggcggagggaccaaggtggagatcaag

SEQ ID NO: 370 - protein, 107 aa, synthetic construct
  REGION 1..107: note = Synthetic
KIVLTQSPGTLPLFPGERATLSCRASQSVNNKFLAWYQQKSGQAPRLLIYGASSRATGIPDRFSGSGSGTDFTLTISGLEPEDFEVYYCQVYGNSLTLGGGTKVEIK

SEQ ID NO: 371 - DNA, 21 bp, synthetic construct
  misc_feature 1..21: note = Synthetic
  source 1..21: mol_type = other DNA
cagagtgttaacaacaaattc

SEQ ID NO: 372 - protein, 7 aa, synthetic construct
  REGION 1..7: note = Synthetic
QSVNNKF

SEQ ID NO: 373-374 - skipped (2 entries)

SEQ ID NO: 375 - DNA, 24 bp, synthetic construct
  misc_feature 1..24: note = Synthetic
  source 1..24: mol_type = other DNA
caagtatatggtaactcactcact

SEQ ID NO: 376 - protein, 8 aa, synthetic construct
  REGION 1..8: note = Synthetic
QVYGNSLT

SEQ ID NO: 377 - DNA, 384 bp, synthetic construct
  misc_feature 1..384: note = Synthetic
  source 1..384: mol_type = other DNA
caggtgcagctggtggagtctgggggaggcttggtcaagcctggagggtccctgagactctcctgtgcagcctctggattcaccttcagtgaccactacatgagctggatccgccaggctccagggaaggggctggagtggatttcatacattagtaatgatggtggtaccaaatactatgtggactctgtggagggccgattcatcatttccagggacaacgccaagaactcattgtatctacatatgaacagcctcagagccgacgacacggccgtgtattactgtgcgagagatcagggatatattggctacgactcgtattattactattcctacggtatggacgtctggggccaagggaccacggtcaccgtctcctca

SEQ ID NO: 378 - protein, 128 aa, synthetic construct
  REGION 1..128: note = Synthetic
QVQLVESGGGLVKPGGSLRLSCAASGFTFSDHYMSWIRQAPGKGLEWISYISNDGGTKYYVDSVEGRFIISRDNAKNSLYLHMNSLRADDTAVYYCARDQGYIGYDSYYYYSYGMDVWGQGTTVTVSS

SEQ ID NO: 379 - DNA, 321 bp, synthetic construct
  misc_feature 1..321: note = Synthetic
  source 1..321: mol_type = other DNA
gaaattgtgttgacgcagtctccaggcaccctgcctttgtttccaggggaaagagccaccctctcctgtagggccagtcagagtgttaacaacaaattcttagcctggtaccagcagaaatctggccaggctcccaggctcctcatctatggtgcatccagcagggccactggcatcccagacaggttcagtggcagtgggtctgggaccgacttcactctcaccatcagcggactggagcctgaagattttgaagtgtattattgtcaagtatatggtaactcactcactctcggcggagggaccaaggtggagatcaaa

SEQ ID NO: 380 - protein, 107 aa, synthetic construct
  REGION 1..107: note = Synthetic
EIVLTQSPGTLPLFPGERATLSCRASQSVNNKFLAWYQQKSGQAPRLLIYGASSRATGIPDRFSGSGSGTDFTLTISGLEPEDFEVYYCQVYGNSLTLGGGTKVEIK

SEQ ID NO: 381 - DNA, 384 bp, synthetic construct
  misc_feature 1..384: note = Synthetic
  source 1..384: mol_type = other DNA
caggtgcagctggtggagtctgggggaggcttggtcaagcctggagggtccctgagactctcctgtgcagcctctggattcaccttcagtgaccactacatgagctggatccgccaggctccagggaaggggctggagtgggtttcatacattagtaatgatggtggtaccaaatactacgcagactctgtgaagggccgattcaccatctccagggacaacgccaagaactcactgtatctgcaaatgaacagcctgagagccgaggacacggccgtgtattactgtgcgagagatcagggatatattggctacgactcgtattattactattcctacggtatggacgtctgggggcaagggaccacggtcaccgtctcctca

SEQ ID NO: 382 - protein, 128 aa, synthetic construct
  REGION 1..128: note = Synthetic
QVQLVESGGGLVKPGGSLRLSCAASGFTFSDHYMSWIRQAPGKGLEWVSYISNDGGTKYYADSVKGRFTISRDNAKNSLYLQMNSLRAEDTAVYYCARDQGYIGYDSYYYYSYGMDVWGQGTTVTVSS

SEQ ID NO: 383 - DNA, 321 bp, synthetic construct
  misc_feature 1..321: note = Synthetic
  source 1..321: mol_type = other DNA
gaaattgtgttgacgcagtctccaggcaccctgtctttgtctccaggggaaagagccaccctctcctgcagggccagtcagagtgttaacaacaaattcttagcctggtaccagcagaaacctggccaggctcccaggctcctcatctatggtgcatccagcagggccactggcatcccagacaggttcagtggcagtgggtctgggacagacttcactctcaccatcagcagactggagcctgaagattttgcagtgtattactgtcaagtatatggtaactcactcactttcggcggagggaccaaggtggagatcaaa

SEQ ID NO: 384 - protein, 107 aa, synthetic construct
  REGION 1..107: note = Synthetic
EIVLTQSPGTLSLSPGERATLSCRASQSVNNKFLAWYQQKPGQAPRLLIYGASSRATGIPDRFSGSGSGTDFTLTISRLEPEDFAVYYCQVYGNSLTFGGGTKVEIK

SEQ ID NO: 385 - DNA, 360 bp, synthetic construct
  misc_feature 1..360: note = Synthetic
  source 1..360: mol_type = other DNA
gaggtgcagaaggtggagtctgggggaggcctggtcaagccgggggggtccctgagactctcctgtacagcctctggattcaccttcagtacttataacatgaattgggtccgccaggctccagggaagggactggagtgggtctcatccattaggagtagtagtaattacatatactacgcagactcagtgaagggccgattcaccatctccagagacaacgccaagaattcactgtatctgcaaatgaacagcctgagagccgatgacacggctgtgtattactgtgcgagagatggcagcagttggtacgactactctgactactggggccagggaaccctggtcaccgtctcctca

SEQ ID NO: 386 - protein, 120 aa, synthetic construct
  REGION 1..120: note = Synthetic
EVQKVESGGGLVKPGGSLRLSCTASGFTFSTYNMNWVRQAPGKGLEWVSSIRSSSNYIYYADSVKGRFTISRDNAKNSLYLQMNSLRADDTAVYYCARDGSSWYDYSDYWGQGTLVTVSS

SEQ ID NO: 387 - DNA, 24 bp, synthetic construct
  misc_feature 1..24: note = Synthetic
  source 1..24: mol_type = other DNA
ggattcaccttcagtacttataac

SEQ ID NO: 388 - protein, 8 aa, synthetic construct
  REGION 1..8: note = Synthetic
GFTFSTYN

SEQ ID NO: 389 - DNA, 24 bp, synthetic construct
  misc_feature 1..24: note = Synthetic
  source 1..24: mol_type = other DNA
attaggagtagtagtaattacata

SEQ ID NO: 390 - protein, 8 aa, synthetic construct
  REGION 1..8: note = Synthetic
IRSSSNYI

SEQ ID NO: 391 - DNA, 39 bp, synthetic construct
  misc_feature 1..39: note = Synthetic
  source 1..39: mol_type = other DNA
gcgagagatggcagcagttggtacgactactctgactac

SEQ ID NO: 392 - protein, 13 aa, synthetic construct
  REGION 1..13: note = Synthetic
ARDGSSWYDYSDY

SEQ ID NO: 393 - DNA, 321 bp, synthetic construct
  misc_feature 1..321: note = Synthetic
  source 1..321: mol_type = other DNA
gacatccagatgacccagtctccttccaccctgtctgcatctgtaggagacagagtcaccatcacttgccgggccagtcagagtattagtagctggttggcctggtatcaacagataccagggaaagcccctaaactcctgatctataaggcgtctagtttagaaaatggggtcccatcaaggttcagcggcagtggatctgggacagaattcactctcatcatcagcagcctgcagcctgatgattttgcaacttattactgccaacagtatattagttattctcggacgttcggccaagggaccaaggtggaaatcaaa

SEQ ID NO: 394 - protein, 107 aa, synthetic construct
  REGION 1..107: note = Synthetic
DIQMTQSPSTLSASVGDRVTITCRASQSISSWLAWYQQIPGKAPKLLIYKASSLENGVPSRFSGSGSGTEFTLIISSLQPDDFATYYCQQYISYSRTFGQGTKVEIK

SEQ ID NO: 395 - DNA, 18 bp, synthetic construct
  misc_feature 1..18: note = Synthetic
  source 1..18: mol_type = other DNA
cagagtattagtagctgg

SEQ ID NO: 396 - protein, 6 aa, synthetic construct
  REGION 1..6: note = Synthetic
QSISSW

SEQ ID NO: 397-398 - skipped (2 entries)

SEQ ID NO: 399 - DNA, 27 bp, synthetic construct
  misc_feature 1..27: note = Synthetic
  source 1..27: mol_type = other DNA
caacagtatattagttattctcggacg

SEQ ID NO: 400 - protein, 9 aa, synthetic construct
  REGION 1..9: note = Synthetic
QQYISYSRT

SEQ ID NO: 401 - DNA, 360 bp, synthetic construct
  misc_feature 1..360: note = Synthetic
  source 1..360: mol_type = other DNA
gaggtgcagctggtggagtctgggggaggcctggtcaagccgggggggtccctgagactctcctgtacagcctctggattcaccttcagtacttataacatgaattgggtccgccaggctccagggaagggactggagtgggtctcatccattaggagtagtagtaattacatatactacgcagactcagtgaagggccgattcaccatctccagagacaacgccaagaattcactgtatctgcaaatgaacagcctgagagccgatgacacggctgtgtattactgtgcgagagatggcagcagttggtacgactactctgactactggggccagggaaccctggtcaccgtctcctca

SEQ ID NO: 402 - protein, 120 aa, synthetic construct
  REGION 1..120: note = Synthetic
EVQLVESGGGLVKPGGSLRLSCTASGFTFSTYNMNWVRQAPGKGLEWVSSIRSSSNYIYYADSVKGRFTISRDNAKNSLYLQMNSLRADDTAVYYCARDGSSWYDYSDYWGQGTLVTVSS

SEQ ID NO: 403 - DNA, 321 bp, synthetic construct; identical to SEQ ID NO: 393
  misc_feature 1..321: note = Synthetic
  source 1..321: mol_type = other DNA

SEQ ID NO: 404 - protein, 107 aa, synthetic construct; identical to SEQ ID NO: 394
  REGION 1..107: note = Synthetic

SEQ ID NO: 405 - DNA, 360 bp, synthetic construct
  misc_feature 1..360: note = Synthetic
  source 1..360: mol_type = other DNA
gaggtgcagctggtggagtctgggggaggcctggtcaagcctggggggtccctgagactctcctgtgcagcctctggattcaccttcagtacttataacatgaactgggtccgccaggctccagggaaggggctggagtgggtctcatccattaggagtagtagtaattacatatactacgcagactcagtgaagggccgattcaccatctccagagacaacgccaagaactcactgtatctgcaaatgaacagcctgagagccgaggacacggctgtgtattactgtgcgagagatggcagcagttggtacgactactctgactactggggccaaggaaccctggtcaccgtctcctca

SEQ ID NO: 406 - protein, 120 aa, synthetic construct
  REGION 1..120: note = Synthetic
EVQLVESGGGLVKPGGSLRLSCAASGFTFSTYNMNWVRQAPGKGLEWVSSIRSSSNYIYYADSVKGRFTISRDNAKNSLYLQMNSLRAEDTAVYYCARDGSSWYDYSDYWGQGTLVTVSS

SEQ ID NO: 407 - DNA, 321 bp, synthetic construct
  misc_feature 1..321: note = Synthetic
  source 1..321: mol_type = other DNA
gacatccagatgacccagtctccttccaccctgtctgcatctgtaggagacagagtcaccatcacttgccgggccagtcagagtattagtagctggttggcctggtatcagcagaaaccagggaaagcccctaagctcctgatctataaggcgtctagtttagaaagtggggtcccatcaaggttcagcggcagtggatctgggacagaattcactctcaccatcagcagcctgcagcctgatgattttgcaacttattactgccaacagtatattagttattctcggacgttcggccaagggaccaaggtggaaatcaaa

SEQ ID NO: 408 - protein, 107 aa, synthetic construct
  REGION 1..107: note = Synthetic
DIQMTQSPSTLSASVGDRVTITCRASQSISSWLAWYQQKPGKAPKLLIYKASSLESGVPSRFSGSGSGTEFTLTISSLQPDDFATYYCQQYISYSRTFGQGTKVEIK

SEQ ID NO: 409 - DNA, 360 bp, synthetic construct; identical to SEQ ID NO: 401
  misc_feature 1..360: note = Synthetic
  source 1..360: mol_type = other DNA

SEQ ID NO: 410 - protein, 120 aa, synthetic construct; identical to SEQ ID NO: 402
  REGION 1..120: note = Synthetic

SEQ ID NO: 411 - DNA, 24 bp, synthetic construct
  misc_feature 1..24: note = Synthetic
  source 1..24: mol_type = other DNA
ggattcaccttcagtacttataac

SEQ ID NO: 412 - protein, 8 aa, synthetic construct
  REGION 1..8: note = Synthetic
GFTFSTYN

SEQ ID NO: 413 - DNA, 24 bp, synthetic construct
  misc_feature 1..24: note = Synthetic
  source 1..24: mol_type = other DNA
attaggagtagtagtaattacata

SEQ ID NO: 414 - protein, 8 aa, synthetic construct
  REGION 1..8: note = Synthetic
IRSSSNYI

SEQ ID NO: 415 - DNA, 39 bp, synthetic construct; identical to SEQ ID NO: 391
  misc_feature 1..39: note = Synthetic
  source 1..39: mol_type = other DNA

SEQ ID NO: 416 - protein, 13 aa, synthetic construct
  REGION 1..13: note = Synthetic
ARDGSSWYDYSDY

SEQ ID NO: 417 - DNA, 321 bp, synthetic construct; identical to SEQ ID NO: 393
  misc_feature 1..321: note = Synthetic
  source 1..321: mol_type = other DNA

SEQ ID NO: 418 - protein, 107 aa, synthetic construct; identical to SEQ ID NO: 394
  REGION 1..107: note = Synthetic

SEQ ID NO: 419 - DNA, 18 bp, synthetic construct
  misc_feature 1..18: note = Synthetic
  source 1..18: mol_type = other DNA
cagagtattagtagctgg

SEQ ID NO: 420 - protein, 6 aa, synthetic construct
  REGION 1..6: note = Synthetic
QSISSW

SEQ ID NO: 421-422 - skipped (2 entries)

SEQ ID NO: 423 - DNA, 27 bp, synthetic construct
  misc_feature 1..27: note = Synthetic
  source 1..27: mol_type = other DNA
caacagtatattagttattctcggacg

SEQ ID NO: 424 - protein, 9 aa, synthetic construct
  REGION 1..9: note = Synthetic
QQYISYSRT

SEQ ID NO: 425 - DNA, 360 bp, synthetic construct; identical to SEQ ID NO: 401
  misc_feature 1..360: note = Synthetic
  source 1..360: mol_type = other DNA

SEQ ID NO: 426 - protein, 120 aa, synthetic construct; identical to SEQ ID NO: 402
  REGION 1..120: note = Synthetic

SEQ ID NO: 427 - DNA, 321 bp, synthetic construct; identical to SEQ ID NO: 393
  misc_feature 1..321: note = Synthetic
  source 1..321: mol_type = other DNA

SEQ ID NO: 428 - protein, 107 aa, synthetic construct; identical to SEQ ID NO: 394
  REGION 1..107: note = Synthetic

SEQ ID NO: 429 - DNA, 360 bp, synthetic construct; identical to SEQ ID NO: 405
  misc_feature 1..360: note = Synthetic
  source 1..360: mol_type = other DNA

SEQ ID NO: 430 - protein, 120 aa, synthetic construct; identical to SEQ ID NO: 406
  REGION 1..120: note = Synthetic

SEQ ID NO: 431 - DNA, 321 bp, synthetic construct; identical to SEQ ID NO: 407
  misc_feature 1..321: note = Synthetic
  source 1..321: mol_type = other DNA

SEQ ID NO: 432 - protein, 107 aa, synthetic construct; identical to SEQ ID NO: 408
  REGION 1..107: note = Synthetic

SEQ ID NO: 433 - DNA, 360 bp, synthetic construct
  misc_feature 1..360: note = Synthetic
  source 1..360: mol_type = other DNA
gaggtgcagctggtggagtctgggggaggcctggtcaagccgggggggtccctgagactctcctgtacagcctctggattcaccttcagtacttataacatgaattgggtccgccaggctccagggaagggactggagtgggtctcatccattaggagtagtagtaattacatatactacgcagactcagtgaagggccgattcaccatctccagagacaacgccaagagttcactgtatctgcaaatgaacagcctgagagccgaggacacggctgtgtattactgtgcgagagatggcagcagttggtacgactactctgactactggggccagggaaccctggtcaccgtctcctca

SEQ ID NO: 434 - protein, 120 aa, synthetic construct
  REGION 1..120: note = Synthetic
EVQLVESGGGLVKPGGSLRLSCTASGFTFSTYNMNWVRQAPGKGLEWVSSIRSSSNYIYYADSVKGRFTISRDNAKSSLYLQMNSLRAEDTAVYYCARDGSSWYDYSDYWGQGTLVTVSS

SEQ ID NO: 435 - DNA, 24 bp, synthetic construct
  misc_feature 1..24: note = Synthetic
  source 1..24: mol_type = other DNA
ggattcaccttcagtacttataac

SEQ ID NO: 436 - protein, 8 aa, synthetic construct
  REGION 1..8: note = Synthetic
GFTFSTYN

SEQ ID NO: 437 - DNA, 24 bp, synthetic construct
  misc_feature 1..24: note = Synthetic
  source 1..24: mol_type = other DNA
attaggagtagtagtaattacata

SEQ ID NO: 438 - protein, 8 aa, synthetic construct
  REGION 1..8: note = Synthetic
IRSSSNYI

SEQ ID NO: 439 - DNA, 39 bp, synthetic construct; identical to SEQ ID NO: 391
  misc_feature 1..39: note = Synthetic
  source 1..39: mol_type = other DNA

SEQ ID NO: 440 - protein, 13 aa, synthetic construct
  REGION 1..13: note = Synthetic
ARDGSSWYDYSDY

SEQ ID NO: 441 - DNA, 321 bp, synthetic construct
  misc_feature 1..321: note = Synthetic
  source 1..321: mol_type = other DNA
gacatccagatgacccagtctccttccaccctgtctgcatctgtaggagacagagtcaccatcacttgccgggccagtcagagtattagtagctggttggcctggtatcaacaggtaccagggaaagcccctaaactcctgatctataaggcgtctagtttagaaaatggggtcccatcaaggttcagcggcagtggatctgggacagaattcactctcatcatcagcagcctgcagcctgatgattttgcaacttattactgccaacagtatattagttattctcggacgttcggccaagggaccaaggtggaaatcaaa

SEQ ID NO: 442 - protein, 107 aa, synthetic construct
  REGION 1..107: note = Synthetic
DIQMTQSPSTLSASVGDRVTITCRASQSISSWLAWYQQVPGKAPKLLIYKASSLENGVPSRFSGSGSGTEFTLIISSLQPDDFATYYCQQYISYSRTFGQGTKVEIK

SEQ ID NO: 443 - DNA, 18 bp, synthetic construct
  misc_feature 1..18: note = Synthetic
  source 1..18: mol_type = other DNA
cagagtattagtagctgg

SEQ ID NO: 444 - protein, 6 aa, synthetic construct
  REGION 1..6: note = Synthetic
QSISSW

SEQ ID NO: 445-446 - skipped (2 entries)

SEQ ID NO: 447 - DNA, 27 bp, synthetic construct
  misc_feature 1..27: note = Synthetic
  source 1..27: mol_type = other DNA
caacagtatattagttattctcggacg

SEQ ID NO: 448 - protein, 9 aa, synthetic construct
  REGION 1..9: note = Synthetic
QQYISYSRT

SEQ ID NO: 449 - DNA, 360 bp, synthetic construct; identical to SEQ ID NO: 433
  misc_feature 1..360: note = Synthetic
  source 1..360: mol_type = other DNA

SEQ ID NO: 450 - protein, 120 aa, synthetic construct; identical to SEQ ID NO: 434
  REGION 1..120: note = Synthetic

SEQ ID NO: 451 - DNA, 321 bp, synthetic construct; identical to SEQ ID NO: 441
  misc_feature 1..321: note = Synthetic
  source 1..321: mol_type = other DNA

SEQ ID NO: 452 - protein, 107 aa, synthetic construct; identical to SEQ ID NO: 442
  REGION 1..107: note = Synthetic

SEQ ID NO: 453 - DNA, 360 bp, synthetic construct
  misc_feature 1..360: note = Synthetic
  source 1..360: mol_type = other DNA
gaggtgcagctggtggagtctgggggaggcctggtcaagcctggggggtccctgagactctcctgtgcagcctctggattcaccttcagtacttataacatgaactgggtccgccaggctccagggaaggggctggagtgggtctcatccattaggagtagtagtaattacatatactacgcagactcagtgaagggccgattcaccatctccagagacaacgccaagaactcactgtatctgcaaatgaacagcctgagagccgaggacacggctgtgtattactgtgcgagagatggcagcagttggtacgactactctgactactggggccagggaaccctggtcaccgtctcctca

SEQ ID NO: 454 - protein, 120 aa, synthetic construct; identical to SEQ ID NO: 406
  REGION 1..120: note = Synthetic

SEQ ID NO: 455 - DNA, 321 bp, synthetic construct; identical to SEQ ID NO: 407
  misc_feature 1..321: note = Synthetic
  source 1..321: mol_type = other DNA

SEQ ID NO: 456 - protein, 107 aa, synthetic construct; identical to SEQ ID NO: 408
  REGION 1..107: note = Synthetic

SEQ ID NO: 457 - DNA, 360 bp, synthetic construct; identical to SEQ ID NO: 401
  misc_feature 1..360: note = Synthetic
  source 1..360: mol_type = other DNA

SEQ ID NO: 458 - protein, 120 aa, synthetic construct; identical to SEQ ID NO: 402
  REGION 1..120: note = Synthetic

SEQ ID NO: 459 - DNA, 24 bp, synthetic construct
  misc_feature 1..24: note = Synthetic
  source 1..24: mol_type = other DNA
ggattcaccttcagtacttataac

SEQ ID NO: 460 - protein, 8 aa, synthetic construct
  REGION 1..8: note = Synthetic
GFTFSTYN

SEQ ID NO: 461 - DNA, 24 bp, synthetic construct
  misc_feature 1..24: note = Synthetic
  source 1..24: mol_type = other DNA
attaggagtagtagtaattacata

SEQ ID NO: 462 - protein, 8 aa, synthetic construct
  REGION 1..8: note = Synthetic
IRSSSNYI

SEQ ID NO: 463 - DNA, 39 bp, synthetic construct; identical to SEQ ID NO: 391
  misc_feature 1..39: note = Synthetic
  source 1..39: mol_type = other DNA

SEQ ID NO: 464 - protein, 13 aa, synthetic construct
  REGION 1..13: note = Synthetic
ARDGSSWYDYSDY

SEQ ID NO: 465 - DNA, 321 bp, synthetic construct; identical to SEQ ID NO: 393
  misc_feature 1..321: note = Synthetic
  source 1..321: mol_type = other DNA

SEQ ID NO: 466 - protein, 107 aa, synthetic construct; identical to SEQ ID NO: 394
  REGION 1..107: note = Synthetic

SEQ ID NO: 467 - DNA, 18 bp, synthetic construct
  misc_feature 1..18: note = Synthetic
  source 1..18: mol_type = other DNA
cagagtattagtagctgg

SEQ ID NO: 468 - protein, 6 aa, synthetic construct
  REGION 1..6: note = Synthetic
QSISSW

SEQ ID NO: 469-470 - skipped (2 entries)

SEQ ID NO: 471 - DNA, 27 bp, synthetic construct
  misc_feature 1..27: note = Synthetic
  source 1..27: mol_type = other DNA
caacagtatattagttattctcggacg

SEQ ID NO: 472 - protein, 9 aa, synthetic construct
  REGION 1..9: note = Synthetic
QQYISYSRT

SEQ ID NO: 473 - DNA, 360 bp, synthetic construct; identical to SEQ ID NO: 401
  misc_feature 1..360: note = Synthetic
  source 1..360: mol_type = other DNA

SEQ ID NO: 474 - protein, 120 aa, synthetic construct; identical to SEQ ID NO: 402
  REGION 1..120: note = Synthetic

SEQ ID NO: 475 - DNA, 321 bp, synthetic construct; identical to SEQ ID NO: 393
  misc_feature 1..321: note = Synthetic
  source 1..321: mol_type = other DNA

SEQ ID NO: 476 - protein, 107 aa, synthetic construct; identical to SEQ ID NO: 394
  REGION 1..107: note = Synthetic

SEQ ID NO: 477 - DNA, 360 bp, synthetic construct; identical to SEQ ID NO: 405
  misc_feature 1..360: note = Synthetic
  source 1..360: mol_type = other DNA

SEQ ID NO: 478 - protein, 120 aa, synthetic construct; identical to SEQ ID NO: 406
  REGION 1..120: note = Synthetic

SEQ ID NO: 479 - DNA, 321 bp, synthetic construct; identical to SEQ ID NO: 407
  misc_feature 1..321: note = Synthetic
  source 1..321: mol_type = other DNA

SEQ ID NO: 480 - protein, 107 aa, synthetic construct; identical to SEQ ID NO: 408
  REGION 1..107: note = Synthetic

SEQ ID NO: 481 - DNA, 354 bp, synthetic construct
  misc_feature 1..354: note = Synthetic
  source 1..354: mol_type = other DNA
gaggtgcaactagtggagtctgggggaggcttggtacagcctggggggtccctgagactctcctgtgtagtctctggattcaccttcggtgactacgacatgcactgggtccgtcaagctacaggaagaggtctggagtgggtctcaggtattgctcctgctggtgacacatcctatacaggctccgtgaagggccgattcaccatctccagagagaatgccaagaactccttgcatcttcaaatgaacagcctgacaaccggggacacggctatatattattgtgctagagaggatatagcagtgcctggttttgattactggggccagggaaccctggtcaccgtctcctca

SEQ ID NO: 482 - protein, 118 aa, synthetic construct
  REGION 1..118: note = Synthetic
EVQLVESGGGLVQPGGSLRLSCVVSGFTFGDYDMHWVRQATGRGLEWVSGIAPAGDTSYTGSVKGRFTISRENAKNSLHLQMNSLTTGDTAIYYCAREDIAVPGFDYWGQGTLVTVSS

SEQ ID NO: 483 - DNA, 24 bp, synthetic construct
  misc_feature 1..24: note = Synthetic
  source 1..24: mol_type = other DNA
ggattcaccttcggtgactacgac

SEQ ID NO: 484 - protein, 8 aa, synthetic construct
  REGION 1..8: note = Synthetic
GFTFGDYD

SEQ ID NO: 485 - DNA, 21 bp, synthetic construct
  misc_feature 1..21: note = Synthetic
  source 1..21: mol_type = other DNA
attgctcctgctggtgacaca

SEQ ID NO: 486 - protein, 7 aa, synthetic construct
  REGION 1..7: note = Synthetic
IAPAGDT

SEQ ID NO: 487 - DNA, 36 bp, synthetic construct
  misc_feature 1..36: note = Synthetic
  source 1..36: mol_type = other DNA
gctagagaggatatagcagtgcctggttttgattac

SEQ ID NO: 488 - protein, 12 aa, synthetic construct
  REGION 1..12: note = Synthetic
AREDIAVPGFDY

SEQ ID NO: 489 - DNA, 324 bp, synthetic construct
  misc_feature 1..324: note = Synthetic
  source 1..324: mol_type = other DNA
gaaatagtgatgacgcagtctccagccaccctgtctgtgtctccaggggaacgaggcaccctctcctgcagggccagtcagagtgttagcagcaacttagcctggtaccagcagaaacctggccaggctcccagactcctcatctatggtgcatccacgagggccactggcttcccagccaggttcagtggcagtgggtctgggacagagttcactctcaccatcagcagcctgcagtctgaagattttgcagtttattactgtcagcagtataataagtggcctccgttcactttcggccctgggaccaaagtggatttcaaa

SEQ ID NO: 490 - protein, 108 aa, synthetic construct
  REGION 1..108: note = Synthetic
EIVMTQSPATLSVSPGERGTLSCRASQSVSSNLAWYQQKPGQAPRLLIYGASTRATGFPARFSGSGSGTEFTLTISSLQSEDFAVYYCQQYNKWPPFTFGPGTKVDFK

SEQ ID NO: 491 - DNA, 18 bp, synthetic construct
  misc_feature 1..18: note = Synthetic
  source 1..18: mol_type = other DNA
cagagtgttagcagcaac

SEQ ID NO: 492 - protein, 6 aa, synthetic construct
  REGION 1..6: note = Synthetic
QSVSSN

SEQ ID NO: 493-494 - skipped (2 entries)

SEQ ID NO: 495 - DNA, 30 bp, synthetic construct
  misc_feature 1..30: note = Synthetic
  source 1..30: mol_type = other DNA
cagcagtataataagtggcctccgttcact

SEQ ID NO: 496 - protein, 10 aa, synthetic construct
  REGION 1..10: note = Synthetic
QQYNKWPPFT

SEQ ID NO: 497 - DNA, 354 bp, synthetic construct; identical to SEQ ID NO: 481
  misc_feature 1..354: note = Synthetic
  source 1..354: mol_type = other DNA

SEQ ID NO: 498 - protein, 118 aa, synthetic construct; identical to SEQ ID NO: 482
  REGION 1..118: note = Synthetic

SEQ ID NO: 499 - DNA, 324 bp, synthetic construct
  misc_feature 1..324: note = Synthetic
  source 1..324: mol_type = other DNA
gaaatagtgatgacgcagtctccagccaccctgtctgtgtctccaggggaacgaggcaccctctcctgcagggccagtcagagtgttagcagcaacttagcctggtaccagcagaaacctggccaggctcccagactcctcatctatggtgcatccacgagggccactggcttcccagccaggttcagtggcagtgggtctgggacagagttcactctcaccatcagcagcctgcagtctgaagattttgcagtttattactgtcagcagtataataagtggcctccgttcactttcggccctgggaccaaagtggatatcaaa

SEQ ID NO: 500 - protein, 108 aa, synthetic construct
  REGION 1..108: note = Synthetic
EIVMTQSPATLSVSPGERGTLSCRASQSVSSNLAWYQQKPGQAPRLLIYGASTRATGFPARFSGSGSGTEFTLTISSLQSEDFAVYYCQQYNKWPPFTFGPGTKVDIK

SEQ ID NO: 501 - DNA, 354 bp, synthetic construct
  misc_feature 1..354: note = Synthetic
  source 1..354: mol_type = other DNA
gaggtgcagctggtggagtctgggggaggcttggtacagcctggggggtccctgagactctcctgtgcagcctctggattcaccttcggtgactacgacatgcactgggtccgccaagctacaggaaaaggtctggagtgggtctcagctattgctcctgctggtgacacatactatccaggctccgtgaagggccgattcaccatctccagagaaaatgccaagaactccttgtatcttcaaatgaacagcctgagagccggggacacggctgtgtattactgtgctagagaggatatagcagtgcctggttttgattactggggccaaggaaccctggtcaccgtctcctca

SEQ ID NO: 502 - protein, 118 aa, synthetic construct
  REGION 1..118: note = Synthetic
EVQLVESGGGLVQPGGSLRLSCAASGFTFGDYDMHWVRQATGKGLEWVSAIAPAGDTYYPGSVKGRFTISRENAKNSLYLQMNSLRAGDTAVYYCAREDIAVPGFDYWGQGTLVTVSS

SEQ ID NO: 503 - DNA, 324 bp, synthetic construct
  misc_feature 1..324: note = Synthetic
  source 1..324: mol_type = other DNA
gaaatagtgatgacgcagtctccagccaccctgtctgtgtctccaggggaaagagccaccctctcctgcagggccagtcagagtgttagcagcaacttagcctggtaccagcagaaacctggccaggctcccaggctcctcatctatggtgcatccaccagggccactggtatcccagccaggttcagtggcagtgggtctgggacagagttcactctcaccatcagcagcctgcagtctgaagattttgcagtttattactgtcagcagtataataagtggcctccgttcactttcggccctgggaccaaagtggatatcaaa

SEQ ID NO: 504 - protein, 108 aa, synthetic construct
  REGION 1..108: note = Synthetic
EIVMTQSPATLSVSPGERATLSCRASQSVSSNLAWYQQKPGQAPRLLIYGASTRATGIPARFSGSGSGTEFTLTISSLQSEDFAVYYCQQYNKWPPFTFGPGTKVDIK

SEQ ID NO: 505 - DNA, 378 bp, synthetic construct
  misc_feature 1..378: note = Synthetic
  source 1..378: mol_type = other DNA
caaattctgctggtgcaatctggacctgaggtgaaggagcctggggcctcagtgaaggtctcctgcaaggcttctggttacacctttaccaactacgctatcagctgggtgcgacaggtccctggacaagggcttgagtggatgggatgggtcagcgcttacaatggtcacacaaactatgcacatgaagtccagggcagagtcaccatgaccacagacacatccacgaccacagcctacatggagctgaggagcctgagatctgacgacacggccatgtattactgtgcgagagggggtgtagtcgtgccagttgctccccacttctacaacggtatggacgtctggggccaagggaccacggtcaccgtctcctca

SEQ ID NO: 506 - protein, 126 aa, synthetic construct
  REGION 1..126: note = Synthetic
QILLVQSGPEVKEPGASVKVSCKASGYTFTNYAISWVRQVPGQGLEWMGWVSAYNGHTNYAHEVQGRVTMTTDTSTTTAYMELRSLRSDDTAMYYCARGGVVVPVAPHFYNGMDVWGQGTTVTVSS

SEQ ID NO: 507 - DNA, 24 bp, synthetic construct
  misc_feature 1..24: note = Synthetic
  source 1..24: mol_type = other DNA
ggttacacctttaccaactacgct

SEQ ID NO: 508 - protein, 8 aa, synthetic construct
  REGION 1..8: note = Synthetic
GYTFTNYA

SEQ ID NO: 509 - DNA, 24 bp, synthetic construct
  misc_feature 1..24: note = Synthetic
  source 1..24: mol_type = other DNA
gtcagcgcttacaatggtcacaca

SEQ ID NO: 510 - protein, 8 aa, synthetic construct
  REGION 1..8: note = Synthetic
VSAYNGHT

SEQ ID NO: 511 - DNA, 57 bp, synthetic construct
  misc_feature 1..57: note = Synthetic
  source 1..57: mol_type = other DNA
gcgagagggggtgtagtcgtgccagttgctccccacttctacaacggtatggacgtc

SEQ ID NO: 512 - protein, 19 aa, synthetic construct
  REGION 1..19: note = Synthetic
ARGGVVVPVAPHFYNGMDV

SEQ ID NO: 513 - DNA, 336 bp, synthetic construct
  misc_feature 1..336: note = Synthetic
  source 1..336: mol_type = other DNA
gatattgtgatgactcagtttccactctccctgcccgtcacccctggagagccggcctccatctcctgcaggtctagtcagagcctcctgcatattaatgaatacaactatttggattggtacctaaagaagccagggcagtctccacagctcctgatctatttgggttttaatcgggcctccggggtccctgacaggttcagtggcagtggatcaggcacagattttacactgaaaatcagcagagtggaggctgaggatgttggggtctattactgcatgcaagctcttcaaactccgtggacgttaggccaagggaccaaggtggaaatcaaa

SEQ ID NO: 514 - protein, 112 aa, synthetic construct
  REGION 1..112: note = Synthetic
DIVMTQFPLSLPVTPGEPASISCRSSQSLLHINEYNYLDWYLKKPGQSPQLLIYLGFNRASGVPDRFSGSGSGTDFTLKISRVEAEDVGVYYCMQALQTPWTLGQGTKVEIK

SEQ ID NO: 515 - DNA, 33 bp, synthetic construct
  misc_feature 1..33: note = Synthetic
  source 1..33: mol_type = other DNA
cagagcctcctgcatattaatgaatacaactat

SEQ ID NO: 516 - protein, 11 aa, synthetic construct
  REGION 1..11: note = Synthetic
QSLLHINEYNY

SEQ ID NO: 517-518 - skipped (2 entries)

SEQ ID NO: 519 - DNA, 27 bp, synthetic construct
  misc_feature 1..27: note = Synthetic
  source 1..27: mol_type = other DNA
atgcaagctcttcaaactccgtggacg

SEQ ID NO: 520 - protein, 9 aa, synthetic construct
  REGION 1..9: note = Synthetic
MQALQTPWT

SEQ ID NO: 521 - DNA, 378 bp, synthetic construct
  misc_feature 1..378: note = Synthetic
  source 1..378: mol_type = other DNA
caggttcagctggtgcagtctggacctgaggtgaaggagcctggggcctcagtgaaggtctcctgcaaggcttctggttacacctttaccaactacgctatcagctgggtgcgacaggtccctggacaagggcttgagtggatgggatgggtcagcgcttacaatggtcacacaaactatgcacatgaagtccagggcagagtcaccatgaccacagacacatccacgaccacagcctacatggagctgaggagcctgagatctgacgacacggccatgtattactgtgcgagagggggtgtagtcgtgccagttgctccccacttctacaacggtatggacgtctggggccaagggaccacggtcaccgtctcctca

SEQ ID NO: 522 - protein, 126 aa, synthetic construct
  REGION 1..126: note = Synthetic
QVQLVQSGPEVKEPGASVKVSCKASGYTFTNYAISWVRQVPGQGLEWMGWVSAYNGHTNYAHEVQGRVTMTTDTSTTTAYMELRSLRSDDTAMYYCARGGVVVPVAPHFYNGMDVWGQGTTVTVSS

SEQ ID NO: 523 - DNA, 336 bp, synthetic construct
  misc_feature 1..336: note = Synthetic
  source 1..336: mol_type = other DNA
gatattgtgatgactcagtctccactctccctgcccgtcacccctggagagccggcctccatctcctgcaggtctagtcagagcctcctgcatattaatgaatacaactatttggattggtacctaaagaagccagggcagtctccacagctcctgatctatttgggttttaatcgggcctccggggtccctgacaggttcagtggcagtggatcaggcacagattttacactgaaaatcagcagagtggaggctgaggatgttggggtctattactgcatgcaagctcttcaaactccgtggacgttaggccaagggaccaaggtggaaatcaaa

SEQ ID NO: 524 - protein, 112 aa, synthetic construct
  REGION 1..112: note = Synthetic
DIVMTQSPLSLPVTPGEPASISCRSSQSLLHINEYNYLDWYLKKPGQSPQLLIYLGFNRASGVPDRFSGSGSGTDFTLKISRVEAEDVGVYYCMQALQTPWTLGQGTKVEIK

SEQ ID NO: 525 - DNA, 378 bp, synthetic construct
  misc_feature 1..378: note = Synthetic
  source 1..378: mol_type = other DNA
caggttcagctggtgcagtctggagctgaggtgaagaagcctggggcctcagtgaaggtctcctgcaaggcttctggttacacctttaccaactacgctatcagctgggtgcgacaggcccctggacaagggcttgagtggatgggatgggtcagcgcttacaatggtcacacaaactatgcacagaagctccagggcagagtcaccatgaccacagacacatccacgagcacagcctacatggagctgaggagcctgagatctgacgacacggccgtgtattactgtgcgagagggggtgtagtcgtgccagttgctccccacttctacaacggtatggacgtctgggggcaagggaccacggtcaccgtctcctca

SEQ ID NO: 526 - protein, 126 aa, synthetic construct
  REGION 1..126: note = Synthetic
QVQLVQSGAEVKKPGASVKVSCKASGYTFTNYAISWVRQAPGQGLEWMGWVSAYNGHTNYAQKLQGRVTMTTDTSTSTAYMELRSLRSDDTAVYYCARGGVVVPVAPHFYNGMDVWGQGTTVTVSS

SEQ ID NO: 527 - DNA, 336 bp, synthetic construct
  misc_feature 1..336: note = Synthetic
  source 1..336: mol_type = other DNA
gatattgtgatgactcagtctccactctccctgcccgtcacccctggagagccggcctccatctcctgcaggtctagtcagagcctcctgcatattaatgaatacaactatttggattggtacctgcagaagccagggcagtctccacagctcctgatctatttgggttctaatcgggcctccggggtccctgacaggttcagtggcagtggatcaggcacagattttacactgaaaatcagcagagtggaggctgaggatgttggggtttattactgcatgcaagctcttcaaactccgtggacgttcggccaagggaccaaggtggaaatcaaa

SEQ ID NO: 528 - protein, 112 aa, synthetic construct
  REGION 1..112: note = Synthetic
DIVMTQSPLSLPVTPGEPASISCRSSQSLLHINEYNYLDWYLQKPGQSPQLLIYLGSNRASGVPDRFSGSGSGTDFTLKISRVEAEDVGVYYCMQALQTPWTFGQGTKVEIK

SEQ ID NO: 529 - DNA, 351 bp, synthetic construct
  misc_feature 1..351: note = Synthetic
  source 1..351: mol_type = other DNA
gaggtgcagctggtggagtctgggggaggcttggtacagcctggggggtccctgagactctcctgtgcagcctctggattcaccctaagtagctacgacatgcactgggtccgccaagcaacaggaaaaggtctggagtgggtctcagctattggcagtactggtgacacatactatacaggctccgtgatgggccgattcaccatctccagagacgctgccaaaaactccttctatcttgaaatgaacagcctgagagtcggggacacggctgtatattactgtgcaagagagggaataagaacaccctatgattattggggccagggagcccgggtcaccgtctcctca

SEQ ID NO: 530 - protein, 117 aa, synthetic construct
  REGION 1..117: note = Synthetic
EVQLVESGGGLVQPGGSLRLSCAASGFTLSSYDMHWVRQATGKGLEWVSAIGSTGDTYYTGSVMGRFTISRDAAKNSFYLEMNSLRVGDTAVYYCAREGIRTPYDYWGQGARVTVSS

SEQ ID NO: 531 - DNA, 24 bp, synthetic construct
  misc_feature 1..24: note = Synthetic
  source 1..24: mol_type = other DNA
ggattcaccctaagtagctacgac

SEQ ID NO: 532 - protein, 8 aa, synthetic construct
  REGION 1..8: note = Synthetic
GFTLSSYD

SEQ ID NO: 533 - DNA, 21 bp, synthetic construct
  misc_feature 1..21: note = Synthetic
  source 1..21: mol_type = other DNA
attggcagtactggtgacaca

SEQ ID NO: 534 - protein, 7 aa, synthetic construct
  REGION 1..7: note = Synthetic
IGSTGDT

SEQ ID NO: 535 - DNA, 33 bp, synthetic construct
  misc_feature 1..33: note = Synthetic
  source 1..33: mol_type = other DNA
gcaagagagggaataagaacaccctatgattat

SEQ ID NO: 536 - protein, 11 aa, synthetic construct
  REGION 1..11: note = Synthetic
AREGIRTPYDY

SEQ ID NO: 537 - DNA, 324 bp, synthetic construct
  misc_feature 1..324: note = Synthetic
  source 1..324: mol_type = other DNA
gaaatagtgatgacgcagtctccagccaccctgtctgtgtctccaggggaaagagccaccctctcctgcagggccagtcagagtgttagcagcaatgtagcctggtaccagcagaaacctggccaggctcccaggctcctcatctatggtgcatccaccagggccactggtatcccagccaggttcagtggcagtgggtctgggacagaattcactctcaccatcagcagcctgcagtctgaagattttgcagtttattactgtcagcagtataataattggcctccattcactttcggccctgggaccaaagtggatatcaaa

SEQ ID NO: 538 - protein, 108 aa, synthetic construct
  REGION 1..108: note = Synthetic
EIVMTQSPATLSVSPGERATLSCRASQSVSSNVAWYQQKPGQAPRLLIYGASTRATGIPARFSGSGSGTEFTLTISSLQSEDFAVYYCQQYNNWPPFTFGPGTKVDIK

SEQ ID NO: 539 - DNA, 18 bp, synthetic construct
  misc_feature 1..18: note = Synthetic
  source 1..18: mol_type = other DNA
cagagtgttagcagcaat

SEQ ID NO: 540 - protein, 6 aa, synthetic construct
  REGION 1..6: note = Synthetic
QSVSSN

SEQ ID NO: 541-542 - skipped (2 entries)

SEQ ID NO: 543 - DNA, 30 bp, synthetic construct
  misc_feature 1..30: note = Synthetic
  source 1..30: mol_type = other DNA
cagcagtataataattggcctccattcact

SEQ ID NO: 544 - protein, 10 aa, synthetic construct
  REGION 1..10: note = Synthetic
QQYNNWPPFT

SEQ ID NO: 545 - DNA, 351 bp, synthetic construct
  misc_feature 1..351: note = Synthetic
  source 1..351: mol_type = other DNA
gaggtgcagctggtggagtctgggggaggcttggtacagcctggggggtccctgagactctcctgtgcagcctctggattcaccctaagtagctacgacatgcactgggtccgccaagcaacaggaaaaggtctggagtgggtctcagctattggcagtactggtgacacatactatacaggctccgtgatgggccgattcaccatctccagagacgctgccaaaaactccttctatcttgaaatgaacagcctgagagtcggggacacggctgtatattactgtgcaagagagggaataagaacaccctatgattattggggccagggaaccctggtcaccgtctcctca

SEQ ID NO: 546 - protein, 117 aa, synthetic construct
  REGION 1..117: note = Synthetic
EVQLVESGGGLVQPGGSLRLSCAASGFTLSSYDMHWVRQATGKGLEWVSAIGSTGDTYYTGSVMGRFTISRDAAKNSFYLEMNSLRVGDTAVYYCAREGIRTPYDYWGQGTLVTVSS

SEQ ID NO: 547 - DNA, 324 bp, synthetic construct; identical to SEQ ID NO: 537
  misc_feature 1..324: note = Synthetic
  source 1..324: mol_type = other DNA

SEQ ID NO: 548 - protein, 108 aa, synthetic construct; identical to SEQ ID NO: 538
  REGION 1..108: note = Synthetic

SEQ ID NO: 549 - DNA, 351 bp, synthetic construct
  misc_feature 1..351: note = Synthetic
  source 1..351: mol_type = other DNA
gaggtgcagctggtggagtctgggggaggcttggtacagcctggggggtccctgagactctcctgtgcagcctctggattcaccctaagtagctacgacatgcactgggtccgccaagctacaggaaaaggtctggagtgggtctcagctattggcagtactggtgacacatactatccaggctccgtgaagggccgattcaccatctccagagaaaatgccaagaactccttgtatcttcaaatgaacagcctgagagccggggacacggctgtgtattactgtgcaagagagggaataagaacaccctatgattattggggccaaggaaccctggtcaccgtctcctca

SEQ ID NO: 550 - protein, 117 aa, synthetic construct
  REGION 1..117: note = Synthetic
EVQLVESGGGLVQPGGSLRLSCAASGFTLSSYDMHWVRQATGKGLEWVSAIGSTGDTYYPGSVKGRFTISRENAKNSLYLQMNSLRAGDTAVYYCAREGIRTPYDYWGQGTLVTVSS

SEQ ID NO: 551 - DNA, 324 bp, synthetic construct
  misc_feature 1..324: note = Synthetic
  source 1..324: mol_type = other DNA
gaaatagtgatgacgcagtctccagccaccctgtctgtgtctccaggggaaagagccaccctctcctgcagggccagtcagagtgttagcagcaatttagcctggtaccagcagaaacctggccaggctcccaggctcctcatctatggtgcatccaccagggccactggtatcccagccaggttcagtggcagtgggtctgggacagagttcactctcaccatcagcagcctgcagtctgaagattttgcagtttattactgtcagcagtataataattggcctccattcactttcggccctgggaccaaagtggatatcaaa

SEQ ID NO: 552 - protein, 108 aa, synthetic construct; identical to SEQ ID NO: 24
  REGION 1..108: note = Synthetic

SEQ ID NO: 553 - DNA, 351 bp, synthetic construct; identical to SEQ ID NO: 529
  misc_feature 1..351: note = Synthetic
  source 1..351: mol_type = other DNA

SEQ ID NO: 554 - protein, 117 aa, synthetic construct; identical to SEQ ID NO: 530
  REGION 1..117: note = Synthetic

SEQ ID NO: 555 - DNA, 24 bp, synthetic construct
  misc_feature 1..24: note = Synthetic
  source 1..24: mol_type = other DNA
ggattcaccctaagtagctacgac

SEQ ID NO: 556 - protein, 8 aa, synthetic construct
  REGION 1..8: note = Synthetic
GFTLSSYD

SEQ ID NO: 557 - DNA, 21 bp, synthetic construct
  misc_feature 1..21: note = Synthetic
  source 1..21: mol_type = other DNA
attggcagtactggtgacaca

SEQ ID NO: 558 - protein, 7 aa, synthetic construct
  REGION 1..7: note = Synthetic
IGSTGDT

SEQ ID NO: 559 - DNA, 33 bp, synthetic construct; identical to SEQ ID NO: 535
  misc_feature 1..33: note = Synthetic
  source 1..33: mol_type = other DNA

SEQ ID NO: 560 - protein, 11 aa, synthetic construct
  REGION 1..11: note = Synthetic
AREGIRTPYDY

SEQ ID NO: 561 - DNA, 324 bp, synthetic construct; identical to SEQ ID NO: 537
  misc_feature 1..324: note = Synthetic
  source 1..324: mol_type = other DNA

SEQ ID NO: 562 - protein, 108 aa, synthetic construct; identical to SEQ ID NO: 538
  REGION 1..108: note = Synthetic

SEQ ID NO: 563 - DNA, 18 bp, synthetic construct
  misc_feature 1..18: note = Synthetic
  source 1..18: mol_type = other DNA
cagagtgttagcagcaat

SEQ ID NO: 564 - protein, 6 aa, synthetic construct
  REGION 1..6: note = Synthetic
QSVSSN

SEQ ID NO: 565-566 - skipped (2 entries)

SEQ ID NO: 567 - DNA, 30 bp, synthetic construct; identical to SEQ ID NO: 543
  misc_feature 1..30: note = Synthetic
  source 1..30: mol_type = other DNA

SEQ ID NO: 568 - protein, 10 aa, synthetic construct
  REGION 1..10: note = Synthetic
QQYNNWPPFT

SEQ ID NO: 569 - DNA, 351 bp, synthetic construct; identical to SEQ ID NO: 545
  misc_feature 1..351: note = Synthetic
  source 1..351: mol_type = other DNA

SEQ ID NO: 570 - protein, 117 aa, synthetic construct; identical to SEQ ID NO: 546
  REGION 1..117: note = Synthetic

SEQ ID NO: 571 - DNA, 324 bp, synthetic construct; identical to SEQ ID NO: 537
  misc_feature 1..324: note = Synthetic
  source 1..324: mol_type = other DNA

SEQ ID NO: 572 - protein, 108 aa, synthetic construct; identical to SEQ ID NO: 538
  REGION 1..108: note = Synthetic

SEQ ID NO: 573 - DNA, 351 bp, synthetic construct; identical to SEQ ID NO: 549
  misc_feature 1..351: note = Synthetic
  source 1..351: mol_type = other DNA

SEQ ID NO: 574 - protein, 117 aa, synthetic construct; identical to SEQ ID NO: 550
  REGION 1..117: note = Synthetic

SEQ ID NO: 575 - DNA, 324 bp, synthetic construct; identical to SEQ ID NO: 551
  misc_feature 1..324: note = Synthetic
  source 1..324: mol_type = other DNA

SEQ ID NO: 576 - protein, 108 aa, synthetic construct; identical to SEQ ID NO: 24
  REGION 1..108: note = Synthetic

SEQ ID NO: 577 - DNA, 363 bp, synthetic construct
  misc_feature 1..363: note = Synthetic
  source 1..363: mol_type = other DNA
gaagtgcagctggtggagtctgggggaggcttggtacagcctggcaggtccctgagactctcctgtgcagcctctggattcacctttgatgattatgccatgcactgggtccggcaagctccagggaagggcctggagtgggtctcaggtattaattggaacagtggtagcataggctatgcggactctgtgaagggccgattcaccatctccagagacaacgccaagcactccctgtatctgcaaatgaacagtctgagacctgaggacacggccttgtattactgtgtaaaagaggtgactacgggatactactacggtatggacgtctggggccaagggaccacggtcaccgtctcctca

SEQ ID NO: 578 - protein, 121 aa, synthetic construct
  REGION 1..121: note = Synthetic
EVQLVESGGGLVQPGRSLRLSCAASGFTFDDYAMHWVRQAPGKGLEWVSGINWNSGSIGYADSVKGRFTISRDNAKHSLYLQMNSLRPEDTALYYCVKEVTTGYYYGMDVWGQGTTVTVSS

SEQ ID NO: 579 - DNA, 24 bp, synthetic construct
  misc_feature 1..24: note = Synthetic
  source 1..24: mol_type = other DNA
ggattcacctttgatgattatgcc

SEQ ID NO: 580 - protein, 8 aa, synthetic construct
  REGION 1..8: note = Synthetic
GFTFDDYA

SEQ ID NO: 581 - DNA, 24 bp, synthetic construct
  misc_feature 1..24: note = Synthetic
  source 1..24: mol_type = other DNA
attaattggaacagtggtagcata

SEQ ID NO: 582 - protein, 8 aa, synthetic construct
  REGION 1..8: note = Synthetic
INWNSGSI

SEQ ID NO: 583 - DNA, 42 bp, synthetic construct
  misc_feature 1..42: note = Synthetic
  source 1..42: mol_type = other DNA
gtaaaagaggtgactacgggatactactacggtatggacgtc

SEQ ID NO: 584 - protein, 14 aa, synthetic construct
  REGION 1..14: note = Synthetic
VKEVTTGYYYGMDV

SEQ ID NO: 585 - DNA, 321 bp, synthetic construct
  misc_feature 1..321: note = Synthetic
  source 1..321: mol_type = other DNA
gacatccagttgacccagtctccatccttcctgtctgcatctgtaggagacagagtcaccatcacttgctgggccagtcagggcattagcagttatttagcctggtatcagaaaaaaccagggaaagcccctaacctcctgatctatgatgcatccactttgcaaagtggggtcccatcaaggttcagcggcagtggatctgggacagaattcactctcacactcagcagcctgcagcctgaagattttgcaacttattactgtcaacagcttaatatttacccattcactttcggccctgggaccaaagtggatatcaaa

SEQ ID NO: 586 - protein, 107 aa, synthetic construct
  REGION 1..107: note = Synthetic
DIQLTQSPSFLSASVGDRVTITCWASQGISSYLAWYQKKPGKAPNLLIYDASTLQSGVPSRFSGSGSGTEFTLTLSSLQPEDFATYYCQQLNIYPFTFGPGTKVDIK

SEQ ID NO: 587 - DNA, 18 bp, synthetic construct
  misc_feature 1..18: note = Synthetic
  source 1..18: mol_type = other DNA
cagggcattagcagttat

SEQ ID NO: 588 - protein, 6 aa, synthetic construct
  REGION 1..6: note = Synthetic
QGISSY

SEQ ID NO: 589-590 - skipped (2 entries)

SEQ ID NO: 591 - DNA, 27 bp, synthetic construct
  misc_feature 1..27: note = Synthetic
  source 1..27: mol_type = other DNA
caacagcttaatatttacccattcact

SEQ ID NO: 592 - protein, 9 aa, synthetic construct
  REGION 1..9: note = Synthetic
QQLNIYPFT

SEQ ID NO: 593 - DNA, 363 bp, synthetic construct; identical to SEQ ID NO: 577
  misc_feature 1..363: note = Synthetic
  source 1..363: mol_type = other DNA

SEQ ID NO: 594 - protein, 121 aa, synthetic construct; identical to SEQ ID NO: 578
  REGION 1..121: note = Synthetic

SEQ ID NO: 595 - DNA, 321 bp, synthetic construct; identical to SEQ ID NO: 585
  misc_feature 1..321: note = Synthetic
  source 1..321: mol_type = other DNA

SEQ ID NO: 596 - protein, 107 aa, synthetic construct; identical to SEQ ID NO: 586
  REGION 1..107: note = Synthetic

SEQ ID NO: 597 - DNA, 363 bp, synthetic construct
  misc_feature 1..363: note = Synthetic
  source 1..363: mol_type = other DNA
gaagtgcagctggtggagtctgggggaggcttggtacagcctggcaggtccctgagactctcctgtgcagcctctggattcacctttgatgattatgccatgcactgggtccggcaagctccagggaagggcctggagtgggtctcaggtattaattggaacagtggtagcataggctatgcggactctgtgaagggccgattcaccatctccagagacaacgccaagaactccctgtatctgcaaatgaacagtctgagagctgaggacacggccttgtattactgtgtaaaagaggtgactacgggatactactacggtatggacgtctgggggcaagggaccacggtcaccgtctcctca

SEQ ID NO: 598 - protein, 121 aa, synthetic construct
  REGION 1..121: note = Synthetic
EVQLVESGGGLVQPGRSLRLSCAASGFTFDDYAMHWVRQAPGKGLEWVSGINWNSGSIGYADSVKGRFTISRDNAKNSLYLQMNSLRAEDTALYYCVKEVTTGYYYGMDVWGQGTTVTVSS

SEQ ID NO: 599 - DNA, 321 bp, synthetic construct
  misc_feature 1..321: note = Synthetic
  source 1..321: mol_type = other DNA
gacatccagttgacccagtctccatccttcctgtctgcatctgtaggagacagagtcaccatcacttgccgggccagtcagggcattagcagttatttagcctggtatcagcaaaaaccagggaaagcccctaagctcctgatctatgatgcatccactttgcaaagtggggtcccatcaaggttcagcggcagtggatctgggacagaattcactctcacaatcagcagcctgcagcctgaagattttgcaacttattactgtcaacagcttaatatttacccattcactttcggccctgggaccaaagtggatatcaaa

SEQ ID NO: 600 - protein, 107 aa, synthetic construct
  REGION 1..107: note = Synthetic
DIQLTQSPSFLSASVGDRVTITCRASQGISSYLAWYQQKPGKAPKLLIYDASTLQSGVPSRFSGSGSGTEFTLTISSLQPEDFATYYCQQLNIYPFTFGPGTKVDIK

SEQ ID NO: 601 - DNA, 366 bp, synthetic construct
  misc_feature 1..366: note = Synthetic
  source 1..366: mol_type = other DNA
gaggtgcagttgttggagtctgggggaggcttggtacagcctggggggtccctgagactctcctgtgcagcctctggattcacgtttagtagctatgccatgaactgggtccgccaggctccagggaaggggctggattgggtctcaggtatcagtggtaatggtggtagcacctactacgcagactccgtgaagggccggttcaccatctccagagacatttccaagaacacgctgtatgtgcaaatgcacagcctgagagtcgaggacacggccgtttactactgtgcgaaagcccgttattacgatttttggggggggaatttcgatctctggggccgtggcacccaggtcactgtctcctca

SEQ ID NO: 602 - protein, 122 aa, synthetic construct
  REGION 1..122: note = Synthetic
EVQLLESGGGLVQPGGSLRLSCAASGFTFSSYAMNWVRQAPGKGLDWVSGISGNGGSTYYADSVKGRFTISRDISKNTLYVQMHSLRVEDTAVYYCAKARYYDFWGGNFDLWGRGTQVTVSS

SEQ ID NO: 603 - DNA, 24 bp, synthetic construct
  misc_feature 1..24: note = Synthetic
  source 1..24: mol_type = other DNA
ggattcacgtttagtagctatgcc

SEQ ID NO: 604 - protein, 8 aa, synthetic construct
  REGION 1..8: note = Synthetic
GFTFSSYA

SEQ ID NO: 605 - DNA, 24 bp, synthetic construct
  misc_feature 1..24: note = Synthetic
  source 1..24: mol_type = other DNA
atcagtggtaatggtggtagcacc

SEQ ID NO: 606 - protein, 8 aa, synthetic construct
  REGION 1..8: note = Synthetic
ISGNGGST

SEQ ID NO: 607 - DNA, 45 bp, synthetic construct
  misc_feature 1..45: note = Synthetic
  source 1..45: mol_type = other DNA
gcgaaagcccgttattacgatttttggggggggaatttcgatctc

SEQ ID NO: 608 - protein, 15 aa, synthetic construct
  REGION 1..15: note = Synthetic
AKARYYDFWGGNFDL

SEQ ID NO: 609 - DNA, 324 bp, synthetic construct
  misc_feature 1..324: note = Synthetic
  source 1..324: mol_type = other DNA
gaaattgtgttgacgcagtctccaggcaccctgtctttgtctccaggggaaagagccaccctctcctgcagggccagtcagagtgttagcatcaggtacttagcctggtatcagcagaaacctggccaggctcccaggctcctcatctatggtgcatccagcagggccactggcatcccagacaggttcagtgtcagtgtgtctgggacagacttcactctcaccatcactagactggagcctgaagattttgcagtctattactgtcagcaatatggtagttcaccgctcactttcggcggagggaccaaggtggagatcaaa

SEQ ID NO: 610 - protein, 108 aa, synthetic construct
  REGION 1..108: note = Synthetic
EIVLTQSPGTLSLSPGERATLSCRASQSVSIRYLAWYQQKPGQAPRLLIYGASSRATGIPDRFSVSVSGTDFTLTITRLEPEDFAVYYCQQYGSSPLTFGGGTKVEIK

SEQ ID NO: 611 - DNA, 21 bp, synthetic construct
  misc_feature 1..21: note = Synthetic
  source 1..21: mol_type = other DNA
cagagtgttagcatcaggtac

SEQ ID NO: 612 - protein, 7 aa, synthetic construct
  REGION 1..7: note = Synthetic
QSVSIRY

SEQ ID NO: 613-614 - skipped (2 entries)

SEQ ID NO: 615 - DNA, 27 bp, synthetic construct
  misc_feature 1..27: note = Synthetic
  source 1..27: mol_type = other DNA
cagcaatatggtagttcaccgctcact

SEQ ID NO: 616 - protein, 9 aa, synthetic construct
  REGION 1..9: note = Synthetic
QQYGSSPLT

SEQ ID NO: 617 - DNA, 366 bp, synthetic construct
  misc_feature 1..366: note = Synthetic
  source 1..366: mol_type = other DNA
gaggtgcagttgttggagtctgggggaggcttggtacagcctggggggtccctgagactctcctgtgcagcctctggattcacgtttagtagctatgccatgaactgggtccgccaggctccagggaaggggctggattgggtctcaggtatcagtggtaatggtggtagcacctactacgcagactccgtgaagggccggttcaccatctccagagacatttccaagaacacgctgtatgtgcaaatgcacagcctgagagtcgaggacacggccgtttactactgtgcgaaagcccgttattacgatttttggggggggaatttcgatctctggggccgtggcaccctggtcactgtctcctca

SEQ ID NO: 618 - protein, 122 aa, synthetic construct
  REGION 1..122: note = Synthetic
EVQLLESGGGLVQPGGSLRLSCAASGFTFSSYAMNWVRQAPGKGLDWVSGISGNGGSTYYADSVKGRFTISRDISKNTLYVQMHSLRVEDTAVYYCAKARYYDFWGGNFDLWGRGTLVTVSS

SEQ ID NO: 619 - DNA, 324 bp, synthetic construct; identical to SEQ ID NO: 609
  misc_feature 1..324: note = Synthetic
  source 1..324: mol_type = other DNA

SEQ ID NO: 620 - protein, 108 aa, synthetic construct; identical to SEQ ID NO: 610
  REGION 1..108: note = Synthetic

SEQ ID NO: 621 - DNA, 366 bp, synthetic construct
  misc_feature 1..366: note = Synthetic
  source 1..366: mol_type = other DNA
gaggtgcagctgttggagtctgggggaggcttggtacagcctggggggtccctgagactctcctgtgcagcctctggattcacgtttagtagctatgccatgagctgggtccgccaggctccagggaaggggctggagtgggtctcagctatcagtggtaatggtggtagcacctactacgcagactccgtgaagggccggttcaccatctccagagacaattccaagaacacgctgtatctgcaaatgaacagcctgagagccgaggacacggccgtatattactgtgcgaaagcccgttattacgatttttggggggggaatttcgatctctggggccgtggcaccctggtcactgtctcctca

SEQ ID NO: 622 - protein, 122 aa, synthetic construct
  REGION 1..122: note = Synthetic
EVQLLESGGGLVQPGGSLRLSCAASGFTFSSYAMSWVRQAPGKGLEWVSAISGNGGSTYYADSVKGRFTISRDNSKNTLYLQMNSLRAEDTAVYYCAKARYYDFWGGNFDLWGRGTLVTVSS

SEQ ID NO: 623 - DNA, 324 bp, synthetic construct
  misc_feature 1..324: note = Synthetic
  source 1..324: mol_type = other DNA
gaaattgtgttgacgcagtctccaggcaccctgtctttgtctccaggggaaagagccaccctctcctgcagggccagtcagagtgttagcatcaggtacttagcctggtaccagcagaaacctggccaggctcccaggctcctcatctatggtgcatccagcagggccactggcatcccagacaggttcagtggcagtgggtctgggacagacttcactctcaccatcagcagactggagcctgaagattttgcagtgtattactgtcagcaatatggtagttcaccgctcactttcggcggagggaccaaggtggagatcaaa

SEQ ID NO: 624 - protein, 108 aa, synthetic construct
  REGION 1..108: note = Synthetic
EIVLTQSPGTLSLSPGERATLSCRASQSVSIRYLAWYQQKPGQAPRLLIYGASSRATGIPDRFSGSGSGTDFTLTISRLEPEDFAVYYCQQYGSSPLTFGGGTKVEIK

SEQ ID NO: 625 - DNA, 381 bp, synthetic construct
  misc_feature 1..381: note = Synthetic
  source 1..381: mol_type = other DNA
caggttcagctggtgcagtctggacctgaggtgaagaaccctggggcctcagtgaaggtctcctgcaaggcttctggttacacctttaccacctatggtatcagttgggtacgacaggcccctggacaagggcttgagtggatgggatggatcagcggttacaatggtaaaacaaacgatgcacagaagttccaggacagagtcgccatgaccacagacacatccacgagcacagcctacatggagctgaggagcctgagatctgacgacacggccatttattactgttcgagagatcgtttagtagtaccacctgccctttattattcctactacgttatggacgtctggggccaagggaccacggtcaccgtctcctca

SEQ ID NO: 626 - protein, 127 aa, synthetic construct
  REGION 1..127: note = Synthetic
QVQLVQSGPEVKNPGASVKVSCKASGYTFTTYGISWVRQAPGQGLEWMGWISGYNGKTNDAQKFQDRVAMTTDTSTSTAYMELRSLRSDDTAIYYCSRDRLVVPPALYYSYYVMDVWGQGTTVTVSS

SEQ ID NO: 627 - DNA, 24 bp, synthetic construct
  misc_feature 1..24: note = Synthetic
  source 1..24: mol_type = other DNA
ggttacacctttaccacctatggt

SEQ ID NO: 628 - protein, 8 aa, synthetic construct
  REGION 1..8: note = Synthetic
GYTFTTYG

SEQ ID NO: 629 - DNA, 24 bp, synthetic construct
  misc_feature 1..24: note = Synthetic
  source 1..24: mol_type = other DNA
atcagcggttacaatggtaaaaca

SEQ ID NO: 630 - protein, 8 aa, synthetic construct
  REGION 1..8: note = Synthetic
ISGYNGKT

SEQ ID NO: 631 - DNA, 60 bp, synthetic construct
  misc_feature 1..60: note = Synthetic
  source 1..60: mol_type = other DNA
tcgagagatcgtttagtagtaccacctgccctttattattcctactacgttatggacgtc

SEQ ID NO: 632 - protein, 20 aa, synthetic construct
  REGION 1..20: note = Synthetic
SRDRLVVPPALYYSYYVMDV

SEQ ID NO: 633 - DNA, 336 bp, synthetic construct
  misc_feature 1..336: note = Synthetic
  source 1..336: mol_type = other DNA
gatgttgtgatgactcagtctccactctccctgcccgtcacccttggacagccggcctccatctcctgcaggtctagtcaaagcctcgtatacagtgatggaaacacctacttgaattggtttcagcagaggccaggtcaatctccaaggcgcctaatttataaggtttctaaccgggactctggggtcccagacagattcagcggcagtgggtcaggcactgatttcacactgaaaatcagcagggtggaggctgaggatgttggggtttattactgcatgcaaggtacacactggccgtacacttttggccaggggaccaagctggagatcaaa

SEQ ID NO: 634 - protein, 112 aa, synthetic construct; identical to SEQ ID NO: 336
  REGION 1..112: note = Synthetic

SEQ ID NO: 635 - DNA, 33 bp, synthetic construct; identical to SEQ ID NO: 323
  misc_feature 1..33: note = Synthetic
  source 1..33: mol_type = other DNA

SEQ ID NO: 636 - protein, 11 aa, synthetic construct
  REGION 1..11: note = Synthetic
QSLVYSDGNTY

SEQ ID NO: 637-638 - skipped (2 entries)

SEQ ID NO: 639 - DNA, 27 bp, synthetic construct
  misc_feature 1..27: note = Synthetic
  source 1..27: mol_type = other DNA
atgcaaggtacacactggccgtacact

SEQ ID NO: 640 - protein, 9 aa, synthetic construct
  REGION 1..9: note = Synthetic
MQGTHWPYT

SEQ ID NO: 641 - DNA, 381 bp, synthetic construct; identical to SEQ ID NO: 625
  misc_feature 1..381: note = Synthetic
  source 1..381: mol_type = other DNA

SEQ ID NO: 642 - protein, 127 aa, synthetic construct; identical to SEQ ID NO: 626
  REGION 1..127: note = Synthetic

SEQ ID NO: 643 - DNA, 336 bp, synthetic construct; identical to SEQ ID NO: 633
  misc_feature 1..336: note = Synthetic
  source 1..336: mol_type = other DNA

SEQ ID NO: 644 - protein, 112 aa, synthetic construct; identical to SEQ ID NO: 336
  REGION 1..112: note = Synthetic

SEQ ID NO: 645 - DNA, 381 bp, synthetic construct
  misc_feature 1..381: note = Synthetic
  source 1..381: mol_type = other DNA
caggttcagctggtgcagtctggagctgaggtgaagaagcctggggcctcagtgaaggtctcctgcaaggcttctggttacacctttaccacctatggtatcagctgggtgcgacaggcccctggacaagggcttgagtggatgggatggatcagcggttacaatggtaaaacaaactatgcacagaagctccagggcagagtcaccatgaccacagacacatccacgagcacagcctacatggagctgaggagcctgagatctgacgacacggccgtgtattactgttcgagagatcgtttagtagtaccacctgccctttattattcctactacgttatggacgtctgggggcaagggaccacggtcaccgtctcctca

SEQ ID NO: 646 - protein, 127 aa, synthetic construct
  REGION 1..127: note = Synthetic
QVQLVQSGAEVKKPGASVKVSCKASGYTFTTYGISWVRQAPGQGLEWMGWISGYNGKTNYAQKLQGRVTMTTDTSTSTAYMELRSLRSDDTAVYYCSRDRLVVPPALYYSYYVMDVWGQGTTVTVSS

SEQ ID NO: 647 - DNA, 336 bp, synthetic construct; identical to SEQ ID NO: 335
  misc_feature 1..336: note = Synthetic
  source 1..336: mol_type = other DNA

SEQ ID NO: 648 - protein, 112 aa, synthetic construct; identical to SEQ ID NO: 336
  REGION 1..112: note = Synthetic

SEQ ID NO: 649 - DNA, 381 bp, synthetic construct
  misc_feature 1..381: note = Synthetic
  source 1..381: mol_type = other DNA
caggttcagctggtgcagtctggacctgaggtgaagaaccctggggcctcagtgaaggtctcctgcaaggcttctggttacacctttaccacctatggtatcagttgggtacgacaggcccctggacaagggcttgagtggatgggatggatcagcggttacaatggtaaaacaaacgatgcacagaagttccaggacagagtcgccatgaccacagacacatccacgagcacagcctacatggagctgaggagcctgagatctgacgacacggccatttattactgttcgagagatcgtttagtagtaccacctgcccttaattattactactacgttatggacgtctggggccaagggaccacggtcaccgtctcctca

SEQ ID NO: 650 - protein, 127 aa, synthetic construct
  REGION 1..127: note = Synthetic
QVQLVQSGPEVKNPGASVKVSCKASGYTFTTYGISWVRQAPGQGLEWMGWISGYNGKTNDAQKFQDRVAMTTDTSTSTAYMELRSLRSDDTAIYYCSRDRLVVPPALNYYYYVMDVWGQGTTVTVSS

SEQ ID NO: 651 - DNA, 24 bp, synthetic construct
  misc_feature 1..24: note = Synthetic
  source 1..24: mol_type = other DNA
ggttacacctttaccacctatggt

SEQ ID NO: 652 - protein, 8 aa, synthetic construct
  REGION 1..8: note = Synthetic
GYTFTTYG

SEQ ID NO: 653 - DNA, 24 bp, synthetic construct
  misc_feature 1..24: note = Synthetic
  source 1..24: mol_type = other DNA
atcagcggttacaatggtaaaaca

SEQ ID NO: 654 - protein, 8 aa, synthetic construct
  REGION 1..8: note = Synthetic
ISGYNGKT

SEQ ID NO: 655 - DNA, 60 bp, synthetic construct
  misc_feature 1..60: note = Synthetic
  source 1..60: mol_type = other DNA
tcgagagatcgtttagtagtaccacctgcccttaattattactactacgttatggacgtc

SEQ ID NO: 656 - protein, 20 aa, synthetic construct
  REGION 1..20: note = Synthetic
SRDRLVVPPALNYYYYVMDV

SEQ ID NO: 657 - DNA, 336 bp, synthetic construct; identical to SEQ ID NO: 633
  misc_feature 1..336: note = Synthetic
  source 1..336: mol_type = other DNA

SEQ ID NO: 658 - protein, 112 aa, synthetic construct; identical to SEQ ID NO: 336
  REGION 1..112: note = Synthetic

SEQ ID NO: 659 - DNA, 33 bp, synthetic construct; identical to SEQ ID NO: 323
  misc_feature 1..33: note = Synthetic
  source 1..33: mol_type = other DNA

SEQ ID NO: 660 - protein, 11 aa, synthetic construct
  REGION 1..11: note = Synthetic
QSLVYSDGNTY

SEQ ID NO: 661-662 - skipped (2 entries)

SEQ ID NO: 663 - DNA, 27 bp, synthetic construct
  misc_feature 1..27: note = Synthetic
  source 1..27: mol_type = other DNA
atgcaaggtacacactggccgtacact

SEQ ID NO: 664 - protein, 9 aa, synthetic construct
  REGION 1..9: note = Synthetic
MQGTHWPYT

SEQ ID NO: 665 - DNA, 381 bp, synthetic construct; identical to SEQ ID NO: 649
  misc_feature 1..381: note = Synthetic
  source 1..381: mol_type = other DNA

SEQ ID NO: 666 - protein, 127 aa, synthetic construct; identical to SEQ ID NO: 650
  REGION 1..127: note = Synthetic

SEQ ID NO: 667 - DNA, 336 bp, synthetic construct; identical to SEQ ID NO: 633
  misc_feature 1..336: note = Synthetic
  source 1..336: mol_type = other DNA

SEQ ID NO: 668 - protein, 112 aa, synthetic construct; identical to SEQ ID NO: 336
  REGION 1..112: note = Synthetic

SEQ ID NO: 669 - DNA, 381 bp, synthetic construct
  misc_feature 1..381: note = Synthetic
  source 1..381: mol_type = other DNA
caggttcagctggtgcagtctggagctgaggtgaagaagcctggggcctcagtgaaggtctcctgcaaggcttctggttacacctttaccacctatggtatcagctgggtgcgacaggcccctggacaagggcttgagtggatgggatggatcagcggttacaatggtaaaacaaactatgcacagaagctccagggcagagtcaccatgaccacagacacatccacgagcacagcctacatggagctgaggagcctgagatctgacgacacggccgtgtattactgttcgagagatcgtttagtagtaccacctgcccttaattattactactacgttatggacgtctgggggcaagggaccacggtcaccgtctcctca

SEQ ID NO: 670 - protein, 127 aa, synthetic construct
  REGION 1..127: note = Synthetic
QVQLVQSGAEVKKPGASVKVSCKASGYTFTTYGISWVRQAPGQGLEWMGWISGYNGKTNYAQKLQGRVTMTTDTSTSTAYMELRSLRSDDTAVYYCSRDRLVVPPALNYYYYVMDVWGQGTTVTVSS

SEQ ID NO: 671 - DNA, 336 bp, synthetic construct; identical to SEQ ID NO: 335
  misc_feature 1..336: note = Synthetic
  source 1..336: mol_type = other DNA

SEQ ID NO: 672 - protein, 112 aa, synthetic construct; identical to SEQ ID NO: 336
  REGION 1..112: note = Synthetic

SEQ ID NO: 673 - DNA, 381 bp, synthetic construct
  misc_feature 1..381: note = Synthetic
  source 1..381: mol_type = other DNA
caggttcagctggtgcagtctggacctgaggtgaagaaccctggggcctcagtgaaggtctcctgcaaggcttctggttacacctttaccacctatggtatcagttgggtacgacaggcccctggacaagggcttgagtggatgggatggatcagcggttacaatggtaaaacaaacgatgcacagaagttccaggacagagtcgccatgaccacagacacatccacgagcacagcctacatggagctgaggagcctgagatctgacgacacggccatttattactgttcgagagatcgtttagtagtaccacctgccctttattattactactacgttatggacgtctggggccaagggaccacggtcaccgtctcctca

SEQ ID NO: 674 - protein, 127 aa, synthetic construct
  REGION 1..127: note = Synthetic
QVQLVQSGPEVKNPGASVKVSCKASGYTFTTYGISWVRQAPGQGLEWMGWISGYNGKTNDAQKFQDRVAMTTDTSTSTAYMELRSLRSDDTAIYYCSRDRLVVPPALYYYYYVMDVWGQGTTVTVSS

SEQ ID NO: 675 - DNA, 24 bp, synthetic construct
  misc_feature 1..24: note = Synthetic
  source 1..24: mol_type = other DNA
ggttacacctttaccacctatggt

SEQ ID NO: 676 - protein, 8 aa, synthetic construct
  REGION 1..8: note = Synthetic
GYTFTTYG

SEQ ID NO: 677 - DNA, 24 bp, synthetic construct
  misc_feature 1..24: note = Synthetic
  source 1..24: mol_type = other DNA
atcagcggttacaatggtaaaaca

SEQ ID NO: 678 - protein, 8 aa, synthetic construct
  REGION 1..8: note = Synthetic
ISGYNGKT

SEQ ID NO: 679 - DNA, 60 bp, synthetic construct
  misc_feature 1..60: note = Synthetic
  source 1..60: mol_type = other DNA
tcgagagatcgtttagtagtaccacctgccctttattattactactacgttatggacgtc

SEQ ID NO: 680 - protein, 20 aa, synthetic construct
  REGION 1..20: note = Synthetic
SRDRLVVPPALYYYYYVMDV

SEQ ID NO: 681 - DNA, 336 bp, synthetic construct; identical to SEQ ID NO: 633
  misc_feature 1..336: note = Synthetic
  source 1..336: mol_type = other DNA

SEQ ID NO: 682 - protein, 112 aa, synthetic construct; identical to SEQ ID NO: 336
  REGION 1..112: note = Synthetic

SEQ ID NO: 683 - DNA, 33 bp, synthetic construct; identical to SEQ ID NO: 323
  misc_feature 1..33: note = Synthetic
  source 1..33: mol_type = other DNA

SEQ ID NO: 684 - protein, 11 aa, synthetic construct
  REGION 1..11: note = Synthetic
QSLVYSDGNTY

SEQ ID NO: 685-686 - skipped (2 entries)

SEQ ID NO: 687 - DNA, 27 bp, synthetic construct
  misc_feature 1..27: note = Synthetic
  source 1..27: mol_type = other DNA
atgcaaggtacacactggccgtacact

SEQ ID NO: 688 - protein, 9 aa, synthetic construct
  REGION 1..9: note = Synthetic
MQGTHWPYT

SEQ ID NO: 689 - DNA, 381 bp, synthetic construct; identical to SEQ ID NO: 673
  misc_feature 1..381: note = Synthetic
  source 1..381: mol_type = other DNA

SEQ ID NO: 690 - protein, 127 aa, synthetic construct; identical to SEQ ID NO: 674
  REGION 1..127: note = Synthetic

SEQ ID NO: 691 - DNA, 336 bp, synthetic construct; identical to SEQ ID NO: 633
  misc_feature 1..336: note = Synthetic
  source 1..336: mol_type = other DNA

SEQ ID NO: 692 - protein, 112 aa, synthetic construct; identical to SEQ ID NO: 336
  REGION 1..112: note = Synthetic

SEQ ID NO: 693 - DNA, 381 bp, synthetic construct
  misc_feature 1..381: note = Synthetic
  source 1..381: mol_type = other DNA
caggttcagctggtgcagtctggagctgaggtgaagaagcctggggcctcagtgaaggtctcctgcaaggcttctggttacacctttaccacctatggtatcagctgggtgcgacaggcccctggacaagggcttgagtggatgggatggatcagcggttacaatggtaaaacaaactatgcacagaagctccagggcagagtcaccatgaccacagacacatccacgagcacagcctacatggagctgaggagcctgagatctgacgacacggccgtgtattactgttcgagagatcgtttagtagtaccacctgccctttattattactactacgttatggacgtctgggggcaagggaccacggtcaccgtctcctca

SEQ ID NO: 694 - protein, 127 aa, synthetic construct
  REGION 1..127: note = Synthetic
QVQLVQSGAEVKKPGASVKVSCKASGYTFTTYGISWVRQAPGQGLEWMGWISGYNGKTNYAQKLQGRVTMTTDTSTSTAYMELRSLRSDDTAVYYCSRDRLVVPPALYYYYYVMDVWGQGTTVTVSS

SEQ ID NO: 695 - DNA, 336 bp, synthetic construct; identical to SEQ ID NO: 335
  misc_feature 1..336: note = Synthetic
  source 1..336: mol_type = other DNA

SEQ ID NO: 696 - protein, 112 aa, synthetic construct; identical to SEQ ID NO: 336
  REGION 1..112: note = Synthetic

SEQ ID NO: 697 - DNA, 384 bp, synthetic construct; identical to SEQ ID NO: 361
  misc_feature 1..384: note = Synthetic
  source 1..384: mol_type = other DNA

SEQ ID NO: 698 - protein, 128 aa, synthetic construct; identical to SEQ ID NO: 362
  REGION 1..128: note = Synthetic

SEQ ID NO: 699 - DNA, 24 bp, synthetic construct
  misc_feature 1..24: note = Synthetic
  source 1..24: mol_type = other DNA
ggattcaccttcagtgaccactac

SEQ ID NO: 700 - protein, 8 aa, synthetic construct
  REGION 1..8: note = Synthetic
GFTFSDHY

SEQ ID NO: 701 - DNA, 24 bp, synthetic construct
  misc_feature 1..24: note = Synthetic
  source 1..24: mol_type = other DNA
attagtaatgatggtggtaccaaa

SEQ ID NO: 702 - protein, 8 aa, synthetic construct
  REGION 1..8: note = Synthetic
ISNDGGTK

SEQ ID NO: 703 - DNA, 63 bp, synthetic construct; identical to SEQ ID NO: 367
  misc_feature 1..63: note = Synthetic
  source 1..63: mol_type = other DNA

SEQ ID NO: 704 - protein, 21 aa, synthetic construct
  REGION 1..21: note = Synthetic
ARDQGYIGYDSYYYYSYGMDV

SEQ ID NO: 705 - DNA, 321 bp, synthetic construct
  misc_feature 1..321: note = Synthetic
  source 1..321: mol_type = other DNA
aaaattgtgttgacgcagtctccaggcaccctgcctttgtttccaggggaaagagccaccctctcctgtagggccagtcagagtgttaacaacaaattcttagcctggtaccagcagaaatctggccaggctcccaggctcctcatctatggtgcatccagcagggccactggcatcccagacaggttcagtggcagtgggtctgggaccgacttcactctcaccatcagcggactggagcctgaagattttgaagtgtattattgtcaagtatatggtaactcactcactttcggcggagggaccaaggtggagatcaag

SEQ ID NO: 706 - protein, 107 aa, synthetic construct
  REGION 1..107: note = Synthetic
KIVLTQSPGTLPLFPGERATLSCRASQSVNNKFLAWYQQKSGQAPRLLIYGASSRATGIPDRFSGSGSGTDFTLTISGLEPEDFEVYYCQVYGNSLTFGGGTKVEIK

SEQ ID NO: 707 - DNA, 21 bp, synthetic construct
  misc_feature 1..21: note = Synthetic
  source 1..21: mol_type = other DNA
cagagtgttaacaacaaattc

SEQ ID NO: 708 - protein, 7 aa, synthetic construct
  REGION 1..7: note = Synthetic
QSVNNKF

SEQ ID NO: 709-710 - skipped (2 entries)

SEQ ID NO: 711 - DNA, 24 bp, synthetic construct
  misc_feature 1..24: note = Synthetic
  source 1..24: mol_type = other DNA
caagtatatggtaactcactcact

SEQ ID NO: 712 - protein, 8 aa, synthetic construct
  REGION 1..8: note = Synthetic
QVYGNSLT

SEQ ID NO: 713 - DNA, 384 bp, synthetic construct; identical to SEQ ID NO: 377
  misc_feature 1..384: note = Synthetic
  source 1..384: mol_type = other DNA

SEQ ID NO: 714 - protein, 128 aa, synthetic construct; identical to SEQ ID NO: 378
  REGION 1..128: note = Synthetic

SEQ ID NO: 715 - DNA, 321 bp, synthetic construct
  misc_feature 1..321: note = Synthetic
  source 1..321: mol_type = other DNA
gaaattgtgttgacgcagtctccaggcaccctgcctttgtttccaggggaaagagccaccctctcctgtagggccagtcagagtgttaacaacaaattcttagcctggtaccagcagaaatctggccaggctcccaggctcctcatctatggtgcatccagcagggccactggcatcccagacaggttcagtggcagtgggtctgggaccgacttcactctcaccatcagcggactggagcctgaagattttgaagtgtattattgtcaagtatatggtaactcactcactttcggcggagggaccaaggtggagatcaaa

SEQ ID NO: 716 - protein, 107 aa, synthetic construct
  REGION 1..107: note = Synthetic
EIVLTQSPGTLPLFPGERATLSCRASQSVNNKFLAWYQQKSGQAPRLLIYGASSRATGIPDRFSGSGSGTDFTLTISGLEPEDFEVYYCQVYGNSLTFGGGTKVEIK

SEQ ID NO: 717 - DNA, 384 bp, synthetic construct; identical to SEQ ID NO: 381
  misc_feature 1..384: note = Synthetic
  source 1..384: mol_type = other DNA

SEQ ID NO: 718 - protein, 128 aa, synthetic construct; identical to SEQ ID NO: 382
  REGION 1..128: note = Synthetic

SEQ ID NO: 719 - DNA, 321 bp, synthetic construct; identical to SEQ ID NO: 383
  misc_feature 1..321: note = Synthetic
  source 1..321: mol_type = other DNA

SEQ ID NO: 720 - protein, 107 aa, synthetic construct; identical to SEQ ID NO: 384
  REGION 1..107: note = Synthetic

SEQ ID NO: 721 - DNA, 378 bp, synthetic construct; identical to SEQ ID NO: 505
  misc_feature 1..378: note = Synthetic
  source 1..378: mol_type = other DNA

SEQ ID NO: 722 - protein, 126 aa, synthetic construct; identical to SEQ ID NO: 506
  REGION 1..126: note = Synthetic

SEQ ID NO: 723 - DNA, 24 bp, synthetic construct
  misc_feature 1..24: note = Synthetic
  source 1..24: mol_type = other DNA
ggttacacctttaccaactacgct

SEQ ID NO: 724 - protein, 8 aa, synthetic construct
  REGION 1..8: note = Synthetic
GYTFTNYA

SEQ ID NO: 725 - DNA, 24 bp, synthetic construct
  misc_feature 1..24: note = Synthetic
  source 1..24: mol_type = other DNA
gtcagcgcttacaatggtcacaca

SEQ ID NO: 726 - protein, 8 aa, synthetic construct
  REGION 1..8: note = Synthetic
VSAYNGHT

SEQ ID NO: 727 - DNA, 57 bp, synthetic construct; identical to SEQ ID NO: 511
  misc_feature 1..57: note = Synthetic
  source 1..57: mol_type = other DNA

SEQ ID NO: 728 - protein, 19 aa, synthetic construct
  REGION 1..19: note = Synthetic
ARGGVVVPVAPHFYNGMDV

SEQ ID NO: 729 - DNA, 336 bp, synthetic construct
  misc_feature 1..336: note = Synthetic
  source 1..336: mol_type = other DNA
gatattgtgatgactcagtttccactctccctgcccgtcacccctggagagccggcctccatctcctgcaggtctagtcagagcctcctgcatattaatgaatacaactatttggattggtacctaaagaagccagggcagtctccacagctcctgatctatttgggttttaatcgggcctccggggtccctgacaggttcagtggcagtggatcaggcacagattttacactgaaaatcagcagagtggaggctgaggatgttggggtctattactgcatgcaagctcttcaaactccgtggacgttcggccaagggaccaaggtggaaatcaaa

SEQ ID NO: 730 - protein, 112 aa, synthetic construct
  REGION 1..112: note = Synthetic
DIVMTQFPLSLPVTPGEPASISCRSSQSLLHINEYNYLDWYLKKPGQSPQLLIYLGFNRASGVPDRFSGSGSGTDFTLKISRVEAEDVGVYYCMQALQTPWTFGQGTKVEIK

SEQ ID NO: 731 - DNA, 33 bp, synthetic construct; identical to SEQ ID NO: 515
  misc_feature 1..33: note = Synthetic
  source 1..33: mol_type = other DNA

SEQ ID NO: 732 - protein, 11 aa, synthetic construct
  REGION 1..11: note = Synthetic
QSLLHINEYNY

SEQ ID NO: 733-734 - skipped (2 entries)

SEQ ID NO: 735 - DNA, 27 bp, synthetic construct
  misc_feature 1..27: note = Synthetic
  source 1..27: mol_type = other DNA
atgcaagctcttcaaactccgtggacg

SEQ ID NO: 736 - protein, 9 aa, synthetic construct
  REGION 1..9: note = Synthetic
MQALQTPWT

SEQ ID NO: 737 - DNA, 378 bp, synthetic construct; identical to SEQ ID NO: 521
  misc_feature 1..378: note = Synthetic
  source 1..378: mol_type = other DNA

SEQ ID NO: 738 - protein, 126 aa, synthetic construct; identical to SEQ ID NO: 522
  REGION 1..126: note = Synthetic

SEQ ID NO: 739 - DNA, 336 bp, synthetic construct
  misc_feature 1..336: note = Synthetic
  source 1..336: mol_type = other DNA
gatattgtgatgactcagtctccactctccctgcccgtcacccctggagagccggcctccatctcctgcaggtctagtcagagcctcctgcatattaatgaatacaactatttggattggtacctaaagaagccagggcagtctccacagctcctgatctatttgggttttaatcgggcctccggggtccctgacaggttcagtggcagtggatcaggcacagattttacactgaaaatcagcagagtggaggctgaggatgttggggtctattactgcatgcaagctcttcaaactccgtggacgttcggccaagggaccaaggtggaaatcaaa

SEQ ID NO: 740 - protein, 112 aa, synthetic construct
  REGION 1..112: note = Synthetic
DIVMTQSPLSLPVTPGEPASISCRSSQSLLHINEYNYLDWYLKKPGQSPQLLIYLGFNRASGVPDRFSGSGSGTDFTLKISRVEAEDVGVYYCMQALQTPWTFGQGTKVEIK

SEQ ID NO: 741 - DNA, 378 bp, synthetic construct; identical to SEQ ID NO: 525
  misc_feature 1..378: note = Synthetic
  source 1..378: mol_type = other DNA

SEQ ID NO: 742 - protein, 126 aa, synthetic construct; identical to SEQ ID NO: 526
  REGION 1..126: note = Synthetic

SEQ ID NO: 743 - DNA, 336 bp, synthetic construct; identical to SEQ ID NO: 527
  misc_feature 1..336: note = Synthetic
  source 1..336: mol_type = other DNA

SEQ ID NO: 744 - protein, 112 aa, synthetic construct; identical to SEQ ID NO: 528
  REGION 1..112: note = Synthetic

SEQ ID NO: 745-750 - skipped (6 entries)

SEQ ID NO: 751 - protein, 330 aa, synthetic construct [sequence omitted]

SEQ ID NO: 752 - protein, 327 aa, synthetic construct
  REGION 1..327: note = Synthetic
ASTKGPSVFPLAPCSRSTSESTAALGCLVKDYFPEPVTVSWNSGALTSGVHTFPAVLQSSGLYSLSSVVTVPSSSLGTKTYTCNVDHKPSNTKVDKRVESKYGPPCPSCPAPEFLGGPSVFLFPPKPKDTLMISRTPEVTCVVVDVSQEDPEVQFNWYVDGVEVHNAKTKPREEQFNSTYRVVSVLTVLHQDWLNGKEYKCKVSNKGLPSSIEKTISKAKGQPREPQVYTLPPSQEEMTKNQVSLTCLVKGFYPSDIAVEWESNGQPENNYKTTPPVLDSDGSFFLYSRLTVDKSRWQEGNVFSCSVMHEALHNHYTQKSLSLSLGK

SEQ ID NO: 753 - protein, 327 aa, synthetic construct
  REGION 1..327: note = Synthetic
ASTKGPSVFPLAPCSRSTSESTAALGCLVKDYFPEPVTVSWNSGALTSGVHTFPAVLQSSGLYSLSSVVTVPSSSLGTKTYTCNVDHKPSNTKVDKRVESKYGPPCPPCPAPEFLGGPSVFLFPPKPKDTLMISRTPEVTCVVVDVSQEDPEVQFNWYVDGVEVHNAKTKPREEQFNSTYRVVSVLTVLHQDWLNGKEYKCKVSNKGLPSSIEKTISKAKGQPREPQVYTLPPSQEEMTKNQVSLTCLVKGFYPSDIAVEWESNGQPENNYKTTPPVLDSDGSFFLYSRLTVDKSRWQEGNVFSCSVMHEALHNHYTQKSLSLSLGK

SEQ ID NO: 754 - DNA, 2076 bp, Homo sapiens
  source 1..2076: mol_type = genomic DNA
atgggcaccgtcagctccaggcggtcctggtggccgctgccactgctgctgctgctgctgctgctcctgggtcccgcgggcgcccgtgcgcaggaggacgaggacggcgactacgaggagctggtgctagccttgcgttccgaggaggacggcctggccgaagcacccgagcacggaaccacagccaccttccaccgctgcgccaaggatccgtggaggttgcctggcacctacgtggtggtgctgaaggaggagacccacctctcgcagtcagagcgcactgcccgccgcctgcaggcccaggctgcccgccggggatacctcaccaagatcctgcatgtcttccatggccttcttcctggcttcctggtgaagatgagtggcgacctgctggagctggccttgaagttgccccatgtcgactacatcgaggaggactcctctgtctttgcccagagcatcccgtggaacctggagcggattacccctccacggtaccgggcggatgaataccagccccccgacggaggcagcctggtggaggtgtatctcctagacaccagcatacagagtgaccaccgggaaatcgagggcagggtcatggtcaccgacttcgagaatgtgcccgaggaggacgggacccgcttccacagacaggccagcaagtgtgacagtcatggcacccacctggcaggggtggtcagcggccgggatgccggcgtggccaagggtgccagcatgcgcagcctgcgcgtgctcaactgccaagggaagggcacggttagcggcaccctcataggcctggagtttattcggaaaagccagctggtccagcctgtggggccactggtggtgctgctgcccctggcgggtgggtacagccgcgtcctcaacgccgcctgccagcgcctggcgagggctggggtcgtgctggtcaccgctgccggcaacttccgggacgatgcctgcctctactccccagcctcagctcccgaggtcatcacagttggggccaccaatgcccaggaccagccggtgaccctggggactttggggaccaactttggccgctgtgtggacctctttgccccaggggaggacatcattggtgcctccagcgactgcagcacctgctttgtgtcacagagtgggacatcacaggctgctgcccacgtggctggcattgcagccatgatgctgtctgccgagccggagctcaccctggccgagttgaggcagagactgatccacttctctgccaaagatgtcatcaatgaggcctggttccctgaggaccagcgggtactgacccccaacctggtggccgccctgccccccagcacccatggggcaggttggcagctgttttgcaggactgtgtggtcagcacactcggggcctacacggatggccacagccatcgcccgctgcgccccagatgaggagctgctgagctgctccagtttctccaggagtgggaagcggcggggcgagcgcatggaggcccaagggggcaagctggtctgccgggcccacaacgcttttgggggtgagggtgtctacgccattgccaggtgctgcctgctaccccaggccaactgcagcgtccacacagctccaccagctgaggccagcatggggacccgtgtccactgccaccaacagggccacgtcctcacaggctgcagctcccactgggaggtggaggaccttggcacccacaagccgcctgtgctgaggccacgaggtcagcccaaccagtgcgtgggccacagggaggccagcatccacgcttcctgctgccatgccccaggtctggaatgcaaagtcaaggagcatggaatcccggcccctcaggagcaggtgaccgtggcctgcgaggagggctggaccctgactggctgcagtgccctccctgggacctcccacgtcctgggggcctacgccgtagacaacacgtgtgtagtcaggagccgggacgtcagcactacaggcagcaccagcgaagaggccgtgacagccgttgccatctgctgccggagccggcacctggcgcaggcctcccaggagctccag

SEQ ID NO: 755 - protein, 692 aa, Homo sapiens
MGTVSSRRSWWPLPLLLLLLLLLGPAGARAQEDEDGDYEELVLALRSEEDGLAEAPEHGTTATFHRCAKDPWRLPGTYVVVLKEETHLSQSERTARRLQAQAARRGYLTKILHVFHGLLPGFLVKMSGDLLELALKLPHVDYIEEDSSVFAQSIPWNLERITPPRYRADEYQPPDGGSLVEVYLLDTSIQSDHREIEGRVMVTDFENVPEEDGTRFHRQASKCDSHGTHLAGVVSGRDAGVAKGASMRSLRVLNCQGKGTVSGTLIGLEFIRKSQLVQPVGPLVVLLPLAGGYSRVLNAACQRLARAGVVLVTAAGNFRDDACLYSPASAPEVITVGATNAQDQPVTLGTLGTNFGRCVDLFAPGEDIIGASSDCSTCFVSQSGTSQAAAHVAGIAAMMLSAEPELTLAELRQRLIHFSAKDVINEAWFPEDQRVLTPNLVAALPPSTHGAGWQLFCRTVWSAHSGPTRMATAIARCAPDEELLSCSSFSRSGKRRGERMEAQGGKLVCRAHNAFGGEGVYAIARCCLLPQANCSVHTAPPAEASMGTRVHCHQQGHVLTGCSSHWEVEDLGTHKPPVLRPRGQPNQCVGHREASIHASCCHAPGLECKVKEHGIPAPQEQVTVACEEGWTLTGCSALPGTSHVLGAYAVDNTCVVRSRDVSTTGSTSEEAVTAVAICCRSRHLAQASQELQ

SEQ ID NO: 756 - protein, 692 aa, Macaca mulatta
MGTVSSRRSWWPLPLPLLLLLLLGPAGARAQEDEDGDYEELVLALRSEEDGLADAPEHGATATFHRCAKDPWRLPGTYVVVLKEETHRSQSERTARRLQAQAARRGYLTKILHVFHHLLPGFLVKMSGDLLELALKLPHVDYIEEDSSVFAQSIPWNLERITPARYRADEYQPPKGGSLVEVYLLDTSIQSDHREIEGRVMVTDFESVPEEDGTRFHRQASKCDSHGTHLAGVVSGRDAGVAKGAGLRSLRVLNCQGKGTVSGTLIGLEFIRKSQLVQPVGPLVVLLPLAGGYSRVFNAACQRLARAGVVLVTAAGNFRDDACLYSPASAPEVITVGATNAQDQPVTLGTLGTNFGRCVDLFAPGEDIIGASSDCSTCFVSRSGTSQAAAHVAGIAAMMLSAEPELTLAELRQRLIHFSAKDVINEAWFPEDQRVLTPNLVAALPPSTHRAGWQLFCRTVWSAHSGPTRMATAVARCAQDEELLSCSSFSRSGKRRGERIEAQGGKRVCRAHNAFGGEGVYAIARCCLLPQVNCSVHTAPPAGASMGTRVHCHQQGHVLTGCSSHWEVEDLGTHKPPVLRPRGQPNQCVGHREASIHASCCHAPGLECKVKEHGIPAPQEQVIVACEDGWTLTGCSPLPGTSHVLGAYAVDNTCVVRSRDVSTTGSTSKEAVAAVAICCRSRHLVQASQELQ

SEQ ID NO: 757 - protein, 694 aa, Mus musculus
MGTHCSAWLRWPLLPLLPPLLLLLLLLCPTGAGAQDEDGDYEELMLALPSQEDGLADEAAHVATATFRRCSKEAWRLPGTYIVVLMEETQRLQIEQTAHRLQTRAARRGYVIKVLHIFYDLFPGFLVKMSSDLLGLALKLPHVEYIEEDSFVFAQSIPWNLERIIPAWHQTEEDRSPDGSSQVEVYLLDTSIQGAHREIEGRVTITDFNSVPEEDGTRFHRQASKCDSHGTHLAGVVSGRDAGVAKGTSLHSLRVLNCQGKGTVSGTLIGLEFIRKSQLIQPSGPLVVLLPLAGGYSRILNAACRHLARTGVVLVAAAGNFRDDACLYSPASAPEVITVGATNAQDQPVTLGTLGTNFGRCVDLFAPGKDIIGASSDCSTCFMSQSGTSQAAAHVAGIVARMLSREPTLTLAELRQRLIHFSTKDVINMAWFPEDQQVLTPNLVATLPPSTHETGGQLLCRTVWSAHSGPTRTATATARCAPEEELLSCSSFSRSGRRRGDWIEAIGGQQVCKALNAFGGEGVYAVARCCLVPRANCSIHNTPAARAGLETHVHCHQKDHVLTGCSFHWEVEDLSVRRQPALRSRRQPGQCVGHQAASVYASCCHAPGLECKIKEHGISGPSEQVTVACEAGWTLTGCNVLPGASLTLGAYSVDNLCVARVHDTARADRTSGEATVAAAICCRSRPSAKASWVQ

SEQ ID NO: 758 - protein, 653 aa, Homo sapiens
EFRCHDGKCISRQFVCDSDRDCLDGSDEASCPVLTCGPASFQCNSSTCIPQLWACDNDPDCEDGSDEWPQRCRGLYVFQGDSSPCSAFEFHCLSGECIHSSWRCDGGPDCKDKSDEENCAVATCRPDEFQCSDGNCIHGSRQCDREYDCKDMSDEVGCVNVTLCEGPNKFKCHSGECITLDKVCNMARDCRDWSDEPIKECGTNECLDNNGGCSHVCNDLKIGYECLCPDGFQLVAQRRCEDIDECQDPDTCSQLCVNLEGGYKCQCEEGFQLDPHTKACKAVGSIAYLFFTNRHEVRKMTLDRSEYTSLIPNLRNVVALDTEVASNRIYWSDLSQRMICSTQLDRAHGVSSYDTVISRDIQAPDGLAVDWIHSNIYWTDSVLGTVSVADTKGVKRKTLFRENGSKPRAIVVDPVHGFMYWTDWGTPAKIKKGGLNGVDIYSLVTENIQWPNGITLDLLSGRLYWVDSKLHSISSIDVNGGNRKTILEDEKRLAHPFSLAVFEDKVFWTDIINEAIFSANRLTGSDVNLLAENLLSPEDMVLFHNLTQPRGVNWCERTTLSNGGCQYLCLPAPQINPHSPKFTCACPDGMLLARDMRSCLTEAEAAVATQETSTVRLKVSSTAVRTQHTTTRPVPDTSRLPGATPGLTTVEIV

SEQ ID NO: 759 - protein, 753 aa, Homo sapiens
MERRAWSLQCTAFVLFCAWCALNSAKAKRQFVNEWAAEIPGGPEAASAIAEELGYDLLGQIGSLENHYLFKHKNHPRRSRRSAFHITKRLSDDDRVIWAEQQYEKERSKRSALRDSALNLFNDPMWNQQWYLQDTRMTAALPKLDLHVIPVWQKGITGKGVVITVLDDGLEWNHTDIYANYDPEASYDFNDNDHDPFPRYDPTNENKHGTRCAGEIAMQANNHKCGVGVAYNSKVGGIRMLDGIVTDAIEASSIGFNPGHVDIYSASWGPNDDGKTVEGPGRLAQKAFEYGVKQGRQGKGSIFVWASGNGGRQGDNCDCDGYTDSIYTISISSASQQGLSPWYAEKCSSTLATSYSSGDYTDQRITSADLHNDCTETHTGTSASAPLAAGIFALALEANPNLTWRDMQHLVVWTSEYDPLANNPGWKKNGAGLMVNSRFGFGLLNAKALVDLADPRTWRSVPEKKECVVKDNDFEPRALKANGEVIIEIPTRACEGQENAIKSLEHVQFEATIEYSRRGDLHVTLTSAAGTSTVLLAERERDTSPNGFKNWDFMSVHTWGENPIGTWTLRITDMSGRIQNEGRIVNWKLILHGTSSQPEHMKQPRVYTSYNTVQNDRRGVEKMVDPGEEQPTQENPKENTLVSKSPSSSSVGGRRDELEEGAPSQAMLRLLQSAFSKNSPPKQSPKKSPSAKLNIPYENFYEALEKLNKPSQLKDSEDSLYNDYVDVFYNTKPYKHRDDRLLQALVDILNEEN

SEQ ID NO: 760 - protein, 785 aa, Homo sapiens
MPKGRQKVPHLDAPLGLPTCLWLELAGLFLLVPWVMGLAGTGGPDGQGTGGPSWAVHLESLEGDGEEETLEQQADALAQAAGLVNAGRIGELQGHYLFVQPAGHRPALEVEAIRQQVEAVLAGHEAVRWHSEQRLLRRAKRSVHFNDPKYPQQWHLNNRRSPGRDINVTGVWERNVTGRGVTVVVVDDGVEHTIQDIAPNYSPEGSYDLNSNDPDPMPHPDVENGNHHGTRCAGEIAAVPNNSFCAVGVAYGSRIAGIRVLDGPLTDSMEAVAFNKHYQINDIYSCSWGPDDDGKTVDGPHQLGKAALQHGVIAGRQGFGSIFVVASGNGGQHNDNCNYDGYANSIYTVTIGAVDEEGRMPFYAEECASMLAVTFSGGDKMLRSIVTTDWDLQKGTGCTEGHTGTSAAAPLAAGMIALMLQVRPCLTWRDVQHIIVFTATRYEDRRAEWVTNEAGFSHSHQHGFGLLNAWRLVNAAKIWTSVPYLASYVSPVLKENKAIPQSPRSLEVLWNVSRMDLEMSGLKTLEHVAVTVSITHPRRGSLELKLFCPSGMMSLIGAPRSMDSDPNGFNDWTFSTVRCWGERARGTYRLVIRDVGDESFQVGILRQWQLTLYGSVWSAVDIRDRQRLLESAMSGKYLHDDFALPCPPGLKIPEEDGYTITPNTLKTLVLVGCFTVFWTVYYMLEVYLSQRNVASNQVCRSGPCHWPHRSRKAKEEGTELESVPLCSSKDPDEVETESRGPPTTSDLLAPDLLEQGDWSLSQNKSALDCPHQHLDVPHGKEEQIC

SEQ ID NO: 761 - protein, 692 aa, Macaca fascicularis
MGTVSSRRSWWPLPLPLLLLLLLGPAGARAQEDEDGDYEELVLALRSEEDGLADAPEHGATATFHRCAKDPWRLPGTYVVVLKEETHRSQSERTARRLQAQAARRGYLTKILHVFHHLLPGFLVKMSGDLLELALKLPHVDYIEEDSSVFAQSIPWNLERITPARYRADEYQPPKGGSLVEVYLLDTSIQSDHREIEGRVMVTDFESVPEEDGTRFHRQASKCDSHGTHLAGVVSGRDAGVAKGAGLRSLRVLNCQGKGTVSGTLIGLEFIRKSQLVQPVGPLVVLLPLAGGYSRVFNAACQRLARAGVVLVTAAGNFRDDACLYSPASAPEVITVGATNAQDQPVTLGTLGTNFGRCVDLFAPGEDIIGASSDCSTCFVSRSGTSQAAAHVAGIAAMMLSAEPELTLAELRQRLIHFSAKDVINEAWFPEDQRVLTPNLVAALPPSTHRAGWQLFCRTVWSAHSGPTRMATAVARCAQDEELLSCSSFSRSGKRRGERIEAQGGKRVCRAHNAFGGEGVYAIARCCLLPQVNCSVHTAPPAGASMGTRVHCHQQGHVLTGCSSHWEVEDLGTHKPPVLRPRGQPNQCVGHREASIHASCCHAPGLECKVKEHGIPAPQEQVIVACEDGWTLTGCSALPGTSHVLGAYAVDNTCVVRSRDVSTTGSTSEEAVAAVAICCRSRHLVQASQELQ

SEQ ID NO: 762 - protein, 698 aa, Mesocricetus auratus
MGTSCSARPRWLLSPLLLLLLLLRYMGASAQDEDAEYEELMLTLQSQDDGLADETDEAPQGATAAFHRCPEEAWRVPGTYIVMLAEEAQWVHIEQTMHRLQTQAARRGYVIKIQHIFYDFLPAFVVKMSSDLLDLALKLPHVKYIEEDSLVFAQSIPWNLDRIIPAGRQAQEYSSSRKVPSGSGQVEVYLLDTSIQSDHREIEGRVTVTDFNSVPEEDGTRFHRQASKCDSHGTHLAGVVSGRDAGVAKGTILHGLRVLNCQGKGIVSGILTGLEFIWKSQLMQPSGPQVVLLPLAGRYSRVLNTACQHLARTGVVLVAAAGNFRDDACLYSPASAPEVITVGATDVQDQPVTLGTLGTNFGRCVDLFAPGKDIIGASSDCSACFMSQSGTSQAAAHVAGIVAMMLTLEPELTLTELRQRLIHFSTKDAINMAWFPEDQRVLTPNLVATLPPSTHGTGGQLLCRTVWSAHSGPTRAATATARCAPGEELLSCSSFSRSGRRRGDRIEAAGTQQVCKALNAFGGEGVYAVARCCLLPRANCSIHTTPAARTSLETHAHCHQKDHVLTGCSLHWEVEGIGVQPLAVLRSRHQPGQCTGHREASVHASCCHAPGLECKIKEHGISGPAEQVTVACEAGWTLTGCNVLPGAFITLGAYAVDNTCVARSRVTDTAGRTGEEATVAAAICCRNRPSAKASWVHQ

SEQ ID NO: 763 - protein, 691 aa, Rattus norvegicus
MGIRCSTWLRWPLSPQLLLLLLLCPTGSRAQDEDGDYEELMLALPSQEDSLVDEASHVATATFRRCSKEAWRLPGTYVVVLMEETQRLQVEQTAHRLQTWAARRGYVIKVLHVFYDLFPGFLVKMSSDLLGLALKLPHVEYIEEDSLVFAQSIPWNLERIIPAWQQTEEDSSPDGSSQVEVYLLDTSIQSGHREIEGRVTITDFNSVPEEDGTRFHRQASKCDSHGTHLAGVVSGRDAGVAKGTSLHSLRVLNCQGKGTVSGTLIGLEFIRKSQLIQPSGPLVVLLPLAGGYSRILNTACQRLARTGVVLVAAAGNFRDDACLYSPASAPEVITVGATNAQDQPVTLGTLGTNFGRCVDLFAPGKDIIGASSDCSTCYMSQSGTSQAAAHVAGIVAMMLNRDPALTLAELRQRLILFSTKDVINMAWFPEDQRVLTPNRVATLPPSTQETGGQLLCRTVWSAHSGPTRTATATARCAPEEELLSCSSFSRSGRRRGDRIEAIGGQQVCKALNAFGGEGVYAVARCCLLPRVNCSIHNTPAARAGPQTPVHCHQKDHVLTGCSFHWEVENLRAQQQPLLRSRHQPGQCVGHQEASVHASCCHAPGLECKIKEHGIAGPAEQVTVACEAGWTLTGCNVLPGASLPLGAYSVDNVCVARIRDAGRADRTSEEATVAAAICCRSRPSAKASWVHQ